European Patent Application EP 4 223 766 A2, published August 9, 2023. Title: ENGINEERED IMINE REDUCTASES AND METHODS FOR THE REDUCTIVE AMINATION OF KETONE AND AMINE COMPOUNDS. Applicant: Codexis, Inc. Application US 62380165, filed August 26, 2016. The sequence listing filed with the application follows.

SEQUENCE LISTING (270 sequences)

SEQ ID NO: 1 - DNA, 879 bp, synthetic construct
  misc_feature 1..879: note = Imine reductase from Pseudonocardia spinosispora
  source 1..879: mol_type = other DNA
atgagtgattcccccgtacctgtgactgttctgggtcttggtctgatgggtcaggccttagcgggagcgtttctggcagccggtcaccctacgacggtttggaatcgcagcgcagctaaagctgatgaactggttggtcgcggtgcaaccctggccgcgtctcccgcggctgccgtcgcagcgggtagtctgatcgttgtttgcgtcacagatcatcgtgcggtgcgcgaactgctggaaccacttggcgatgcactgccaggtcgcgttctggtcaacctgacgagcggtacgtcgcgtgaagcccgtgagaacgcagaacatactgcggctcagggagccacctacctggatggtgtgattctgaccattccaagcggcattggcaccccagaagctaccattctgtattcgggaccgcgcagtaccttcgatgaacatgaaagcgcactgcgcgcattaggtccgggggcgacctttgtaggggaagatcacggactggctgcactgtatgatgcagcaatgctgagcgtcatgtggggcctgctgaatggtttcctgcatggaaccgcactgctgggaaccgcgggcgtttcggcaacctctgtggttccgatgctgggtcaaggtatcgaagcggtgaccggttggattgcgcgctacgcagatcagattgatgccggtgtctatccagcagacgacgccacgattgatacccagcgtgctgcaatgcagcacctggtcgaggagagccgtgcggcgggcatcaatggcgaacttccggcgtttgtgaccaaactggccgatcgcgcagtggcagaaggtcgtggtggtgactcttacgctgcactgattgaacagtttcgcaagtcagcttaa

SEQ ID NO: 2 - protein, 292 aa, synthetic construct
  REGION 1..292: note = Imine reductase from Pseudonocardia spinosispora
MSDSPVPVTVLGLGLMGQALAGAFLAAGHPTTVWNRSAAKADELVGRGATLAASPAAAVAAGSLIVVCVTDHRAVRELLEPLGDALPGRVLVNLTSGTSREARENAEHTAAQGATYLDGVILTIPSGIGTPEATILYSGPRSTFDEHESALRALGPGATFVGEDHGLAALYDAAMLSVMWGLLNGFLHGTALLGTAGVSATSVVPMLGQGIEAVTGWIARYADQIDAGVYPADDATIDTQRAAMQHLVEESRAAGINGELPAFVTKLADRAVAEGRGGDSYAALIEQFRKSA

SEQ ID NO: 3 - DNA, 879 bp, synthetic construct
  misc_feature 1..879: note = Imine reductase variant from Pseudonocardia spinosispora
  source 1..879: mol_type = other DNA
atgagtgattcccccgtacctgtgactgttctgggtcttggtctgatgggtcaggccttagcgggagcgtttctggcagccggtcaccctacgacggtttggaatcgcagcgcagctaaagctgatgaactggttggtcgcggtgcaaccctggccgcgtctcccgcggctgccgtcgcagcgggtagtctgatcgttgtttgcgtcacagatcatcgtgcggtgcgcgaactgctggaaccacttggcgatgcactgccaggtcgcgttctggtcaacctgacgagcggtacgtcgcgtgaagcccgtgagaacgcagaacatactgcggctcagggagccacctacctggatggtgtgattctgggtattccaagcggcattggcaccccagaagctaccattctgtattcgggaccgcgcagtaccttcgatgaacatgaaagcgcactgcgcgcattaggtccgggggcgacctttgtaggggaagatcacggactggctgcactgtatgatgcagcaatgctgagcgtcatgtggggcctgctgaatggtttcctgcatggaaccgcactgctgggaaccgcgggcgtttcggcaacctctgtggttccgatgctgggtcaaggtatcgaagcggtgaccggttggattgcgcgctacgcagatcagattgatgccggtgtctatccagcagacgacgccacgattgatacccagcgtgctgcaatgcagcacctggtcgaggagagccgtgcggcgggcatcaatggcgaacttccggcgtttgtgaccaaactggccgatcgcgcagtggcagaaggtcgtggtggtgactcttacgctgcactgattgaacagtttcgcaagtcagcttaa

SEQ ID NO: 4 - protein, 292 aa, synthetic construct
  REGION 1..292: note = Imine reductase variant from Pseudonocardia spinosispora
MSDSPVPVTVLGLGLMGQALAGAFLAAGHPTTVWNRSAAKADELVGRGATLAASPAAAVAAGSLIVVCVTDHRAVRELLEPLGDALPGRVLVNLTSGTSREARENAEHTAAQGATYLDGVILGIPSGIGTPEATILYSGPRSTFDEHESALRALGPGATFVGEDHGLAALYDAAMLSVMWGLLNGFLHGTALLGTAGVSATSVVPMLGQGIEAVTGWIARYADQIDAGVYPADDATIDTQRAAMQHLVEESRAAGINGELPAFVTKLADRAVAEGRGGDSYAALIEQFRKSA

SEQ ID NO: 5 - DNA, 879 bp, synthetic construct
  misc_feature 1..879: note = Imine reductase variant from Pseudonocardia spinosispora
  source 1..879: mol_type = other DNA
atgagtgattcccccgtacctgtgactgttctgggtcttggtctgatgggtcaggccttagcgggagcgtttctggcagccggtcaccctacgacggtttggaatcgcagcgcagctaaagctgatgaactggttggtcgcggtgcaaccctggccgcgtctcccgcggctgccgtcgcagcgggtagtctgatcgttgtttgcgtcacagatcatcgtgcggtgcgcgaactgctggaaccacttggcgatgcactgccaggtcgcgttctggtcaacctgacgagcggtacgtcgcgtgaagcccgtgagaacgcagaacatactgcggctcagggagccacctacctggatggtgtgattctgaccattccaagcggcattggcaccccacatgctaccattctgtattcgggaccgcgcagtaccttcgatgaacatgaaagcgcactgcgcgcattaggtccgggggcgacctttgtaggggaagatcacggactggctgcactgtatgatgcagcaatgctgagcgtcatgtggggcctgctgaatggtttcctgcatggaaccgcactgctgggaaccgcgggcgtttcggcaacctctgtggttccgatgctgggtcaaggtatcgaagcggtgaccggttggattgcgcgctacgcagatcagattgatgccggtgtctatccagcagacgacgccacgattgatacccagcgtgctgcaatgcagcacctggtcgaggagagccgtgcggcgggcatcaatggcgaacttccggcgtttgtgaccaaactggccgatcgcgcagtggcagaaggtcgtggtggtgactcttacgctgcactgattgaacagtttcgcaagtcagcttaa

SEQ ID NO: 6 - protein, 292 aa, synthetic construct
  REGION 1..292: note = Imine reductase variant from Pseudonocardia spinosispora
MSDSPVPVTVLGLGLMGQALAGAFLAAGHPTTVWNRSAAKADELVGRGATLAASPAAAVAAGSLIVVCVTDHRAVRELLEPLGDALPGRVLVNLTSGTSREARENAEHTAAQGATYLDGVILTIPSGIGTPHATILYSGPRSTFDEHESALRALGPGATFVGEDHGLAALYDAAMLSVMWGLLNGFLHGTALLGTAGVSATSVVPMLGQGIEAVTGWIARYADQIDAGVYPADDATIDTQRAAMQHLVEESRAAGINGELPAFVTKLADRAVAEGRGGDSYAALIEQFRKSA

SEQ ID NO: 7 - DNA, 879 bp, synthetic construct
  misc_feature 1..879: note = Imine reductase variant from Pseudonocardia spinosispora
  source 1..879: mol_type = other DNA
atgagtgattcccccgtacctgtgactgttctgggtcttggtctgatgggtcaggccttagcgggagcgtttctggcagccggtcaccctacgacggtttggaatcgcagcgcagctaaagctgatgaactggttggtcgcggtgcaaccctggccgcgtctcccgcggctgccgtcgcagcgggtagtctgatcgttgtttgcgtcacagatcatcgtgcggtgcgcgaactgctggaaccacttggcgatgcactgccaggtcgcgttctggtcaacctgacgagcggtacgtcgcgtgaagcccgtgagaacgcagaacatactgcggctcagggagccacctacctggatggtgtgattctgaccgcaccaagcggcattggcaccccagaagctaccattctgtattcgggaccgcgcagtaccttcgatgaacatgaaagcgcactgcgcgcattaggtccgggggcgacctttgtaggggaagatcacggactggctgcactgtatgatgcagcaatgctgagcatcatgtggggcctgctgaatggtttcctgcatggaaccgcactgctgggaaccgcgggcgtttcggcaacctctgtggttccgatgctgggtcaaggtatcgaagcggtgaccggttggattgcgcgctacgcagatcagattgatgccggtgtctatccagcagacgacgccacgattgatacccagcgtgctgcaatgcagcacctggtcgaggagagccgtgcggcgggcatcaatggcgaacttccggcgtttgtgaccaaactggccgatcgcgcagtggcagaaggtcgtggtggtgactcttacgctgcactgattgaacagtttcgcaagtcagcttaa

SEQ ID NO: 8 - protein, 292 aa, synthetic construct
  REGION 1..292: note = Imine reductase variant from Pseudonocardia spinosispora
MSDSPVPVTVLGLGLMGQALAGAFLAAGHPTTVWNRSAAKADELVGRGATLAASPAAAVAAGSLIVVCVTDHRAVRELLEPLGDALPGRVLVNLTSGTSREARENAEHTAAQGATYLDGVILTAPSGIGTPEATILYSGPRSTFDEHESALRALGPGATFVGEDHGLAALYDAAMLSIMWGLLNGFLHGTALLGTAGVSATSVVPMLGQGIEAVTGWIARYADQIDAGVYPADDATIDTQRAAMQHLVEESRAAGINGELPAFVTKLADRAVAEGRGGDSYAALIEQFRKSA

SEQ ID NO: 9 - DNA, 879 bp, synthetic construct
  misc_feature 1..879: note = Imine reductase variant from Pseudonocardia spinosispora
  source 1..879: mol_type = other DNA
atgagtgattcccccgtacctgtgactgttctgggtcttggtctgatgggtcaggccttagcgggagcgtttctggcagccggtcaccctacgacggtttggaatcgcagcgcagctaaagctgatgaactggttggtcgcggtgcaaccctggccgcgtctcccgcggctgccgtcgcagcgggtagtctgatcgttgtttgcgtcacagatcatcgtgcggtgcgcgaactgctggaaccacttggcgatgcactgccaggtcgcgttctggtcaacctgacgagcggtacgtcgcgtgaagcccgtgagaacgcagaacatactgcggctcagggagccacctacctggatggtgtgattctgaccggtccaagcggcattggcaccccagaagctaccattctgtattcgggaccgcgcagtaccttcgatgaacatgaaagcgcactgcgcgcattaggtccgggggcgacctttgtaggggaagatcacggactggctgcactgtatgatgcagcaatgctgagcgtcatgtggggcctgctgaatggtttcctgcatggaaccgcactgctgggaaccgcgggcgtttcggcaacctctgtggttccgatgctgggtcaaggtatcgaagcggtgaccggttggattgcgcgctacgcagatcagattgatgccggtgtctatccagcagacgacgccacgattgatacccagcgtgctgcaatgcagcacctggtcgaggagagccgtgcggcgggcatcaatggcgaacttccggcgtttgtgaccaaactggccgatcgcgcagtggcagaaggtcgtggtggtgactcttacgctgcactgattgaacagtttcgcaagtcagcttaa

SEQ ID NO: 10 - protein, 292 aa, synthetic construct
  REGION 1..292: note = Imine reductase variant from Pseudonocardia spinosispora
MSDSPVPVTVLGLGLMGQALAGAFLAAGHPTTVWNRSAAKADELVGRGATLAASPAAAVAAGSLIVVCVTDHRAVRELLEPLGDALPGRVLVNLTSGTSREARENAEHTAAQGATYLDGVILTGPSGIGTPEATILYSGPRSTFDEHESALRALGPGATFVGEDHGLAALYDAAMLSVMWGLLNGFLHGTALLGTAGVSATSVVPMLGQGIEAVTGWIARYADQIDAGVYPADDATIDTQRAAMQHLVEESRAAGINGELPAFVTKLADRAVAEGRGGDSYAALIEQFRKSA

SEQ ID NO: 11 - DNA, 879 bp, synthetic construct
  misc_feature 1..879: note = Imine reductase variant from Pseudonocardia spinosispora
  source 1..879: mol_type = other DNA
atgagtgattcccccgtacctgtgactgttctgggtcttggtctgatgggtcaggccttagcgggagcgtttctggcagccggtcaccctacgacggtttggaatcgcagcgcagctaaagctgatgaactggttggtcgcggtgcaaccctggccgcgtctcccgcggctgccgtcgcagcgggtagtctgatcgttgtttgcgtcacagatcatcgtgcggtgcgcgaactgctggaaccacttggcgatgcactgccaggtcgcgttctggtcaacctgacgagcggtacgtcgcgtgaagcccgtgagaacgcagaacatactgcggctcagggagccacctacctggatggtgtgattctgaccattccaagcggcattggcaccccagaagctaccattctgtattcgggaccgcgcagtaccttcgatgaacatgaaagcgcactgcgcgcattaggtccgggggcgacctttgtaggggaagatcacggactggctgcactgtatgatcatgcaatgctgagcgtcatgtggggcctgctgaatggtttcctgcatggaaccgcactgctgggaaccgcgggcgtttcggcaacctctgtggttccgatgctgggtcaaggtatcgaagcggtgaccggttggattgcgcgctacgcagatcagattgatgccggtgtctatccagcagacgacgccacgattgatacccagcgtgctgcaatgcagcacctggtcgaggagagccgtgcggcgggcatcaatggcgaacttccggcgtttgtgaccaaactggccgatcgcgcagtggcagaaggtcgtggtggtgactcttacgctgcactgattgaacagtttcgcaagtcagcttaa

SEQ ID NO: 12 - protein, 292 aa, synthetic construct
  REGION 1..292: note = Imine reductase variant from Pseudonocardia spinosispora
MSDSPVPVTVLGLGLMGQALAGAFLAAGHPTTVWNRSAAKADELVGRGATLAASPAAAVAAGSLIVVCVTDHRAVRELLEPLGDALPGRVLVNLTSGTSREARENAEHTAAQGATYLDGVILTIPSGIGTPEATILYSGPRSTFDEHESALRALGPGATFVGEDHGLAALYDHAMLSVMWGLLNGFLHGTALLGTAGVSATSVVPMLGQGIEAVTGWIARYADQIDAGVYPADDATIDTQRAAMQHLVEESRAAGINGELPAFVTKLADRAVAEGRGGDSYAALIEQFRKSA

SEQ ID NO: 13 - DNA, 879 bp, synthetic construct
  misc_feature 1..879: note = Imine reductase variant from Pseudonocardia spinosispora
  source 1..879: mol_type = other DNA
atgagtgattcccccgtacctgtgactgttctgggtcttggtctgatgggtcaggccttagcgggagcgtttctggcagccggtcaccctacgacggtttggaatcgcagcgcagctaaagctgatgaactggttggtcgcggtgcaaccctggccgcgtctcccgcggctgccgtcgcagcgggtagtctgatcgttgtttgcgtcacagatcatcgtgcggtgcgcgaactgctggaaccacttggcgatgcactgccaggtcgcgttctggtcaacctgacgagcggtacgtcgcgtgaagcccgtgagaacgcagaacatactgcggctcagggagccacctacctggatggtgtgattctgaccattccaagcggcattggcaccccagaagctaccattctgtattcgggaccgcgcagtaccttcgatgaacatgaaagcgcactgcgcgcattaggtccgggggcgacctttgtaggggaagatcacggactggctaatctgtatgatgcagcaatgctgagcgtcatgtggggcctgctgaatggtttcctgcatggaaccgcactgctgggaaccgcgggcgtttcggcaacctctgtggttccgatgctgggtcaaggtatcgaagcggtgaccggttggattgcgcgctacgcagatcagattgatgccggtgtctatccagcagacgacgccacgattgatacccagcgtgctgcaatgcagcacctggtcgaggagagccgtgcggcgggcatcaatggcgaacttccggcgtttgtgaccaaactggccgatcgcgcagtggcagaaggtcgtggtggtgactcttacgctgcactgattgaacagtttcgcaagtcagcttaa

SEQ ID NO: 14 - protein, 292 aa, synthetic construct
  REGION 1..292: note = Imine reductase variant from Pseudonocardia spinosispora
MSDSPVPVTVLGLGLMGQALAGAFLAAGHPTTVWNRSAAKADELVGRGATLAASPAAAVAAGSLIVVCVTDHRAVRELLEPLGDALPGRVLVNLTSGTSREARENAEHTAAQGATYLDGVILTIPSGIGTPEATILYSGPRSTFDEHESALRALGPGATFVGEDHGLANLYDAAMLSVMWGLLNGFLHGTALLGTAGVSATSVVPMLGQGIEAVTGWIARYADQIDAGVYPADDATIDTQRAAMQHLVEESRAAGINGELPAFVTKLADRAVAEGRGGDSYAALIEQFRKSA

SEQ ID NO: 15 - DNA, 879 bp, synthetic construct
  misc_feature 1..879: note = Imine reductase variant from Pseudonocardia spinosispora
  source 1..879: mol_type = other DNA
atgagtgattcccccgtacctgtgactgttctgggtcttggtctgatgggtcaggccttagcgggagcgtttctggcagccggtcaccctacgacggtttggaatcgcagcgcagctaaagctgatgaactggttggtcgcggtgcaaccctggccgcgtctcccgcggctgccgtcgcagcgggtagtctgatcgttgtttgcgtcacagatcatcgtgcggtgcgcgaactgctggaaccacttggcgatgcactgccaggtcgcgttctggtcaacctgacgagcggtacgtcgcgtgaagcccgtgagaacgcagaacatactgcggctcagggagccacctacctggatggtgtgattctgaccattccaagcggcattggcaccccagaagctaccattctgtattcgggaccgcgcagtaccttcgatgaacatgaaagcgcactgcgcgcattaggtccgggggcgacctttgtaggggaagatcacggactggctgcactgtatgatgcagcaatgctgagcgtcatgtggggcctgctgaatggtttcctgcatggaaccgcactgctgggaaccgcgggcgtttcggcaacctctgtggttccgatgctgggtcaaggtatcgaagcggtgaccggttggattgcgcgctacgcagatcagattgatgccggtgtctatccagcagacttggccacgattgatacccagcgtgctgcaatgcagcacctggtcgaggagagccgtgcggcgggcatcaatggcgaacttccggcgtttgtgaccaaactggccgatcgcgcagtggcagaaggtcgtggtggtgactcttacgctgcactgattgaacagtttcgcaagtcagcttaa

SEQ ID NO: 16 - protein, 292 aa, synthetic construct
  REGION 1..292: note = Imine reductase variant from Pseudonocardia spinosispora
MSDSPVPVTVLGLGLMGQALAGAFLAAGHPTTVWNRSAAKADELVGRGATLAASPAAAVAAGSLIVVCVTDHRAVRELLEPLGDALPGRVLVNLTSGTSREARENAEHTAAQGATYLDGVILTIPSGIGTPEATILYSGPRSTFDEHESALRALGPGATFVGEDHGLAALYDAAMLSVMWGLLNGFLHGTALLGTAGVSATSVVPMLGQGIEAVTGWIARYADQIDAGVYPADLATIDTQRAAMQHLVEESRAAGINGELPAFVTKLADRAVAEGRGGDSYAALIEQFRKSA

SEQ ID NO: 17 - DNA, 879 bp, synthetic construct
  misc_feature 1..879: note = Imine reductase variant from Pseudonocardia spinosispora
  source 1..879: mol_type = other DNA
atgagtgattcccccgtacctgtgactgttctgggtcttggtctgatgggtcaggccttagcgggagcgtttctggcagccggtcaccctacgacggtttggaatcgcagcgcagctaaagctgatgaactggttggtcgcggtgcaaccctggccgcgtctcccgcggctgccgtcgcagcgggtagtctgatcgttgtttgcgtcacagatcatcgtgcggtgcgcgaactgctggaaccacttggcgatgcactgccaggtcgcgttctggtcaacctgacgagcggtacgtcgcgtgaagcccgtgagaacgcagaacatactgcggctcagggagccacctacctggatggtgtgattctgaccattccaagcggcattggcaccccagaagctaccattctgtattcgggaccgcgcagtaccttcgatgaacatgaaagcgcactgcgcgcattaggtccgggggcgacctttgtaggggaagatcacggactggctgcactgtgggatgcagcaatgctgagcgtcatgtggggcctgctgaatggtttcctgcatggaaccgcactgctgggaaccgcgggcgtttcggcaacctctgtggttccgatgctgggtcaaggtatcgaagcggtgaccggttggattgcgcgctacgcagatcagattgatgccggtgtctatccagcagacgacgccacgattgatacccagcgtgctgcaatgcagcacctggtcgaggagagccgtgcggcgggcatcaatggcgaacttccggcgtttgtgaccaaactggccgatcgcgcagtggcagaaggtcgtggtggtgactcttacgctgcactgattgaacagtttcgcaagtcagcttaa

SEQ ID NO: 18 - protein, 292 aa, synthetic construct
  REGION 1..292: note = Imine reductase variant from Pseudonocardia spinosispora
MSDSPVPVTVLGLGLMGQALAGAFLAAGHPTTVWNRSAAKADELVGRGATLAASPAAAVAAGSLIVVCVTDHRAVRELLEPLGDALPGRVLVNLTSGTSREARENAEHTAAQGATYLDGVILTIPSGIGTPEATILYSGPRSTFDEHESALRALGPGATFVGEDHGLAALWDAAMLSVMWGLLNGFLHGTALLGTAGVSATSVVPMLGQGIEAVTGWIARYADQIDAGVYPADDATIDTQRAAMQHLVEESRAAGINGELPAFVTKLADRAVAEGRGGDSYAALIEQFRKSA

SEQ ID NO: 19 - DNA, 879 bp, synthetic construct
  misc_feature 1..879: note = Imine reductase variant from Pseudonocardia spinosispora
  source 1..879: mol_type = other DNA
atgagtgattcccccgtacctgtgactgttctgggtcttggtctgatgggtcaggccttagcgggagcgtttctggcagccggtcaccctacgacggtttggaatcgcagcgcagctaaagctgatgaactggttggtcgcggtgcaaccctggccgcgtctcccgcggctgccgtcgcagcgggtagtctgatcgttgtttgcgtcacagatcatcgtgcggtgcgcgaactgctggaaccacttggcgatgcactgccaggtcgcgttctggtcaacctgacgagcggtacgtcgcgtgaagcccgtgagaacgcagaacatactgcggctcagggagccacctacctggatggtgtgattctgaccattccaagcggcattggcaccccagaagctaccattctgtattcgggaccgcgcagtaccttcgatgaacatgaaagcgcactgcgcgcattaggtccgggggcgacctttgtaggggaagatcacggactggctgcactgtatgatgcagcaatgctgagcatcatgtggggcctgctgaatggtttcctgcatggaaccgcactgctgggaaccgcgggcgtttcggcaacctctgtggttccgatgctgggtcaaggtatcgaagcggtgaccggttggattgcgcgctacgcagatcagattgatgccggtgtctatccagcagacgacgccacgattgatacccagcgttatgcaatgcagcacctggtcgaggagagccgtgcggcgggcatcaatggcgaacttccggcgtttgtgaccaaactggccgatcgcgcagtggcagaaggtcgtggtggtgactcttacgctgcactgattgaacagtttcgcaagtcagcttaa

SEQ ID NO: 20 - protein, 292 aa, synthetic construct
  REGION 1..292: note = Imine reductase variant from Pseudonocardia spinosispora
MSDSPVPVTVLGLGLMGQALAGAFLAAGHPTTVWNRSAAKADELVGRGATLAASPAAAVAAGSLIVVCVTDHRAVRELLEPLGDALPGRVLVNLTSGTSREARENAEHTAAQGATYLDGVILTIPSGIGTPEATILYSGPRSTFDEHESALRALGPGATFVGEDHGLAALYDAAMLSIMWGLLNGFLHGTALLGTAGVSATSVVPMLGQGIEAVTGWIARYADQIDAGVYPADDATIDTQRYAMQHLVEESRAAGINGELPAFVTKLADRAVAEGRGGDSYAALIEQFRKSA

SEQ ID NO: 21 - DNA, 879 bp, synthetic construct
  misc_feature 1..879: note = Imine reductase variant from Pseudonocardia spinosispora
  source 1..879: mol_type = other DNA
atgagtgattcccccgtacctgtgactgttctgggtcttggtctgatgggtcaggccttagcgggagcgtttctggcagccggtcaccctacgacggtttggaatcgcagcgcagctaaagctgatgaactggttggtcgcggtgcaaccctggccgcgtctcccgcggctgccgtcgcagcgggtagtctgatcgttgtttgcgtcacagatcatcgtgcggtgcgcgaactgctggaaccacttggcgatgcactgccaggtcgcgttctggtcaacctgacgagcggtacgtcgcgtgaagcccgtgagaacgcagaacatactgcggctcagggagccacctacctggatggtgtgattctgaccattccaagcggcattggcaccccagaagctaccattctgtattcgggaccgcgcagtaccttcgatgaacatgaaagcgcactgcgcgcattaggtccgggggcgacctttgtaggggaagatcacggactggctgcactgtatgatgcagcaatgctgagcgtcatgtggggcctgctgaatggtttcctgcatggaaccgcactgctgggaaccgcgggcgtttcggcaacctctgtggttccgatgctgggtcaaggtatcgaaacagtgaccggttggattgcgcgctacgcagatcagattgatgccggtgtctatccagcagacgacgccacgattgatacccagcgtgctgcaatgcagcacctggtcgaggagagccgtgcggcgggcatcaatggcgaacttccggcgtttgtgaccaaactggccgatcgcgcagtggcagaaggtcgtggtggtgactcttacgctgcactgattgaacagtttcgcaagtcagcttaa

SEQ ID NO: 22 - protein, 292 aa, synthetic construct
  REGION 1..292: note = Imine reductase variant from Pseudonocardia spinosispora
MSDSPVPVTVLGLGLMGQALAGAFLAAGHPTTVWNRSAAKADELVGRGATLAASPAAAVAAGSLIVVCVTDHRAVRELLEPLGDALPGRVLVNLTSGTSREARENAEHTAAQGATYLDGVILTIPSGIGTPEATILYSGPRSTFDEHESALRALGPGATFVGEDHGLAALYDAAMLSVMWGLLNGFLHGTALLGTAGVSATSVVPMLGQGIETVTGWIARYADQIDAGVYPADDATIDTQRAAMQHLVEESRAAGINGELPAFVTKLADRAVAEGRGGDSYAALIEQFRKSA

SEQ ID NO: 23 - DNA, 879 bp, synthetic construct
  misc_feature 1..879: note = Imine reductase variant from Pseudonocardia spinosispora
  source 1..879: mol_type = other DNA
atgagtgattcccccgtacctgtgactgttctgggtcttggtctgatgggtcaggccttagcgggagcgtttctggcagccggtcaccctacgacggtttggaatcgcagcgcagctaaagctgatgaactggttggtcgcggtgcaaccctggccgcgtctcccgcggctgccgtcgcagcgggtagtctgatcgttgtttgcgtcacagatcatcgtgcggtgcgcgaactgctggaaccacttggcgatgcactgccaggtcgcgttctggtcaacctgacgagcggtacgtcgcgtgaagcccgtgagaacgcagaacatactgcggctcagggagccacctacctggatggtgtgattctgaccattccaagcggcattggcaccccagaagctaccattctgtattcgggaccgcgcagtaccttcgatgaacatgaaagcgcactgcgcgcattaggtccgggggcgacctttgtaggggaagatcacggactggctgcactgtatgatgcagcaatgctgagcgtcatgtggggcctgctgaatggtttcctgcatggaaccgcactgctgggaaccgcgggcgtttcggcaacctctgtggttccgatgctgggtcaaggtatcgaagcggtgaccggtcttattgcgcgctacgcagatcagattgatgccggtgtctatccagcagacgacgccacgattgatacccagcgtgctgcaatgcagcacctggtcgaggagagccgtgcggcgggcatcaatggcgaacttccggcgtttgtgaccaaactggccgatcgcgcagtggcagaaggtcgtggtggtgactcttacgctgcactgattgaacagtttcgcaagtcagcttaa

SEQ ID NO: 24 - protein, 292 aa, synthetic construct
  REGION 1..292: note = Imine reductase variant from Pseudonocardia spinosispora
MSDSPVPVTVLGLGLMGQALAGAFLAAGHPTTVWNRSAAKADELVGRGATLAASPAAAVAAGSLIVVCVTDHRAVRELLEPLGDALPGRVLVNLTSGTSREARENAEHTAAQGATYLDGVILTIPSGIGTPEATILYSGPRSTFDEHESALRALGPGATFVGEDHGLAALYDAAMLSVMWGLLNGFLHGTALLGTAGVSATSVVPMLGQGIEAVTGLIARYADQIDAGVYPADDATIDTQRAAMQHLVEESRAAGINGELPAFVTKLADRAVAEGRGGDSYAALIEQFRKSA

SEQ ID NO: 25 - DNA, 879 bp, synthetic construct
  misc_feature 1..879: note = Imine reductase variant from Pseudonocardia spinosispora
  source 1..879: mol_type = other DNA
atgagtgattcccccgtacctgtgactgttctgggtcttggtctgatgggtcaggccttagcgggagcgtttctggcagccggtcaccctacgacggtttggaatcgcagcgcagctaaagctgatgaactggttggtcgcggtgcaaccctggccgcgtctcccgcggctgccgtcgcagcgggtagtctgatcgttgtttgcgtcacagatcatcgtgcggtgcgcgaactgctggaaccacttggcgatgcactgccaggtcgcgttctggtcaacctgacgagcggtacgtcgcgtgaagcccgtgagaacgcagaacatactgcggctcagggagccacctacctggatggtgtgattctgaccattccaagcggcattggcaccccagaagctaccattctgtattcgggaccgcgcagtaccttcgatgaacatgaaagcgcactgcgcgcattaggtccgggggcgacctttgtaggggaagatcacggactggctgcactgtatgatgcagcaatgctgagcgtcatgtggggcctgctgaatggtttcctgcatggaaccgcactgctgggaaccgcgggcgtttcggcaacctctgtggttccgatgctgggtcaaggtatcgaaagggtgaccggttggattgcgcgctacgcagatcagattgatgccggtgtctatccagcagacgacgccacgattgatacccagcgtgctgcaatgcagcacctggtcgaggagagccgtgcggcgggcatcaatggcgaacttccggcgtttgtgaccaaactggccgatcgcgcagtggcagaaggtcgtggtggtgactcttacgctgcactgattgaacagtttcgcaagtcagcttaa

SEQ ID NO: 26 - protein, 292 aa, synthetic construct
  REGION 1..292: note = Imine reductase variant from Pseudonocardia spinosispora
MSDSPVPVTVLGLGLMGQALAGAFLAAGHPTTVWNRSAAKADELVGRGATLAASPAAAVAAGSLIVVCVTDHRAVRELLEPLGDALPGRVLVNLTSGTSREARENAEHTAAQGATYLDGVILTIPSGIGTPEATILYSGPRSTFDEHESALRALGPGATFVGEDHGLAALYDAAMLSVMWGLLNGFLHGTALLGTAGVSATSVVPMLGQGIERVTGWIARYADQIDAGVYPADDATIDTQRAAMQHLVEESRAAGINGELPAFVTKLADRAVAEGRGGDSYAALIEQFRKSA

SEQ ID NO: 27 - DNA, 879 bp, synthetic construct
  misc_feature 1..879: note = Imine reductase variant from Pseudonocardia spinosispora
  source 1..879: mol_type = other DNA
atgagtgattcccccgtacctgtgactgttctgggtcttggtctgatgggtcaggccttagcgggagcgtttctggcagccggtcaccctacgacggtttggaatcgcagcgcagctaaagctgatgaactggttggtcgcggtgcaaccctggccgcgtctcccgcggctgccgtcgcagcgggtagtctgatcgttgtttgcgtcacagatcatcgtgcggtgcgcgaactgctggaaccacttggcgatgcactgccaggtcgcgttctggtcaacctgacgagcggtacgtcgcgtgaagcccgtgagaacgcagaacatactgcggctcagggagccacctacctggatggtgtgattctgaccattccaagcggcattggcaccccaagggctaccattctgtattcgggaccgcgcagtaccttcgatgaacatgaaagcgcactgcgcgcattaggtccgggggcgacctttgtaggggaagatcacggactggctgcactgtatgatgcagcaatgctgagcgtcatgtggggcctgctgaatggtttcctgcatggaaccgcactgctgggaaccgcgggcgtttcggcaacctctgtggttccgatgctgggtcaaggtatcgaagcggtgaccggttggattgcgcgctacgcagatcagattgatgccggtgtctatccagcagacgacgccacgattgatacccagcgtgctgcaatgcagcacctggtcgaggagagccgtgcggcgggcatcaatggcgaacttccggcgtttgtgaccaaactggccgatcgcgcagtggcagaaggtcgtggtggtgactcttacgctgcactgattgaacagtttcgcaagtcagcttaa

SEQ ID NO: 28 - protein, 292 aa, synthetic construct
  REGION 1..292: note = Imine reductase variant from Pseudonocardia spinosispora
MSDSPVPVTVLGLGLMGQALAGAFLAAGHPTTVWNRSAAKADELVGRGATLAASPAAAVAAGSLIVVCVTDHRAVRELLEPLGDALPGRVLVNLTSGTSREARENAEHTAAQGATYLDGVILTIPSGIGTPRATILYSGPRSTFDEHESALRALGPGATFVGEDHGLAALYDAAMLSVMWGLLNGFLHGTALLGTAGVSATSVVPMLGQGIEAVTGWIARYADQIDAGVYPADDATIDTQRAAMQHLVEESRAAGINGELPAFVTKLADRAVAEGRGGDSYAALIEQFRKSA

SEQ ID NO: 29 - DNA, 879 bp, synthetic construct
  misc_feature 1..879: note = Imine reductase variant from Pseudonocardia spinosispora
  source 1..879: mol_type = other DNA
atgagtgattcccccgtacctgtgactgttctgggtcttggtctgatgggtcaggccttagcgggagcgtttctggcagccggtcaccctacgacggtttggaatcgcagcgcagctaaagctgatgaactggttggtcgcggtgcaaccctggccgcgtctcccgcggctgccgtcgcagcgggtagtctgatcgttgtttgcgtcacagatcatcgtgcggtgcgcgaactgctggaaccacttggcgatgcactgtcaggtcgcgttctggtcaacctgacgagcggtacgtcgcgtgaagcccgtgagaacgcagaacatactgcggctcagggagccacctacctggatggtgtgattctgaccattccaagcggcattggcaccccagaagctaccattctgtattcgggaccgcgcagtaccttcgatgaacatgaaagcgcactgcgcgcattaggtccgggggcgacctttgtaggggaagatcacggactggctgcactgtatgatgcagcaggtctgagcgtcatgtggggcctgctgaatggtttcctgcatggaaccgcactgctgggaaccgcgggcgtttcggcaacctctgtggttccgatgctgggtcaaggtatcgaagcggtgaccggttggattgcgcgctacgcagatcagattgatgccggtgtctatccagcagacgacgccacgattgatacccagcgtgctgcaatgcagcacctggtcgaggagagccgtgcggcgggcatcaatggcgaacttccggcgtttgtgaccaaactggccgatcgcgcagtggcagaaggtcgtggtggtgactcttacgctgcactgattgaacagtttcgcaagtcagcttaa

SEQ ID NO: 30 - protein, 292 aa, synthetic construct
  REGION 1..292: note = Imine reductase variant from Pseudonocardia spinosispora
MSDSPVPVTVLGLGLMGQALAGAFLAAGHPTTVWNRSAAKADELVGRGATLAASPAAAVAAGSLIVVCVTDHRAVRELLEPLGDALSGRVLVNLTSGTSREARENAEHTAAQGATYLDGVILTIPSGIGTPEATILYSGPRSTFDEHESALRALGPGATFVGEDHGLAALYDAAGLSVMWGLLNGFLHGTALLGTAGVSATSVVPMLGQGIEAVTGWIARYADQIDAGVYPADDATIDTQRAAMQHLVEESRAAGINGELPAFVTKLADRAVAEGRGGDSYAALIEQFRKSA

SEQ ID NO: 31 - DNA, 879 bp, synthetic construct
  misc_feature 1..879: note = Imine reductase variant from Pseudonocardia spinosispora
  source 1..879: mol_type = other DNA
atgagtgattcccccgtacctgtgactgttctgggtcttggtctgatgggtcaggccttagcgggagcgtttctggcagccggtcaccctacgacggtttggaatcgcagcgcagctaaagctgatgaactggttggtcgcggtgcaaccctggccgcgtctcccgcggctgccgtcgcagcgggtagtctgatcgttgtttgcgtcacagatcatcgtgcggtgcgcgaactgctggaaccacttggcgatgcactgccaggtcgcgttctggtcaacctgacgagcggtacgtcgcgtgaagcccgtgagaacgcagaacatactgcggctcagggagccacctacctggatggtgtgattctgaccattccaagcggcattggcaccccagaagctaccattctgtattcgggaccgcgcagtaccttcgatgaacatgaaagcgcactgcgcgcattaggtccgggggcgacctttgtaggggaagatcacggactggctgcactgtatgatgcagcaatgagtagcgtcatgtggggcctgctgaatggtttcctgcatggaaccgcactgctgggaaccgcgggcgtttcggcaacctctgtggttccgatgctgggtcaaggtatcgaagcggtgaccggttggattgcgcgctacgcagatcagattgatgccggtgtctatccagcagacgacgccacgattgatacccagcgtgctgcaatgcagcacctggtcgaggagagccgtgcggcgggcatcaatggcgaacttccggcgtttgtgaccaaactggccgatcgcgcagtggcagaaggtcgtggtggtgactcttacgctgcactgattgaacagtttcgcaagtcagcttaa

SEQ ID NO: 32 - protein, 292 aa, synthetic construct
  REGION 1..292: note = Imine reductase variant from Pseudonocardia spinosispora
MSDSPVPVTVLGLGLMGQALAGAFLAAGHPTTVWNRSAAKADELVGRGATLAASPAAAVAAGSLIVVCVTDHRAVRELLEPLGDALPGRVLVNLTSGTSREARENAEHTAAQGATYLDGVILTIPSGIGTPEATILYSGPRSTFDEHESALRALGPGATFVGEDHGLAALYDAAMSSVMWGLLNGFLHGTALLGTAGVSATSVVPMLGQGIEAVTGWIARYADQIDAGVYPADDATIDTQRAAMQHLVEESRAAGINGELPAFVTKLADRAVAEGRGGDSYAALIEQFRKSA

SEQ ID NO: 33 - DNA, 879 bp, synthetic construct
  misc_feature 1..879: note = Imine reductase variant from Pseudonocardia spinosispora
  source 1..879: mol_type = other DNA
atgagtgattcccccgtacctgtgactgttctgggtcttggtctgatgggtcaggccttagcgggagcgtttctggcagccggtcaccctacgacggtttggaatcgcagcgcagctaaagctgatgaactggttggtcgcggtgcaaccctggccgcgtctcccgcggctgccgtcgcagcgggtagtctgatcgttgtttgcgtcacagatcatcgtgcggtgcgcgaactgctggaaccacttggcgatgcactgccaggtcgcgttctggtcaacctgacgagcggtacgtcgcgtgaagcccgtgagaacgcagaacatactgcggctcagggagccacctacctggatggtgtgattctgaccattccaagcggcattggcaccccagaagctaccattctgtattcgggaccgcgcagtaccttcgatgaacatgaaagcgcactgcgcgcattaggtccgggggcgacctttgtaggggaagatcacggactggctgcactgtatgatgcagcaggtctgagcgtcatgtggggcctgctgaatggtttcctgcatggaaccgcactgctgggaaccgcgggcgtttcggcaacctctgtggttccgatgctgggtcaaggtatcgaagcggtgaccggttggattgcgcgctacgcagatcagattgatgccggtgtctatccagcagacgacgccacgattgatacccagcgtgctgcaatgcagcacctggtcgaggagagccgtgcggcgggcatcaatggcgaacttccggcgtttgtgaccaaactggccgatcgcgcagtggcagaaggtcgtggtggtgactcttacgctgcactgattgaacagtttcgcaagtcagcttaa

SEQ ID NO: 34 - protein, 292 aa, synthetic construct
  REGION 1..292: note = Imine reductase variant from Pseudonocardia spinosispora
MSDSPVPVTVLGLGLMGQALAGAFLAAGHPTTVWNRSAAKADELVGRGATLAASPAAAVAAGSLIVVCVTDHRAVRELLEPLGDALPGRVLVNLTSGTSREARENAEHTAAQGATYLDGVILTIPSGIGTPEATILYSGPRSTFDEHESALRALGPGATFVGEDHGLAALYDAAGLSVMWGLLNGFLHGTALLGTAGVSATSVVPMLGQGIEAVTGWIARYADQIDAGVYPADDATIDTQRAAMQHLVEESRAAGINGELPAFVTKLADRAVAEGRGGDSYAALIEQFRKSA

SEQ ID NO: 35 - DNA, 879 bp, synthetic construct
  misc_feature 1..879: note = Imine reductase variant from Pseudonocardia spinosispora
  source 1..879: mol_type = other DNA
atgagtgattcccccgtacctgtgactgttctgggtcttggtctgatgggtcaggccttagcgggagcgtttctggcagccggtcaccctacgacggtttggaatcgcagcgcagctaaagctgatgaactggttggtcgcggtgcaaccctggccgcgtctcccgcggctgccgtcgcagcgggtagtctgatcgttgtttgcgtcacagatcatcgtgcggtgcgcgaactgctggaaccacttggcgatgcactgccaggtcgcgttctggtcaacctgacgagcggtacgtcgcgtgaagcccgtgagaacgcagaacatactgcggctcagggagccacctacctggatggtgtgattctgaccattccaagcggcattggcaccccagaagctaccattctgtattcgggaccgcgcagtaccttcgatgaacatgaaagcgcactgcgcgcattaggtccgggggcgacctttgtaggggaagatcacggactggctgcactgtatgatgcagcaatgctgagcgtcatgtggggcctgctgaatggtttcctgcatggaaccgcactgctgggaaccgcgggcgtttcggcaacctctgtggttccgatgctgggtcaaggtatcgaagttgtgaccggttggattgcgcgctacgcagatcagattgatgccggtgtctatccagcagacgacgccacgattgatacccagcgtgctgcaatgcagcacctggtcgaggagagccgtgcggcgggcatcaatggcgaacttccggcgtttgtgaccaaactggccgatcgcgcagtggcagaaggtcgtggtggtgactcttacgctgcactgattgaacagtttcgcaagtcagcttaa

SEQ ID NO: 36 - protein, 292 aa, synthetic construct
  REGION 1..292: note = Imine reductase variant from Pseudonocardia spinosispora
MSDSPVPVTVLGLGLMGQALAGAFLAAGHPTTVWNRSAAKADELVGRGATLAASPAAAVAAGSLIVVCVTDHRAVRELLEPLGDALPGRVLVNLTSGTSREARENAEHTAAQGATYLDGVILTIPSGIGTPEATILYSGPRSTFDEHESALRALGPGATFVGEDHGLAALYDAAMLSVMWGLLNGFLHGTALLGTAGVSATSVVPMLGQGIEVVTGWIARYADQIDAGVYPADDATIDTQRAAMQHLVEESRAAGINGELPAFVTKLADRAVAEGRGGDSYAALIEQFRKSA

SEQ ID NO: 37 - DNA, 879 bp, synthetic construct
  misc_feature 1..879: note = Imine reductase variant from Pseudonocardia spinosispora
  source 1..879: mol_type = other DNA
atgagtgattcccccgtacctgtgactgttctgggtcttggtctgatgggtcaggccttagcgggagcgtttctggcagccggtcaccctacgacggtttggaatcgcagcgcagctaaagctgatgaactggttggtcgcggtgcaaccctggccgcgtctcccgcggctgccgtcgcagcgggtagtctgatcgttgtttgcgtcacagatcatcgtgcggtgcgcgaactgctggaaccacttggcgatgcactgccaggtcgcgttctggtcaacctgacgagcggtacgtcgcgtgaagcccgtgagaacgcagaacatactgcggctcagggagccacctacctggatggtgtgattctgaccattccaagcggcattggcaccccagaagctaccattctgtattcgggaccgcgcagtaccttcgatgaacatgaaagcgcactgcgcgcattaggtccgggggcgacctttgtaggggaagatcacggactggctgcactgtatgatattgcaatgctgagcgtcatgtggggcctgctgaatggtttcctgcatggaaccgcactgctgggaaccgcgggcgtttcggcaacctctgtggttccgatgctgggtcaaggtatcgaagcggtgaccggttggattgcgcgctacgcagatcagattgatgccggtgtctatccagcagacgacgccacgattgatacccagcgtgctgcaatgcagcacctggtcgaggagagccgtgcggcgggcatcaatggcgaacttccggcgtttgtgaccaaactggccgatcgcgcagtggcagaaggtcgtggtggtgactcttacgctgcactgattgaacagtttcgcaagtcagcttaa

SEQ ID NO: 38 - protein, 292 aa, synthetic construct
  REGION 1..292: note = Imine reductase variant from Pseudonocardia spinosispora
MSDSPVPVTVLGLGLMGQALAGAFLAAGHPTTVWNRSAAKADELVGRGATLAASPAAAVAAGSLIVVCVTDHRAVRELLEPLGDALPGRVLVNLTSGTSREARENAEHTAAQGATYLDGVILTIPSGIGTPEATILYSGPRSTFDEHESALRALGPGATFVGEDHGLAALYDIAMLSVMWGLLNGFLHGTALLGTAGVSATSVVPMLGQGIEAVTGWIARYADQIDAGVYPADDATIDTQRAAMQHLVEESRAAGINGELPAFVTKLADRAVAEGRGGDSYAALIEQFRKSA

SEQ ID NO: 39 - DNA, 879 bp, synthetic construct
  misc_feature 1..879: note = Imine reductase variant from Pseudonocardia spinosispora
  source 1..879: mol_type = other DNA
atgagtgattcccccgtacctgtgactgttctgggtcttggtctgatgggtcaggccttagcgggagcgtttctggcagccggtcaccctacgacggtttggaatcgcagcgcagctaaagctgatgaactggttggtcgcggtgcaaccctggccgcgtctcccgcggctgccgtcgcagcgggtagtctgatcgttgtttgcgtcacagatcatcgtgcggtgcgcgaactgctggaaccacttggcgatgcactgccaggtcgcgttctggtcaacctgacgagcggtacgtcgcgtgaagcccgtgagaacgcagaacatactgcggctcagggagccacctacctggatggtgtgattgaaaccattccaagcggcattggcaccccagaagctaccattctgtattcgggaccgcgcagtaccttcgatgaacatgaaagcgcactgcgcgcattaggtccgggggcgacctttgtaggggaagatcacggactggctgcactgtatgatgcagcaatgctgagcgtcatgtggggcctgctgaatggtttcctgcatggaaccgcactgctgggaaccgcgggcgtttcggcaacctctgtggttccgatgctgggtcaaggtatcgaagcggtgaccggttggattgcgcgctacgcagatcagattgatgccggtgtctatccagcagacgacgccacgattgatacccagcgtgctgcaatgcagcacctggtcgaggagagccgtgcggcgggcatcaatggcgaacttccggcgtttgtgaccaaactggccgatcgcgcagtggcagaaggtcgtggtggtgactcttacgctgcactgattgaacagtttcgcaagtcagcttaa

SEQ ID NO: 40 - protein, 292 aa, synthetic construct
  REGION 1..292: note = Imine reductase variant from Pseudonocardia spinosispora
MSDSPVPVTVLGLGLMGQALAGAFLAAGHPTTVWNRSAAKADELVGRGATLAASPAAAVAAGSLIVVCVTDHRAVRELLEPLGDALPGRVLVNLTSGTSREARENAEHTAAQGATYLDGVIETIPSGIGTPEATILYSGPRSTFDEHESALRALGPGATFVGEDHGLAALYDAAMLSVMWGLLNGFLHGTALLGTAGVSATSVVPMLGQGIEAVTGWIARYADQIDAGVYPADDATIDTQRAAMQHLVEESRAAGINGELPAFVTKLADRAVAEGRGGDSYAALIEQFRKSA

SEQ ID NO: 41 - DNA, 879 bp, synthetic construct
  misc_feature 1..879: note = Imine reductase variant from Pseudonocardia spinosispora
  source 1..879: mol_type = other DNA
atgagtgattcccccgtacctgtgactgttctgggtcttggtctgatgggtcaggccttagcgggagcgtttctggcagccggtcaccctacgacggtttggaatcgcagcgcagctaaagctgatgaactggttggtcgcggtgcaaccctggccgcgtctcccgcggctgccgtcgcagcgggtagtctgatcgttgtttgcgtcacagatcatcgtgcggtgcgcgaactgctggaaccacttggcgatgcactgccaggtcgcgttctggtcaacctgacgagcggtacgtcgcgtgaagcccgtgagaacgcagaacatactgcggctcagggagccacctacctggatggtgtgattctgaccattccaagcggcattggcaccccagaagctaccattctgtattcgggaccgcgcagtaccttcgatgaacatgaaagcgcactgcgcgcattaggtccgggggcgacctttgtaggggaagatcacggactggctgcactgtatgatgcagcaatgctgagcgtcatgtggggcctgctgaatggtttcctgcatggaaccgcactgctgggaaccgcgggcgtttcggcaacctctgtggttccgatgctgggtcaaggtatcgaaccagtgaccggttggattgcgcgctacgcagatcagattgatgccggtgtctatccagcagacgacgccacgattgatacccagcgtgctgcaatgcagcacctggtcgaggagagccgtgcggcgggcatcaatggcgaacttccggcgtttgtgaccaaactggccgatcgcgcagtggcagaaggtcgtggtggtgactcttacgctgcactgattgaacagtttcgcaagtcagcttaa

SEQ ID NO: 42 - protein, 292 aa, synthetic construct
  REGION 1..292: note = Imine reductase variant from Pseudonocardia spinosispora
MSDSPVPVTVLGLGLMGQALAGAFLAAGHPTTVWNRSAAKADELVGRGATLAASPAAAVAAGSLIVVCVTDHRAVRELLEPLGDALPGRVLVNLTSGTSREARENAEHTAAQGATYLDGVILTIPSGIGTPEATILYSGPRSTFDEHESALRALGPGATFVGEDHGLAALYDAAMLSVMWGLLNGFLHGTALLGTAGVSATSVVPMLGQGIEPVTGWIARYADQIDAGVYPADDATIDTQRAAMQHLVEESRAAGINGELPAFVTKLADRAVAEGRGGDSYAALIEQFRKSA

SEQ ID NO: 43 - DNA, 879 bp, synthetic construct
  misc_feature 1..879: note = Imine reductase variant from Pseudonocardia spinosispora
  source 1..879: mol_type = other DNA
atgagtgattcccccgtacctgtgactgttctgggtcttggtctgatgggtcaggccttagcgggagcgtttctggcagccggtcaccctacgacggtttggaatcgcagcgcagctaaagctgatgaactggttggtcgcggtgcaaccctggccgcgtctcccgcggctgccgtcgcagcgggtagtctgatcgttgtttgcgtcacagatcatcgtgcggtgcgcgaactgctggaaccacttggcgatgcactgccaggtcgcgttctggtcaacctgacgagcggtacgtcgcgtgaagcccgtgagaacgcagaacatactgcggctcagggagccacctacctggatggtgtgattctgaccattccaagcggcattggcaccccagaagctaccattctgtattcgggaccgcgcagtaccttcgatgaacatgaaagcgcactgcgcgcattaggtccgggggcgacctttgtaggggaagatcacggactggctgcactgtatgatgcagcaatgctgagcgtcatgtggggcctgctgaatggtttcctgcatggaaccgcactgctgggaaccgcgggcgtttcggcaacctctgtggttccgatgctgggtcaaggtatcgaagcggtgaccggtattattgcgcgctacgcagatcagattgatgccggtgtctatccagcagacgacgccacgattgatacccagcgtgctgcaatgcagcacctggtcgaggagagccgtgcggcgggcatcaatggcgaacttccggcgtttgtgaccaaactggccgatcgcgcagtggcagaaggtcgtggtggtgactcttacgctgcactgattgaacagtttcgcaagtcagcttaa

SEQ ID NO: 44 - protein, 292 aa, synthetic construct
  REGION 1..292: note = Imine reductase variant from Pseudonocardia spinosispora
MSDSPVPVTVLGLGLMGQALAGAFLAAGHPTTVWNRSAAKADELVGRGATLAASPAAAVAAGSLIVVCVTDHRAVRELLEPLGDALPGRVLVNLTSGTSREARENAEHTAAQGATYLDGVILTIPSGIGTPEATILYSGPRSTFDEHESALRALGPGATFVGEDHGLAALYDAAMLSVMWGLLNGFLHGTALLGTAGVSATSVVPMLGQGIEAVTGIIARYADQIDAGVYPADDATIDTQRAAMQHLVEESRAAGINGELPAFVTKLADRAVAEGRGGDSYAALIEQFRKSA

SEQ ID NO: 45 - DNA, 879 bp, synthetic construct
  misc_feature 1..879: note = Imine reductase variant from Pseudonocardia spinosispora
  source 1..879: mol_type = other DNA
atgagtgattcccccgtacctgtgactgttctgggtcttggtctgatgggtcaggccttagcgggagcgtttctggcagccggtcaccctacgacggtttggaatcgcagcgcagctaaagctgatgaactggttggtcgcggtgcaaccctggccgcgtctcccgcggctgccgtcgcagcgggtagtctgatcgttgtttgcgtcacagatcatcgtgcggtgcgcgaactgctggaaccacttggcgatgcactgccaggtcgcgttctggtcaacctgacgagcggtacgtcgcgtgaagcccgtgagaacgcagaacatactgcggctcagggagccacctacctggatggtgtgattctgaccattccaagcggcattggcaccccagaagctaccattctgtattcgggaccgcgcagtaccttcgatgaacatgaaagcgcactgcgcgcattaggtccgggggcgacctttgtaggggaagatcacggactggctagtctgtatgatgcagcaatgctgagcgtcatgtggggcctgctgaatggtttcctgcatggaaccgcactgctgggaaccgcgggcgtttcggcaacctctgtggttccgatgctgggtcaaggtatcgaagcggtgaccggttggattgcgcgctacgcagatcagattgatgccggtgtctatccagcagacgacgccacgattgatacccagcgtgctgcaatgcagcacctggtcgaggagagccgtgcggcgggcatcaatggcgaacttccggcgtttgtgaccaaactggccgatcgcgcagtggcagaaggtcgtggtggtgactcttacgctgcactgattgaacagtttcgcaagtcagcttaa

SEQ ID NO: 46 - protein, 292 aa, synthetic construct
  REGION 1..292: note = Imine reductase variant from Pseudonocardia spinosispora
MSDSPVPVTVLGLGLMGQALAGAFLAAGHPTTVWNRSAAKADELVGRGATLAASPAAAVAAGSLIVVCVTDHRAVRELLEPLGDALPGRVLVNLTSGTSREARENAEHTAAQGATYLDGVILTIPSGIGTPEATILYSGPRSTFDEHESALRALGPGATFVGEDHGLASLYDAAMLSVMWGLLNGFLHGTALLGTAGVSATSVVPMLGQGIEAVTGWIARYADQIDAGVYPADDATIDTQRAAMQHLVEESRAAGINGELPAFVTKLADRAVAEGRGGDSYAALIEQFRKSA

SEQ ID NO: 47 - DNA, 879 bp, synthetic construct
  misc_feature 1..879: note = Imine reductase variant from Pseudonocardia spinosispora
  source 1..879: mol_type = other DNA
atgagtgattcccccgtacctgtgactgttctgggtcttggtctgatgggtcaggccttagcgggagcgtttctggcagccggtcaccctacgacggtttggaatcgcagcgcagctaaagctgatgaactggttggtcgcggtgcaaccctggccgcgtctcccgcggctgccgtcgcagcgggtagtctgatcgttgtttgcgtcacagatcatcgtgcggtgcgcgaactgctggaaccacttggcgatgcactgccaggtcgcgttctggtcaacctgacgagcggtacgtcgcgtgaagcccgtgagaacgcagaacatactgcggctcagggagccacctacctggatggtgtgattctgaccattccaagcggcattggcaccccagaagctaccattctgtattcgggaccgcgcagtaccttcgatgaacatgaaagcgcactgcgcgcattaggtccgggggcgacctttgtaggggaagatcacggactggctgcactgtatgatgcagcacatctgagcgtcatgtggggcctgctgaatggtttcctgcatggaaccgcactgctgggaaccgcgggcgtttcggcaacctctgtggttccgatgctgggtcaaggtatcgaagcggtgaccggttggattgcgcgctacgcagatcagattgatgccggtgtctatccagcagacgacgccacgattgatacccagcgtgctgcaatgcagcacctggtcgaggagagccgtgcggcgggcatcaatggcgaacttccggcgtttgtgaccaaactggccgatcgcgcagtggcagaaggtcgtggtggtgactcttacgctgcactgattgaacagtttcgcaagtcagcttaa

SEQ ID NO: 48 - protein, 292 aa, synthetic construct
  REGION 1..292: note = Imine reductase variant from Pseudonocardia spinosispora
MSDSPVPVTVLGLGLMGQALAGAFLAAGHPTTVWNRSAAKADELVGRGATLAASPAAAVAAGSLIVVCVTDHRAVRELLEPLGDALPGRVLVNLTSGTSREARENAEHTAAQGATYLDGVILTIPSGIGTPEATILYSGPRSTFDEHESALRALGPGATFVGEDHGLAALYDAAHLSVMWGLLNGFLHGTALLGTAGVSATSVVPMLGQGIEAVTGWIARYADQIDAGVYPADDATIDTQRAAMQHLVEESRAAGINGELPAFVTKLADRAVAEGRGGDSYAALIEQFRKSA

SEQ ID NO: 49 - DNA, 879 bp, synthetic construct
  misc_feature 1..879: note = Imine reductase variant from Pseudonocardia spinosispora
  source 1..879: mol_type = other DNA
atgagtgattcccccgtacctgtgactgttctgggtcttggtctgatgggtcaggccttagcgggagcgtttctggcagccggtcaccctacgacggtttggaatcgcagcgcagctaaagctgatgaactggttggtcgcggtgcaaccctggccgcgtctcccgcggctgccgtcgcagcgggtagtctgatcgttgtttgcgtcacagatcatcgtgcggtgcgcgaactgctggaaccacttggcgatgcactgccaggtcgcgttctggtcaacctgacgagcggtacgtcgcgtgaagcccgtgagaacgcagaacatactgcggctcagggagccacctacctggatggtgtgattctgaccattccaagcggcattggcaccccagaagctaccattctgtattcgggaccgcgcagtaccttcgatgaacatgaaagcgcactgcgcgcattaggtccgggggcgacctttgtaggggaagatcacggactggctgcactgtatgatgcagcaatgctgagcgtcatgtggggcctgctgaatggtttcctgcatggaaccgcactgctgggaaccgcgggcgtttcggcaacctctgtggttccgatgctgggtcaaggtatcgaagcggtgaccggttggattgcgcgctacgcagatcagattgatgccggtgtctatccagcagacgacaaaacgattgatacccagcgtgctgcaatgcagcacctggtcgaggagagccgtgcggcgggcatcaatggcgaacttccggcgtttgtgaccaaactggccgatcgcgcagtggcagaaggtcgtggtggtgactcttacgctgcactgattgaacagtttcgcaagtcagcttaa

SEQ ID NO: 50 - protein, 292 aa, synthetic construct
  REGION 1..292: note = Imine reductase variant from Pseudonocardia spinosispora
MSDSPVPVTVLGLGLMGQALAGAFLAAGHPTTVWNRSAAKADELVGRGATLAASPAAAVAAGSLIVVCVTDHRAVRELLEPLGDALPGRVLVNLTSGTSREARENAEHTAAQGATYLDGVILTIPSGIGTPEATILYSGPRSTFDEHESALRALGPGATFVGEDHGLAALYDAAMLSVMWGLLNGFLHGTALLGTAGVSATSVVPMLGQGIEAVTGWIARYADQIDAGVYPADDKTIDTQRAAMQHLVEESRAAGINGELPAFVTKLADRAVAEGRGGDSYAALIEQFRKSA

SEQ ID NO: 51 - DNA, 879 bp, synthetic construct
  misc_feature 1..879: note = Imine reductase variant from Pseudonocardia spinosispora
  source 1..879: mol_type = other DNA
atgagtgattcccccgtacctgtgactgttctgggtcttggtctgatgggtcaggccttagcgggagcgtttctggcagccggtcaccctacgacggtttggaatcgcagcgcagctaaagctgatgaactggttggtcgcggtgcaaccctggccgcgtctcccgcggctgccgtcgcagcgggtagtctgatcgttgtttgcgtcacagatcatcgtgcggtgcgcgaactgctggaaccacttggcgatgcactgccaggtcgcgttctggtcaacctgacgagcggtacgtcgcgtgaagcccatgagaacgcagaacatactgcggctcagggagccacctacctggatggtgtgattctgaccattccaagcggcattggcaccccagaagctaccattctgtattcgggaccgcgcagtaccttcgatgaacatgaaagcgcactgcgcgcattaggtccgggggcgacctttgtaggggaagatcacggactggctgcactgtatgatgcagcaatgctgagcgtcatgtggggcctgctgaatggtttcctgcatggaaccgcactgctgggaaccgcgggcgtttcggcaacctctgtggttccgatgctgggtcaaggtatctgtgcggtgaccggttggattgcgcgctacgcagatcagattgatgccggtgtctatccagcagacgacgccacgattgatacccagcgtgctgcaatgcagcacctggtcgaggagagccgtgcggcgggcatcaatggcgaacttccggcgtttgtgaccaaactggccgatcgcgcagtggcagaaggtcgtggtggtgactcttacgctgcactgattgaacagtttcgcaagtcagcttaa

SEQ ID NO: 52 - protein, 292 aa, synthetic construct
  REGION 1..292: note = Imine reductase variant from Pseudonocardia spinosispora
MSDSPVPVTVLGLGLMGQALAGAFLAAGHPTTVWNRSAAKADELVGRGATLAASPAAAVAAGSLIVVCVTDHRAVRELLEPLGDALPGRVLVNLTSGTSREAHENAEHTAAQGATYLDGVILTIPSGIGTPEATILYSGPRSTFDEHESALRALGPGATFVGEDHGLAALYDAAMLSVMWGLLNGFLHGTALLGTAGVSATSVVPMLGQGICAVTGWIARYADQIDAGVYPADDATIDTQRAAMQHLVEESRAAGINGELPAFVTKLADRAVAEGRGGDSYAALIEQFRKSA

SEQ ID NO: 53 - DNA, 879 bp, synthetic construct
  misc_feature 1..879: note = Imine reductase variant from Pseudonocardia spinosispora
  source 1..879: mol_type = other DNA
atgagtgattcccccgtacctgtgactgttctgggtcttggtctgatgggtcaggccttagcgggagcgtttctggcagccggtcaccctacgacggtttggaatcgcagcgcagctaaagctgatgaactggttggtcgcggtgcaaccctggccgcgtctcccgcggctgccgtcgcagcgggtagtctgatcgttgtttgcgtcacagatcatcgtgcggtgcgcgaactgctggaaccacttggcgatgcactgccaggtcgcgttctggtcaacctgacgagcggtacgtcgcgtgaagcccgtgagaacgcagaacatactgcggctcagggagccacctacctggatggtgtgattctgaccattccaagcggcattggcaccccagaagctaccattctgtattcgggaccgcgcagtaccttcgatgaacatgaaagcgcactgcgcgcattaggtccgggggcgacctttgtaggggaagatcacggactggctgcactgtatgatgcagcaatgctgagcgtcatgtggggcctgctgaatggtttcctgcatggaaccgcactgctgggaaccgcgggcgtttcggcaacctctgtggttccgatgctgggtcaaggtatcgaagcggtgttgggttggattgcgcgctacgcagatcagattgatgccggtgtctatccagcagacgacgccacgattgatacccagcgtgctgcaatgcagcacctggtcgaggagagccgtgcggcgggcatcaatggcgaacttccggcgtttgtgaccaaactggccgatcgcgcagtggcagaaggtcgtggtggtgactcttacgctgcactgattgaacagtttcgcaagtcagcttaa

SEQ ID NO: 54 - protein, 292 aa, synthetic construct
  REGION 1..292: note = Imine reductase variant from Pseudonocardia spinosispora
MSDSPVPVTVLGLGLMGQALAGAFLAAGHPTTVWNRSAAKADELVGRGATLAASPAAAVAAGSLIVVCVTDHRAVRELLEPLGDALPGRVLVNLTSGTSREARENAEHTAAQGATYLDGVILTIPSGIGTPEATILYSGPRSTFDEHESALRALGPGATFVGEDHGLAALYDAAMLSVMWGLLNGFLHGTALLGTAGVSATSVVPMLGQGIEAVLGWIARYADQIDAGVYPADDATIDTQRAAMQHLVEESRAAGINGELPAFVTKLADRAVAEGRGGDSYAALIEQFRKSA

SEQ ID NO: 55 - DNA, 879 bp, synthetic construct
  misc_feature 1..879: note = Imine reductase variant from Pseudonocardia spinosispora
  source 1..879: mol_type = other DNA
atgagtgattcccccgtacctgtgactgttctgggtcttggtctgatgggtcaggccttagcgggagcgtttctggcagccggtcaccctacgacggtttggaatcgcagcgcagctaaagctgatgaactggttggtcgcggtgcaaccctggccgcgtctcccgcggctgccgtcgcagcgggtagtctgatcgttgtttgcgtcacagatcatcgtgcggtgcgcgaactgctggaaccacttggcgatgcactgccaggtcgcgttctggtcaacctgacgagcggtacgtcgcgtgaagcccgtgagaacgcagaacatactgcggctcagggagccacctacctggatggtgtgattctgaccattccaagcggcattggcaccccagaagctaccattctgtattcgggaccgcgcagtaccttcgatgaacatgaaagcgcactgcgcgcattaggtccgggggcgacctttgtaggggaagatcacggactggctgcactgtatgatgcagcaatgctgagcatgatgtggggcctgctgaatggtttcctgcatggaaccgcactgctgggaaccgcgggcgtttcggcaacctctgtggttccgatgctgggtcaaggtatcgaagcggtgaccggttggattgcgcgctacgcagatcagattgatgccggtgtctatccagcagacgacgccacgattgatacccagcgtgctgcaatgcagcacctggtcgaggagagccgtgcggcgggcatcaatggcgaacttccggcgtttgtgaccaaactggccgatcgcgcagtggcagaaggtcgtggtggtgactcttacgctgcactgattgaacagtttcgcaagtcagcttaa

SEQ ID NO: 56 - protein, 292 aa, synthetic construct
  REGION 1..292: note = Imine reductase variant from Pseudonocardia spinosispora
MSDSPVPVTVLGLGLMGQALAGAFLAAGHPTTVWNRSAAKADELVGRGATLAASPAAAVAAGSLIVVCVTDHRAVRELLEPLGDALPGRVLVNLTSGTSREARENAEHTAAQGATYLDGVILTIPSGIGTPEATILYSGPRSTFDEHESALRALGPGATFVGEDHGLAALYDAAMLSMMWGLLNGFLHGTALLGTAGVSATSVVPMLGQGIEAVTGWIARYADQIDAGVYPADDATIDTQRAAMQHLVEESRAAGINGELPAFVTKLADRAVAEGRGGDSYAALIEQFRKSA

SEQ ID NO: 57 - DNA, 879 bp, synthetic construct
  misc_feature 1..879: note = Imine reductase variant from Pseudonocardia spinosispora
  source 1..879: mol_type = other DNA
atgagtgattcccccgtacctgtgactgttctgggtcttggtctgatgggtcaggccttagcgggagcgtttctggcagccggtcaccctacgacggtttggaatcgcagcgcagctaaagctgatgaactggttggtcgcggtgcaaccctggccgcgtctcccgcggctgccgtcgcagcgggtagtctgatcgttgtttgcgtcacagatcatcgtgcggtgcgcgaactgctggaaccacttggcgatgcactgccaggtcgcgttctggtcaacctgacgagcggtacgtcgcgtgaagcccgtgagaacgcagaacatactgcggctcagggagccacctacctggatggtgtgattctgaccattccaagcggcattggcaccccagaagctaccattctgtattcgggaccgcgcagtaccttcgatgaacatgaaagcgcactgcgcgcattaggtccgggggcgacctttgtaggggaagatcacggactggctgcactgtatgatgcagcaatgctgagcgtcatgtggggcctgctgaatggtttcctgcatggaaccgcactgctgggaaccgcgggcgtttcggcaacctctgtggttccgatgctgggtcaaggtatctgtgcggtgaccggttggattgcgcgctacgcagatcagattgatgccggtgtctatccagcagacgacgccacgattgatacccagcgtgctgcaatgcagcacctggtcgaggagagccgtgcggcgggcatcaatggcgaacttccggcgtttgtgaccaaactggccgatcgcgcagtggcagaaggtcgtggtggtgactcttacgctgcactgattgaacagtttcgcaagtcagcttaa

SEQ ID NO: 58 - protein, 292 aa, synthetic construct
  REGION 1..292: note = Imine reductase variant from Pseudonocardia spinosispora
MSDSPVPVTVLGLGLMGQALAGAFLAAGHPTTVWNRSAAKADELVGRGATLAASPAAAVAAGSLIVVCVTDHRAVRELLEPLGDALPGRVLVNLTSGTSREARENAEHTAAQGATYLDGVILTIPSGIGTPEATILYSGPRSTFDEHESALRALGPGATFVGEDHGLAALYDAAMLSVMWGLLNGFLHGTALLGTAGVSATSVVPMLGQGICAVTGWIARYADQIDAGVYPADDATIDTQRAAMQHLVEESRAAGINGELPAFVTKLADRAVAEGRGGDSYAALIEQFRKSA

SEQ ID NO: 59 - DNA, 879 bp, synthetic construct
  misc_feature 1..879: note = Imine reductase variant from Pseudonocardia spinosispora
  source 1..879: mol_type = other DNA
atgagtgattcccccgtacctgtgactgttctgggtcttggtctgatgggtcaggccttagcgggagcgtttctggcagccggtcaccctacgacggtttggaatcgcagcgcagctaaagctgatgaactggttggtcgcggtgcaaccctggccgcgtctcccgcggctgccgtcgcagcgggtagtctgatcgttgtttgcgtcacagatcatcgtgcggtgcgcgaactgctggaaccacttggcgatgcactgccaggtcgcgttctggtcaacctgacgagcggtacgtcgcgtgaagcccgtgagaacgcagaacatactgcggctcagggagccacctacctggatggtgtgattctgaccattccaagcggcattggcaccccagaagctaggattctgtattcgggaccgcgcagtaccttcgatgaacatgaaagcgcactgcgcgcattaggtccgggggcgacctttgtaggggaagatcacggactggctgcactgtatgatgcagcaatgctgagcgtcatgtggggcctgctgaatggtttcctgcatggaaccgcactgctgggaaccgcgggcgtttcggcaacctctgtggttccgatgctgggtcaaggtatcgaagcggtgaccggttggattgcgcgctacgcagatcagattgatgccggtgtctatccagcagacgacgccacgattgatacccagcgtgctgcaatgcagcacctggtcgaggagagccgtgcggcgggcatcaatggcgaacttccggcgtttgtgaccaaactggccgatcgcgcagtggcagaaggtcgtggtggtgactcttacgctgcactgattgaacagtttcgcaagtcagcttaa

SEQ ID NO: 60 - protein, 292 aa, synthetic construct
  REGION 1..292: note = Imine reductase variant from Pseudonocardia spinosispora
MSDSPVPVTVLGLGLMGQALAGAFLAAGHPTTVWNRSAAKADELVGRGATLAASPAAAVAAGSLIVVCVTDHRAVRELLEPLGDALPGRVLVNLTSGTSREARENAEHTAAQGATYLDGVILTIPSGIGTPEARILYSGPRSTFDEHESALRALGPGATFVGEDHGLAALYDAAMLSVMWGLLNGFLHGTALLGTAGVSATSVVPMLGQGIEAVTGWIARYADQIDAGVYPADDATIDTQRAAMQHLVEESRAAGINGELPAFVTKLADRAVAEGRGGDSYAALIEQFRKSA

SEQ ID NO: 61 - DNA, 879 bp, synthetic construct
  misc_feature 1..879: note = Imine reductase variant from Pseudonocardia spinosispora
  source 1..879: mol_type = other DNA
atgagtgattcccccgtacctgtgactgttctgggtcttggtctgatgggtcaggccttagcgggagcgtttctggcagccggtcaccctacgacggtttggaatcgcagcgcagctaaagctgatgaactggttggtcgcggtgcaaccctggccgcgtctcccgcggctgccgtcgcagcgggtagtctgatcgttgtttgcgtcacagatcatcgtgcggtgcgcgaactgctggaaccacttggcgatgcactgccaggtcgcgttctggtcaacctgacgagcggtacgtcgcgtgaagcccgtgagaacgcagaacatactgcggctcagggagccacctacctggatggtgtgattctgaccattccaagcggcattggcaccccagaagctaccattctgtattcgggaccgcgcagtaccttcgatgaacatgaaagcgcactgcgcgcattaggtccgggggcgacctttgtaggggaagatcacggactggctgcactgtatgatgcagcaatgctgagcgtcatgtggggcctgctgaatggtttcctgcatggaaccgcactgctgggaaccgcgggcgtttcggcaacctctgtggttccgatgctgggtcaaggtatcgttgcggtgaccggttggattgcgcgctacgcagatcagattgatgccggtgtctatccagcagacgacgccacgattgatacccagcgtgctgcaatgcagcacctggtcgaggagagccgtgcggcgggcatcaatggcgaacttccggcgtttgtgaccaaactggccgatcgcgcagtggcagaaggtcgtggtggtgactcttacgctgcactgattgaacagtttcgcaagtcagcttaa

SEQ ID NO: 62 - protein, 292 aa, synthetic construct
  REGION 1..292: note = Imine reductase variant from Pseudonocardia spinosispora
MSDSPVPVTVLGLGLMGQALAGAFLAAGHPTTVWNRSAAKADELVGRGATLAASPAAAVAAGSLIVVCVTDHRAVRELLEPLGDALPGRVLVNLTSGTSREARENAEHTAAQGATYLDGVILTIPSGIGTPEATILYSGPRSTFDEHESALRALGPGATFVGEDHGLAALYDAAMLSVMWGLLNGFLHGTALLGTAGVSATSVVPMLGQGIVAVTGWIARYADQIDAGVYPADDATIDTQRAAMQHLVEESRAAGINGELPAFVTKLADRAVAEGRGGDSYAALIEQFRKSA

SEQ ID NO: 63 - DNA, 879 bp, synthetic construct
  misc_feature 1..879: note = Imine reductase variant from Pseudonocardia spinosispora
  source 1..879: mol_type = other DNA
atgagtgattcccccgtacctgtgactgttctgggtcttggtctgatgggtcaggccttagcgggagcgtttctggcagccggtcaccctacgacggtttggaatcgcagcgcagctaaagctgatgaactggttggtcgcggtgcaaccctggccgcgtctcccgcggctgccgtcgcagcgggtagtctgatcgttgtttgcgtcacagatcatcgtgcggtgcgcgaactgctggaaccacttggcgatgcactgccaggtcgcgttctggtcaacctgacgagcggtacgtcgcgtgaagcccgtgagaacgcagaacatactgcggctcagggagccacctacctggatggtgtgattctgaccattccaagcggcattggcaccccagaagctaccattctgtattcgggaccgcgcagtaccttcgatgaacatgaaagcgcactgcgcgcattaggtccgggggcgacctttgtaggggaagatcacggactggctgcactgtatgatgcagcaatgctgagcgtcatgtggggcctgctgaatggtttcctgcatggaaccgcactgctgggaaccgcgggcgtttcggcaacctctgtggttccgatgctgggtcaaggtatcgaagcggtgatgggttggattgcgcgctacgcagatcagattgatgccggtgtctatccagcagacgacgccacgattgatacccagcgtgctgcaatgcagcacctggtcgaggagagccgtgcggcgggcatcaatggcgaacttccggcgtttgtgaccaaactggccgatcgcgcagtggcagaaggtcgtggtggtgactcttacgctgcactgattgaacagtttcgcaagtcagcttaa

SEQ ID NO: 64 - protein, 292 aa, synthetic construct
  REGION 1..292: note = Imine reductase variant from Pseudonocardia spinosispora
MSDSPVPVTVLGLGLMGQALAGAFLAAGHPTTVWNRSAAKADELVGRGATLAASPAAAVAAGSLIVVCVTDHRAVRELLEPLGDALPGRVLVNLTSGTSREARENAEHTAAQGATYLDGVILTIPSGIGTPEATILYSGPRSTFDEHESALRALGPGATFVGEDHGLAALYDAAMLSVMWGLLNGFLHGTALLGTAGVSATSVVPMLGQGIEAVMGWIARYADQIDAGVYPADDATIDTQRAAMQHLVEESRAAGINGELPAFVTKLADRAVAEGRGGDSYAALIEQFRKSA

SEQ ID NO: 65 - DNA, 879 bp, synthetic construct
  misc_feature 1..879: note = Imine reductase variant from Pseudonocardia spinosispora
  source 1..879: mol_type = other DNA
atgagtgattcccccgtacctgtgactgttctgggtcttggtctgatgggtcaggccttagcgggagcgtttctggcagccggtcaccctacgacggtttggaatcgcagcgcagctaaagctgatgaactggttggtcgcggtgcaaccctggccgcgtctcccgcggctgccgtcgcagcgggtagtctgatcgttgtttgcgtcacagatcatcgtgcggtgcgcgaactgctggaaccacttggcgatgcactgccaggtcgcgttctggtcaacctgacgagcggtacgtcgcgtgaagcccgtgagaacgcagaacatactgcggctcagggagccacctacctggatggtgtgattctgaccattccaagcggcattggcaccccagaagctaccattctgtattcgggaccgcgcagtaccttcgatgaacatgaaagcgcactgcgcgcattaggtccgggggcgacctttgtaggggaagatcacggactggctgcactgtatgatgcagcaatgctgagcgtcatgtggggcctgctgaatggtttcctgcatggaaccgcactgctgggaaccgcgggcgtttcggcaacctctgtggttccgatgctgggtcaaggttgggaagcggtgaccggttggattgcgcgctacgcagatcagattgatgccggtgtctatccagcagacgacgccacgattgatacccagcgtgctgcaatgcagcacctggtcgaggagagccgtgcggcgggcatcaatggcgaacttccggcgtttgtgaccaaactggccgatcgcgcagtggcagaaggtcgtggtggtgactcttacgctgcactgattgaacagtttcgcaagtcagcttaa

SEQ ID NO: 66 - protein, 292 aa, synthetic construct
  REGION 1..292: note = Imine reductase variant from Pseudonocardia spinosispora
MSDSPVPVTVLGLGLMGQALAGAFLAAGHPTTVWNRSAAKADELVGRGATLAASPAAAVAAGSLIVVCVTDHRAVRELLEPLGDALPGRVLVNLTSGTSREARENAEHTAAQGATYLDGVILTIPSGIGTPEATILYSGPRSTFDEHESALRALGPGATFVGEDHGLAALYDAAMLSVMWGLLNGFLHGTALLGTAGVSATSVVPMLGQGWEAVTGWIARYADQIDAGVYPADDATIDTQRAAMQHLVEESRAAGINGELPAFVTKLADRAVAEGRGGDSYAALIEQFRKSA

SEQ ID NO: 67 - DNA, 879 bp, synthetic construct
  misc_feature 1..879: note = Imine reductase variant from Pseudonocardia spinosispora
  source 1..879: mol_type = other DNA
atgagtgattcccccgtacctgtgactgttctgggtcttggtctgatgggtcaggccttagcgggagcgtttctggcagccggtcaccctacgacggtttggaatcgcagcgcagctaaagctgatgaactggttggtcgcggtgcaaccctggccgcgtctcccgcgactgccgtcgcagcgggtagtctgatcgttgtttgcgtcacagatcatcgtgcggtgcgcgaactgctggaaccacttggcgatgcactgccaggtcgcgttctggtcaacctgacgagcggtacgtcgcgtgaagcccgtgagaacgcagaacatactgcggctcagggagccacctacctggatggtgtgattctgaccattccaagcggcattggcaccccagaagctaccattctgtattcgggaccgcgcagtaccttcgatgaacatgaaagcgcactgcgcgcattaggtccgggggcgacctttgtaggggaagatcacggactggctgcactgtatgatgcagcaatgctgagcgtcatgtggggcctgctgaatggtttcctgcatggaaccgcactgctgggaaccgcgggcgtttcggcaacctctgtggttccgatgctgggtcaaggtcttgaagcggtgaccggttggattgcgcgctacgcagatcagattgatgccggtgtctatccagcagacgacgccacgattgatacccagcgtgctgcaatgcagcacctggtcgaggagagccgtgcggcgggcatcaatggcgaacttccggcgtttgtgaccaaactggccgatcgcgcagtggcagaaggtcgtggtggtgactcttacgctgcactgattgaacagtttcgcaagtcagcttaa

SEQ ID NO: 68 - protein, 292 aa, synthetic construct
  REGION 1..292: note = Imine reductase variant from Pseudonocardia spinosispora
MSDSPVPVTVLGLGLMGQALAGAFLAAGHPTTVWNRSAAKADELVGRGATLAASPATAVAAGSLIVVCVTDHRAVRELLEPLGDALPGRVLVNLTSGTSREARENAEHTAAQGATYLDGVILTIPSGIGTPEATILYSGPRSTFDEHESALRALGPGATFVGEDHGLAALYDAAMLSVMWGLLNGFLHGTALLGTAGVSATSVVPMLGQGLEAVTGWIARYADQIDAGVYPADDATIDTQRAAMQHLVEESRAAGINGELPAFVTKLADRAVAEGRGGDSYAALIEQFRKSA

SEQ ID NO: 69 - DNA, 879 bp, synthetic construct
  misc_feature 1..879: note = Imine reductase variant from Pseudonocardia spinosispora
  source 1..879: mol_type = other DNA
atgagtgattcccccgtacctgtgactgttctgggtcttggtctgatgggtcaggccttagcgggagcgtttctggcagccggtcaccctacgacggtttggaatcgcagcgcagctaaagctgatgaactggttggtcgcggtgcaaccctggccgcgtctcccgcggctgccgtcgcagcgggtagtctgatcgttgtttgcgtcacagatcatcgtgcggtgcgcgaactgctggaaccacttggcgatgcactgccaggtcgcgttctggtcaacctgacgagcggtacgtcgcgtgaagcccgtgagaacgcagaacatactgcggctcagggagccacctacctggatggtgtgattctgaccattccaagcggcattggcaccccagaagctaccattctgtattcgggaccgcgcagtaccttcgatgaacatgaaagcgcactgcgcgcattaggtccgggggcgacctttgtaggggaagatcacggactggctgcactgtatgatgcagcaatgctgagcgtcatgtggggcctgctgaatggtttcctgcatggaaccgcactgctgggaaccgcgggcgtttcggcaacctctgtggttccgatgctgggtcaaggtcttgaagcggtgaccggttggattgcgcgctacgcagatcagattgatgccggtgtctatccagcagacgacgccacgattgatacccagcgtgctgcaatgcagcacctggtcgaggagagccgtgcggcgggcatcaatggcgaacttccggcgtttgtgaccaaactggccgatcgcgcagtggcagaaggtcgtggtggtgactcttacgctgcactgattgaacagtttcgcaagtcagcttaa

SEQ ID NO: 70 - protein, 292 aa, synthetic construct
  REGION 1..292: note = Imine reductase variant from Pseudonocardia spinosispora
MSDSPVPVTVLGLGLMGQALAGAFLAAGHPTTVWNRSAAKADELVGRGATLAASPAAAVAAGSLIVVCVTDHRAVRELLEPLGDALPGRVLVNLTSGTSREARENAEHTAAQGATYLDGVILTIPSGIGTPEATILYSGPRSTFDEHESALRALGPGATFVGEDHGLAALYDAAMLSVMWGLLNGFLHGTALLGTAGVSATSVVPMLGQGLEAVTGWIARYADQIDAGVYPADDATIDTQRAAMQHLVEESRAAGINGELPAFVTKLADRAVAEGRGGDSYAALIEQFRKSA

SEQ ID NO: 71 - DNA, 879 bp, synthetic construct
  misc_feature 1..879: note = Imine reductase variant from Pseudonocardia spinosispora
  source 1..879: mol_type = other DNA
atgagtgattcccccgtacctgtgactgttctgggtcttggtctgatgggtcaggccttagcgggagcgtttctggcagccggtcaccctacgacggtttggaatcgcagcgcagctaaagctgatgaactggttggtcgcggtgcaaccctggccgcgtctcccgcggctgccgtcgcagcgggtagtctgatcgttgtttgcgtcacagatcatcgtgcggtgcgcgaactgctggaaccacttggcgatgcactgccaggtcgcgttctggtcaacctgacgagcggtacgtcgcgtgaagcccgtgagaacgcagaacatactgcggctcagggagccacctacctggatggtgtgattctgaccattccaagcggcattggcaccccagaagctaccattctgtattcgggaccgcgcagtaccttcgatgaacatgaaagcgcactgcgcgcattaggtccgggggcgacctttgtaggggaagatcacggactggctgcactgtatgatgcagcaatgctgagcgtcatgtggggcctgctgaatggtttcctgcatggaaccgcactgctgggaaccgcgggcgtttcggcaacctctgtggttccgatgctgggtcaaggtatcggtgcggtgaccggttggattgcgcgctacgcagatcagattgatgccggtgtctatccagcagacgacgccacgattgatacccagcgtgctgcaatgcagcacctggtcgaggagagccgtgcggcgggcatcaatggcgaacttccggcgtttgtgaccaaactggccgatcgcgcagtggcagaaggtcgtggtggtgactcttacgctgcactgattgaacagtttcgcaagtcagcttaa

SEQ ID NO: 72 - protein, 292 aa, synthetic construct
  REGION 1..292: note = Imine reductase variant from Pseudonocardia spinosispora
MSDSPVPVTVLGLGLMGQALAGAFLAAGHPTTVWNRSAAKADELVGRGATLAASPAAAVAAGSLIVVCVTDHRAVRELLEPLGDALPGRVLVNLTSGTSREARENAEHTAAQGATYLDGVILTIPSGIGTPEATILYSGPRSTFDEHESALRALGPGATFVGEDHGLAALYDAAMLSVMWGLLNGFLHGTALLGTAGVSATSVVPMLGQGIGAVTGWIARYADQIDAGVYPADDATIDTQRAAMQHLVEESRAAGINGELPAFVTKLADRAVAEGRGGDSYAALIEQFRKSA

SEQ ID NO: 73 - DNA, 879 bp, synthetic construct
  misc_feature 1..879: note = Imine reductase variant from Pseudonocardia spinosispora
  source 1..879: mol_type = other DNA
atgagtgattcccccgtacctgtgactgttctgggtcttggtctgatgggtcaggccttagcgggagcgtttctggcagccggtcaccctacgacggtttggaatcgcagcgcagctaaagctgatgaactggttggtcgcggtgcaaccctggccgcgtctcccgcggctgccgtcgcagcgggtagtctgatcgttgtttgcgtcacagatcatcgtgcggtgcgcgaactgctggaaccacttggcgatgcactgccaggtcgcgttctggtcaacctgacgagcggtacgtcgcgtgaagcccgtgagaacgcagaacatactgcggctcagggagccacctacctggatggtgtgattctgaccattccaagcggcattggcaccccagaagctaccattctgtattcgggaccgcgcagtaccttcgatgaacatgaaagcgcactgcgcgcattaggtccgggggcgacctttgtaggggaagatcacggactggctgcactgtatgatgcagcaatgctgagcgtcatgtggggcctgctgaatggtttcctgcatggaaccgcactgctgggaaccgcgggcgtttcggcaacctctgtggttccgatgctgggtcaaggtatcgaagcgatgaccggttggattgcgcgctacgcagatcagattgatgccggtgtctatccagcagacgacgccacgattgatacccagcgtgctgcaatgcagcacctggtcgaggagagccgtgcggcgggcatcaatggcgaacttccggcgtttgtgaccaaactggccgatcgcgcagtggcagaaggtcgtggtggtgactcttacgctgcactgattgaacagtttcgcaagtcagcttaa

SEQ ID NO: 74 - protein, 292 aa, synthetic construct
  REGION 1..292: note = Imine reductase variant from Pseudonocardia spinosispora
MSDSPVPVTVLGLGLMGQALAGAFLAAGHPTTVWNRSAAKADELVGRGATLAASPAAAVAAGSLIVVCVTDHRAVRELLEPLGDALPGRVLVNLTSGTSREARENAEHTAAQGATYLDGVILTIPSGIGTPEATILYSGPRSTFDEHESALRALGPGATFVGEDHGLAALYDAAMLSVMWGLLNGFLHGTALLGTAGVSATSVVPMLGQGIEAMTGWIARYADQIDAGVYPADDATIDTQRAAMQHLVEESRAAGINGELPAFVTKLADRAVAEGRGGDSYAALIEQFRKSA

SEQ ID NO: 75 - DNA, 879 bp, synthetic construct
  misc_feature 1..879: note = Imine reductase variant from Pseudonocardia spinosispora
  source 1..879: mol_type = other DNA
atgagtgattcacctgtgcccgtgacagttctgggtcttggtctgatgggtcaggccttagcgggagcgtttctggcagccggtcaccctacgacggtttggaatcgcagcgcagctaaagctgatgaactggttggtcgcggtgcaaccctggccgcgtctcccgcggctgccgtcgcagcgggtagtctgatcgttgtttgcgtcacagatcatcgtgcggtgcgcgaactgctggaaccacttggcgatgcactgccaggtcgcgttctggtcaacctgacgagcggtacgtcgcgtgaagcccgtgagaacgcagaacatactgcggctcagggagccacctacctggatggtgtgattctgggtggcccaagcggcattggcaccccagaagctaccattctgtattcgggaccgcgcagtaccttcgatgaacatgaaagcgcactgcgcgcattaggtccgggggcgacctttgtaggggaagatcacggactggctaatctggttgatcatgcaatgctgagcgtcatgtggggcctgctgaatggtttcctgcatggaaccgcactgctgggaaccgcgggcgtttcggcaacctctgtggttccgatgctgggtcaaggtatcgaagtggtgaccggttggattgcgcgctacgcagatcagattgatgccggtgtctatccagcagacgacaagacgattgatacccagcgtgctgcaatgcagcacctggtcgaggagagccgtgcggcgggcatcaatggcgaacttccggcgtttgtgaccaaactggccgatcgcgcagtggcagaaggtcgtggtggtgactcttacgctgcactgattgaacagtttcgcaagtcagcttaa

SEQ ID NO: 76 - protein, 292 aa, synthetic construct
  REGION 1..292: note = Imine reductase variant from Pseudonocardia spinosispora
MSDSPVPVTVLGLGLMGQALAGAFLAAGHPTTVWNRSAAKADELVGRGATLAASPAAAVAAGSLIVVCVTDHRAVRELLEPLGDALPGRVLVNLTSGTSREARENAEHTAAQGATYLDGVILGGPSGIGTPEATILYSGPRSTFDEHESALRALGPGATFVGEDHGLANLVDHAMLSVMWGLLNGFLHGTALLGTAGVSATSVVPMLGQGIEVVTGWIARYADQIDAGVYPADDKTIDTQRAAMQHLVEESRAAGINGELPAFVTKLADRAVAEGRGGDSYAALIEQFRKSA

SEQ ID NO: 77 - DNA, 879 bp, synthetic construct
  misc_feature 1..879: note = Imine reductase variant from Pseudonocardia spinosispora
  source 1..879: mol_type = other DNA
atgagtgattcacctgtgcccgtgacagttctgggtcttggtctgatgggtcaggccttagcgggagcgtttctggcagccggtcaccctacgacggtttggaatcgcagcgcagctaaagctgatgaactggttggtcgcggtgcaaccctggccgcgtctcccgcggctgccgtcgcagcgggtagtctgatcgttgtttgcgtcacagatcatcgtgcggtgcgcgaactgctggaaccacttggcgatgcactgccaggtcgcgttctggtcaacctgacgagcggtacgtcgcgtgaagcccgtgagaacgcagaacatactgcggctcagggagccacctacctggatggtgtgattctgacgggcccaagcggcattggcaccccagaagctaccattctgtattcgggaccgcgcagtaccttcgatgaacatgaaagcgcactgcgcgcattaggtccgggggcgacctttgtaggggaagatcacggactggctaatctgtacgatattgcaatgctgagcgtcatgtggggcctgctgaatggtttcctgcatggaaccgcactgctgggaaccgcgggcgtttcggcaacctctgtggttccgatgctgggtcaaggtatcggagtggtgaccggttggattgcgcgctacgcagatcagattgatgccggtgtctatccagcagacgacgcgacgattgatacccagcgtgctgcaatgcagcacctggtcgaggagagccgtgcggcgggcatcaatggcgaacttccggcgtttgtgaccaaactggccgatcgcgcagtggcagaaggtcgtggtggtgactcttacgctgcactgattgaacagtttcgcaagtcagcttaa

SEQ ID NO: 78 - protein, 292 aa, synthetic construct
  REGION 1..292: note = Imine reductase variant from Pseudonocardia spinosispora
MSDSPVPVTVLGLGLMGQALAGAFLAAGHPTTVWNRSAAKADELVGRGATLAASPAAAVAAGSLIVVCVTDHRAVRELLEPLGDALPGRVLVNLTSGTSREARENAEHTAAQGATYLDGVILTGPSGIGTPEATILYSGPRSTFDEHESALRALGPGATFVGEDHGLANLYDIAMLSVMWGLLNGFLHGTALLGTAGVSATSVVPMLGQGIGVVTGWIARYADQIDAGVYPADDATIDTQRAAMQHLVEESRAAGINGELPAFVTKLADRAVAEGRGGDSYAALIEQFRKSA

SEQ ID NO: 79 - DNA, 879 bp, synthetic construct
  misc_feature 1..879: note = Imine reductase variant from Pseudonocardia spinosispora
  source 1..879: mol_type = other DNA
atgagtgattcacctgtgcccgtgacagttctgggtcttggtctgatgggtcaggccttagcgggagcgtttctggcagccggtcaccctacgacggtttggaatcgcagcgcagctaaagctgatgaactggttggtcgcggtgcaaccctggccgcgtctcccgcggctgccgtcgcagcgggtagtctgatcgttgtttgcgtcacagatcatcgtgcggtgcgcgaactgctggaaccacttggcgatgcactgccaggtcgcgttctggtcaacctgacgagcggtacgtcgcgtgaagcccgtgagaacgcagaacatactgcggctcagggagccacctacctggatggtgtgattctgacgggcccaagcggcattggcaccccagaagctaccattctgtattcgggaccgcgcagtaccttcgatgaacatgaaagcgcactgcgcgcattaggtccgggggcgacctttgtaggggaagatcacggactggctaatctgtacgatgccgcaggcctgagcgtcatgtggggcctgctgaatggtttcctgcatggaaccgcactgctgggaaccgcgggcgtttcggcaacctctgtggttccgatgctgggtcaaggtatctgcgtggtgaccggttggattgcgcgctacgcagatcagattgatgccggtgtctatccagcagacgacaagacgattgatacccagcgtgctgcaatgcagcacctggtcgaggagagccgtgcggcgggcatcaatggcgaacttccggcgtttgtgaccaaactggccgatcgcgcagtggcagaaggtcgtggtggtgactcttacgctgcactgattgaacagtttcgcaagtcagcttaa

SEQ ID NO: 80 - protein, 292 aa, synthetic construct
  REGION 1..292: note = Imine reductase variant from Pseudonocardia spinosispora
MSDSPVPVTVLGLGLMGQALAGAFLAAGHPTTVWNRSAAKADELVGRGATLAASPAAAVAAGSLIVVCVTDHRAVRELLEPLGDALPGRVLVNLTSGTSREARENAEHTAAQGATYLDGVILTGPSGIGTPEATILYSGPRSTFDEHESALRALGPGATFVGEDHGLANLYDAAGLSVMWGLLNGFLHGTALLGTAGVSATSVVPMLGQGICVVTGWIARYADQIDAGVYPADDKTIDTQRAAMQHLVEESRAAGINGELPAFVTKLADRAVAEGRGGDSYAALIEQFRKSA

SEQ ID NO: 81 - DNA, 879 bp, synthetic construct
  misc_feature 1..879: note = Imine reductase variant from Pseudonocardia spinosispora
  source 1..879: mol_type = other DNA
atgagtgattcacctgtgcccgtgacagttctgggtcttggtctgatgggtcaggccttagcgggagcgtttctggcagccggtcaccctacgacggtttggaatcgcagcgcagctaaagctgatgaactggttggtcgcggtgcaaccctggccgcgtctcccgcggctgccgtcgcagcgggtagtctgatcgttgtttgcgtcacagatcatcgtgcggtgcgcgaactgctggaaccacttggcgatgcactgccaggtcgcgttctggtcaacctgacgagcggtacgtcgcgtgaagcccgtgagaacgcagaacatactgcggctcagggagccacctacctggatggtgtgattctgacgattccaagcggcattggcaccccagaagctaccattctgtattcgggaccgcgcagtaccttcgatgaacatgaaagcgcactgcgcgcattaggtccgggggcgacctttgtaggggaagatcacggactggctgccctggttgatattgcaatgctgagcgtcatgtggggcctgctgaatggtttcctgcatggaaccgcactgctgggaaccgcgggcgtttcggcaacctctgtggttccgatgctgggtcaaggtatcggagtggtgaccggttggattgcgcgctacgcagatcagattgatgccggtgtctatccagcagacgacaagacgattgatacccagcgtgctgcaatgcagcacctggtcgaggagagccgtgcggcgggcatcaatggcgaacttccggcgtttgtgaccaaactggccgatcgcgcagtggcagaaggtcgtggtggtgactcttacgctgcactgattgaacagtttcgcaagtcagcttaa

SEQ ID NO: 82 - protein, 292 aa, synthetic construct
  REGION 1..292: note = Imine reductase variant from Pseudonocardia spinosispora
MSDSPVPVTVLGLGLMGQALAGAFLAAGHPTTVWNRSAAKADELVGRGATLAASPAAAVAAGSLIVVCVTDHRAVRELLEPLGDALPGRVLVNLTSGTSREARENAEHTAAQGATYLDGVILTIPSGIGTPEATILYSGPRSTFDEHESALRALGPGATFVGEDHGLAALVDIAMLSVMWGLLNGFLHGTALLGTAGVSATSVVPMLGQGIGVVTGWIARYADQIDAGVYPADDKTIDTQRAAMQHLVEESRAAGINGELPAFVTKLADRAVAEGRGGDSYAALIEQFRKSA

SEQ ID NO: 83 - DNA, 879 bp, synthetic construct
  misc_feature 1..879: note = Imine reductase variant from Pseudonocardia spinosispora
  source 1..879: mol_type = other DNA
atgagtgattcacctgtgcccgtgacagttctgggtcttggtctgatgggtcaggccttagcgggagcgtttctggcagccggtcaccctacgacggtttggaatcgcagcgcagctaaagctgatgaactggttggtcgcggtgcaaccctggccgcgtctcccgcggctgccgtcgcagcgggtagtctgatcgttgtttgcgtcacagatcatcgtgcggtgcgcgaactgctggaaccacttggcgatgcactgccaggtcgcgttctggtcaacctgacgagcggtacgtcgcgtgaagcccgtgagaacgcagaacatactgcggctcagggagccacctacctggatggtgtgattctgacgattccaagcggcattggcaccccagaagctaccattctgtattcgggaccgcgcagtaccttcgatgaacatgaaagcgcactgcgcgcattaggtccgggggcgacctttgtaggggaagatcacggactggctaatctgtacgatgcagcaatgctgagcgtcatgtggggcctgctgaatggtttcctgcatggaaccgcactgctgggaaccgcgggcgtttcggcaacctctgtggttccgatgctgggtcaaggtatcgaagcggtgaccggttggattgcgcgctacgcagatcagattgatgccggtgtctatccagcagacgacaagacgattgatacccagcgtgctgcaatgcagcacctggtcgaggagagccgtgcggcgggcatcaatggcgaacttccggcgtttgtgaccaaactggccgatcgcgcagtggcagaaggtcgtggtggtgactcttacgctgcactgattgaacagtttcgcaagtcagcttaa

SEQ ID NO: 84 - protein, 292 aa, synthetic construct
  REGION 1..292: note = Imine reductase variant from Pseudonocardia spinosispora
MSDSPVPVTVLGLGLMGQALAGAFLAAGHPTTVWNRSAAKADELVGRGATLAASPAAAVAAGSLIVVCVTDHRAVRELLEPLGDALPGRVLVNLTSGTSREARENAEHTAAQGATYLDGVILTIPSGIGTPEATILYSGPRSTFDEHESALRALGPGATFVGEDHGLANLYDAAMLSVMWGLLNGFLHGTALLGTAGVSATSVVPMLGQGIEAVTGWIARYADQIDAGVYPADDKTIDTQRAAMQHLVEESRAAGINGELPAFVTKLADRAVAEGRGGDSYAALIEQFRKSA

SEQ ID NO: 85 - DNA, 879 bp, synthetic construct
  misc_feature 1..879: note = Imine reductase variant from Pseudonocardia spinosispora
  source 1..879: mol_type = other DNA
atgagtgattcacctgtgcccgtgacagttctgggtcttggtctgatgggtcaggccttagcgggagcgtttctggcagccggtcaccctacgacggtttggaatcgcagcgcagctaaagctgatgaactggttggtcgcggtgcaaccctggccgcgtctcccgcggctgccgtcgcagcgggtagtctgatcgttgtttgcgtcacagatcatcgtgcggtgcgcgaactgctggaaccacttggcgatgcactgccaggtcgcgttctggtcaacctgacgagcggtacgtcgcgtgaagcccgtgagaacgcagaacatactgcggctcagggagccacctacctggatggtgtgattctgggtattccaagcggcattggcaccccagaagctaccattctgtattcgggaccgcgcagtaccttcgatgaacatgaaagcgcactgcgcgcattaggtccgggggcgacctttgtaggggaagatcacggactggctaatctgtacgatcatgcacacctgagcgtcatgtggggcctgctgaatggtttcctgcatggaaccgcactgctgggaaccgcgggcgtttcggcaacctctgtggttccgatgctgggtcaaggtatcgaagtggtgaccggttggattgcgcgctacgcagatcagattgatgccggtgtctatccagcagacgacaagacgattgatacccagcgtgctgcaatgcagcacctggtcgaggagagccgtgcggcgggcatcaatggcgaacttccggcgtttgtgaccaaactggccgatcgcgcagtggcagaaggtcgtggtggtgactcttacgctgcactgattgaacagtttcgcaagtcagcttaa

SEQ ID NO: 86 - protein, 292 aa, synthetic construct
  REGION 1..292: note = Imine reductase variant from Pseudonocardia spinosispora
MSDSPVPVTVLGLGLMGQALAGAFLAAGHPTTVWNRSAAKADELVGRGATLAASPAAAVAAGSLIVVCVTDHRAVRELLEPLGDALPGRVLVNLTSGTSREARENAEHTAAQGATYLDGVILGIPSGIGTPEATILYSGPRSTFDEHESALRALGPGATFVGEDHGLANLYDHAHLSVMWGLLNGFLHGTALLGTAGVSATSVVPMLGQGIEVVTGWIARYADQIDAGVYPADDKTIDTQRAAMQHLVEESRAAGINGELPAFVTKLADRAVAEGRGGDSYAALIEQFRKSA

SEQ ID NO: 87 - DNA, 879 bp, synthetic construct
  misc_feature 1..879: note = Imine reductase variant from Pseudonocardia spinosispora
  source 1..879: mol_type = other DNA
atgagtgattcacctgtgcccgtgacagttctgggtcttggtctgatgggtcaggccttagcgggagcgtttctggcagccggtcaccctacgacggtttggaatcgcagcgcagctaaagctgatgaactggttggtcgcggtgcaaccctggccgcgtctcccgcggctgccgtcgcagcgggtagtctgatcgttgtttgcgtcacagatcatcgtgcggtgcgcgaactgctggaaccacttggcgatgcactgccaggtcgcgttctggtcaacctgacgagcggtacgtcgcgtgaagcccgtgagaacgcagaacatactgcggctcagggagccacctacctggatggtgtgattctgggtattccaagcggcattggcaccccagaagctaccattctgtattcgggaccgcgcagtaccttcgatgaacatgaaagcgcactgcgcgcattaggtccgggggcgacctttgtaggggaagatcacggactggctaatctgtacgatattgcaatgctgagcgtcatgtggggcctgctgaatggtttcctgcatggaaccgcactgctgggaaccgcgggcgtttcggcaacctctgtggttccgatgctgggtcaaggtatcggaactgtgaccggttggattgcgcgctacgcagatcagattgatgccggtgtctatccagcagacgacgccacgattgatacccagcgtgctgcaatgcagcacctggtcgaggagagccgtgcggcgggcatcaatggcgaacttccggcgtttgtgaccaaactggccgatcgcgcagtggcagaaggtcgtggtggtgactcttacgctgcactgattgaacagtttcgcaagtcagcttaa

SEQ ID NO: 88 - protein, 292 aa, synthetic construct
  REGION 1..292: note = Imine reductase variant from Pseudonocardia spinosispora
MSDSPVPVTVLGLGLMGQALAGAFLAAGHPTTVWNRSAAKADELVGRGATLAASPAAAVAAGSLIVVCVTDHRAVRELLEPLGDALPGRVLVNLTSGTSREARENAEHTAAQGATYLDGVILGIPSGIGTPEATILYSGPRSTFDEHESALRALGPGATFVGEDHGLANLYDIAMLSVMWGLLNGFLHGTALLGTAGVSATSVVPMLGQGIGTVTGWIARYADQIDAGVYPADDATIDTQRAAMQHLVEESRAAGINGELPAFVTKLADRAVAEGRGGDSYAALIEQFRKSA

SEQ ID NO: 89 - DNA, 879 bp, synthetic construct
  misc_feature 1..879: note = Imine reductase variant from Pseudonocardia spinosispora
  source 1..879: mol_type = other DNA
atgagtgattcacctgtgcccgtgacagttctgggtcttggtctgatgggtcaggccttagcgggagcgtttctggcagccggtcaccctacgacggtttggaatcgcagcgcagctaaagctgatgaactggttggtcgcggtgcaaccctggccgcgtctcccgcggctgccgtcgcagcgggtagtctgatcgttgtttgcgtcacagatcatcgtgcggtgcgcgaactgctggaaccacttggcgatgcactgccaggtcgcgttctggtcaacctgacgagcggtacgtcgcgtgaagcccgtgagaacgcagaacatactgcggctcagggagccacctacctggatggtgtgattctgacgggcccaagcggcattggcaccccagaagctaccattctgtattcgggaccgcgcagtaccttcgatgaacatgaaagcgcactgcgcgcattaggtccgggggcgacctttgtaggggaagatcacggactggctgcactgtatgatgcagcaatgctgagcgtcatgtggggcctgctgaatggtttcctgcatggaaccgcactgctgggaaccgcgggcgtttcggcaacctctgtggttccgatgctgggtcaaggtatcggagtggtgaccggttggattgcgcgctacgcagatcagattgatgccggtgtctatccagcagacgacaagacgattgatacccagcgtgctgcaatgcagcacctggtcgaggagagccgtgcggcgggcatcaatggcgaacttccggcgtttgtgaccaaactggccgatcgcgcagtggcagaaggtcgtggtggtgactcttacgctgcactgattgaacagtttcgcaagtcagcttaa

SEQ ID NO: 90 - protein, 292 aa, synthetic construct
  REGION 1..292: note = Imine reductase variant from Pseudonocardia spinosispora
MSDSPVPVTVLGLGLMGQALAGAFLAAGHPTTVWNRSAAKADELVGRGATLAASPAAAVAAGSLIVVCVTDHRAVRELLEPLGDALPGRVLVNLTSGTSREARENAEHTAAQGATYLDGVILTGPSGIGTPEATILYSGPRSTFDEHESALRALGPGATFVGEDHGLAALYDAAMLSVMWGLLNGFLHGTALLGTAGVSATSVVPMLGQGIGVVTGWIARYADQIDAGVYPADDKTIDTQRAAMQHLVEESRAAGINGELPAFVTKLADRAVAEGRGGDSYAALIEQFRKSA

SEQ ID NO: 91 - DNA, 879 bp, synthetic construct
  misc_feature 1..879: note = Imine reductase variant from Pseudonocardia spinosispora
  source 1..879: mol_type = other DNA
atgagtgattcacctgtgcccgtgacagttctgggtcttggtctgatgggtcaggccttagcgggagcgtttctggcagccggtcaccctacgacggtttggaatcgcagcgcagctaaagctgatgaactggttggtcgcggtgcaaccctggccgcgtctcccgcggctgccgtcgcagcgggtagtctgatcgttgtttgcgtcacagatcatcgtgcggtgcgcgaactgctggaaccacttggcgatgcactgccaggtcgcgttctggtcaacctgacgagcggtacgtcgcgtgaagcccgtgagaacgcagaacatactgcggctcagggagccacctacctggatggtgtgattctgggtattccaagcggcattggcaccccagaagctaccattctgtattcgggaccgcgcagtaccttcgatgaacatgaaagcgcactgcgcgcattaggtccgggggcgacctttgtaggggaagatcacggactggctgccctgtacgatcatgcacacctgagcgtcatgtggggcctgctgaatggtttcctgcatggaaccgcactgctgggaaccgcgggcgtttcggcaacctctgtggttccgatgctgggtcaaggtatctgcgtggtgaccggttggattgcgcgctacgcagatcagattgatgccggtgtctatccagcagacgacaagacgattgatacccagcgtgctgcaatgcagcacctggtcgaggagagccgtgcggcgggcatcaatggcgaacttccggcgtttgtgaccaaactggccgatcgcgcagtggcagaaggtcgtggtggtgactcttacgctgcactgattgaacagtttcgcaagtcagcttaa

SEQ ID NO: 92 - protein, 292 aa, synthetic construct
  REGION 1..292: note = Imine reductase variant from Pseudonocardia spinosispora
MSDSPVPVTVLGLGLMGQALAGAFLAAGHPTTVWNRSAAKADELVGRGATLAASPAAAVAAGSLIVVCVTDHRAVRELLEPLGDALPGRVLVNLTSGTSREARENAEHTAAQGATYLDGVILGIPSGIGTPEATILYSGPRSTFDEHESALRALGPGATFVGEDHGLAALYDHAHLSVMWGLLNGFLHGTALLGTAGVSATSVVPMLGQGICVVTGWIARYADQIDAGVYPADDKTIDTQRAAMQHLVEESRAAGINGELPAFVTKLADRAVAEGRGGDSYAALIEQFRKSA

SEQ ID NO: 93 - DNA, 879 bp, synthetic construct
  misc_feature 1..879: note = Imine reductase variant from Pseudonocardia spinosispora
  source 1..879: mol_type = other DNA
atgagtgattcacctgtgcccgtgacagttctgggtcttggtctgatgggtcaggccttagcgggagcgtttctggcagccggtcaccctacgacggtttggaatcgcagcgcagctaaagctgatgaactggttggtcgcggtgcaaccctggccgcgtctcccgcggctgccgtcgcagcgggtagtctgatcgttgtttgcgtcacagatcatcgtgcggtgcgcgaactgctggaaccacttggcgatgcactgccaggtcgcgttctggtcaacctgacgagcggtacgtcgcgtgaagcccgtgagaacgcagaacatactgcggctcagggagccacctacctggatggtgtgattctgacgattccaagcggcattggcaccccagaagctaccattctgtattcgggaccgcgcagtaccttcgatgaacatgaaagcgcactgcgcgcattaggtccgggggcgacctttgtaggggaagatcacggactggctaatctgtacgatgccgcaatgctgagcgtcatgtggggcctgctgaatggtttcctgcatggaaccgcactgctgggaaccgcgggcgtttcggcaacctctgtggttccgatgctgggtcaaggtatcggagtggtgaccggttggattgcgcgctacgcagatcagattgatgccggtgtctatccagcagacgacgccacgattgatacccagcgtgctgcaatgcagcacctggtcgaggagagccgtgcggcgggcatcaatggcgaacttccggcgtttgtgaccaaactggccgatcgcgcagtggcagaaggtcgtggtggtgactcttacgctgcactgattgaacagtttcgcaagtcagcttaa

SEQ ID NO: 94 - protein, 292 aa, synthetic construct
  REGION 1..292: note = Imine reductase variant from Pseudonocardia spinosispora
MSDSPVPVTVLGLGLMGQALAGAFLAAGHPTTVWNRSAAKADELVGRGATLAASPAAAVAAGSLIVVCVTDHRAVRELLEPLGDALPGRVLVNLTSGTSREARENAEHTAAQGATYLDGVILTIPSGIGTPEATILYSGPRSTFDEHESALRALGPGATFVGEDHGLANLYDAAMLSVMWGLLNGFLHGTALLGTAGVSATSVVPMLGQGIGVVTGWIARYADQIDAGVYPADDATIDTQRAAMQHLVEESRAAGINGELPAFVTKLADRAVAEGRGGDSYAALIEQFRKSA

SEQ ID NO: 95 - DNA, 879 bp, synthetic construct
  misc_feature 1..879: note = Imine reductase variant from Pseudonocardia spinosispora
  source 1..879: mol_type = other DNA
atgagtgattcacctgtgcccgtgacagttctgggtcttggtctgatgggtcaggccttagcgggagcgtttctggcagccggtcaccctacgacggtttggaatcgcagcgcagctaaagctgatgaactggttggtcgcggtgcaaccctggccgcgtctcccgcggctgccgtcgcagcgggtagtctgatcgttgtttgcgtcacagatcatcgtgcggtgcgcgaactgctggaaccacttggcgatgcactgccaggtcgcgttctggtcaacctgacgagcggtacgtcgcgtgaagcccgtgagaacgcagaacatactgcggctcagggagccacctacctggatggtgtgattctgacgattccaagcggcattggcaccccagaagctaccattctgtattcgggaccgcgcagtaccttcgatgaacatgaaagcgcactgcgcgcattaggtccgggggcgacctttgtaggggaagatcacggactggctgccctgtacgatgccgcacacctgagcgtcatgtggggcctgctgaatggtttcctgcatggaaccgcactgctgggaaccgcgggcgtttcggcaacctctgtggttccgatgctgggtcaaggtatcgaagcggtgaccggttggattgcgcgctacgcagatcagattgatgccggtgtctatccagcagacgacaagacgattgatacccagcgtgctgcaatgcagcacctggtcgaggagagccgtgcggcgggcatcaatggcgaacttccggcgtttgtgaccaaactggccgatcgcgcagtggcagaaggtcgtggtggtgactcttacgctgcactgattgaacagtttcgcaagtcagcttaa

SEQ ID NO: 96 - protein, 292 aa, synthetic construct
  REGION 1..292: note = Imine reductase variant from Pseudonocardia spinosispora
MSDSPVPVTVLGLGLMGQALAGAFLAAGHPTTVWNRSAAKADELVGRGATLAASPAAAVAAGSLIVVCVTDHRAVRELLEPLGDALPGRVLVNLTSGTSREARENAEHTAAQGATYLDGVILTIPSGIGTPEATILYSGPRSTFDEHESALRALGPGATFVGEDHGLAALYDAAHLSVMWGLLNGFLHGTALLGTAGVSATSVVPMLGQGIEAVTGWIARYADQIDAGVYPADDKTIDTQRAAMQHLVEESRAAGINGELPAFVTKLADRAVAEGRGGDSYAALIEQFRKSA

SEQ ID NO: 97 - DNA, 879 bp, synthetic construct
  misc_feature 1..879: note = Imine reductase variant from Pseudonocardia spinosispora
  source 1..879: mol_type = other DNA
atgagtgattcacctgtgcccgtgacagttctgggtcttggtctgatgggtcaggccttagcgggagcgtttctggcagccggtcaccctacgacggtttggaatcgcagcgcagctaaagctgatgaactggttggtcgcggtgcaaccctggccgcgtctcccgcggctgccgtcgcagcgggtagtctgatcgttgtttgcgtcacagatcatcgtgcggtgcgcgaactgctggaaccacttggcgatgcactgccaggtcgcgttctggtcaacctgacgagcggtacgtcgcgtgaagcccgtgagaacgcagaacatactgcggctcagggagccacctacctggatggtgtgattctgacgggcccaagcggcattggcaccccagaagctaccattctgtattcgggaccgcgcagtaccttcgatgaacatgaaagcgcactgcgcgcattaggtccgggggcgacctttgtaggggaagatcacggactggctaatctgtacgatgccgcaatgctgagcgtcatgtggggcctgctgaatggtttcctgcatggaaccgcactgctgggaaccgcgggcgtttcggcaacctctgtggttccgatgctgggtcaaggtatcgaagcggtgaccggttggattgcgcgctacgcagatcagattgatgccggtgtctatccagcagacgacgcgacgattgatacccagcgtgctgcaatgcagcacctggtcgaggagagccgtgcggcgggcatcaatggcgaacttccggcgtttgtgaccaaactggccgatcgcgcagtggcagaaggtcgtggtggtgactcttacgctgcactgattgaacagtttcgcaagtcagcttaa

SEQ ID NO: 98 - protein, 292 aa, synthetic construct
  REGION 1..292: note = Imine reductase variant from Pseudonocardia spinosispora
MSDSPVPVTVLGLGLMGQALAGAFLAAGHPTTVWNRSAAKADELVGRGATLAASPAAAVAAGSLIVVCVTDHRAVRELLEPLGDALPGRVLVNLTSGTSREARENAEHTAAQGATYLDGVILTGPSGIGTPEATILYSGPRSTFDEHESALRALGPGATFVGEDHGLANLYDAAMLSVMWGLLNGFLHGTALLGTAGVSATSVVPMLGQGIEAVTGWIARYADQIDAGVYPADDATIDTQRAAMQHLVEESRAAGINGELPAFVTKLADRAVAEGRGGDSYAALIEQFRKSA

SEQ ID NO: 99 - DNA, 879 bp, synthetic construct
  misc_feature 1..879: note = Imine reductase variant from Pseudonocardia spinosispora
  source 1..879: mol_type = other DNA
atgagtgattcacctgtgcccgtgacagttctgggtcttggtctgatgggtcaggccttagcgggagcgtttctggcagccggtcaccctacgacggtttggaatcgcagcgcagctaaagctgatgaactggttggtcgcggtgcaaccctggccgcgtctcccgcggctgccgtcgcagcgggtagtctgatcgttgtttgcgtcacagatcatcgtgcggtgcgcgaactgctggaaccacttggcgatgcactgccaggtcgcgttctggtcaacctgacgagcggtacgtcgcgtgaagcccgtgagaacgcagaacatactgcggctcagggagccacctacctggatggtgtgattctgacgattccaagcggcattggcaccccagaagctaccattctgtattcgggaccgcgcagtaccttcgatgaacatgaaagcgcactgcgcgcattaggtccgggggcgacctttgtaggggaagatcacggactggctaatctgtacgatgccgcaatgctgagcgtcatgtggggcctgctgaatggtttcctgcatggaaccgcactgctgggaaccgcgggcgtttcggcaacctctgtggttccgatgctgggtcaaggtatctgcgctgtgaccggttggattgcgcgctacgcagatcagattgatgccggtgtctatccagcagacgacaagacgattgatacccagcgtgctgcaatgcagcacctggtcgaggagagccgtgcggcgggcatcaatggcgaacttccggcgtttgtgaccaaactggccgatcgcgcagtggcagaaggtcgtggtggtgactcttacgctgcactgattgaacagtttcgcaagtcagcttaa

SEQ ID NO: 100 - protein, 292 aa, synthetic construct
  REGION 1..292: note = Imine reductase variant from Pseudonocardia spinosispora
MSDSPVPVTVLGLGLMGQALAGAFLAAGHPTTVWNRSAAKADELVGRGATLAASPAAAVAAGSLIVVCVTDHRAVRELLEPLGDALPGRVLVNLTSGTSREARENAEHTAAQGATYLDGVILTIPSGIGTPEATILYSGPRSTFDEHESALRALGPGATFVGEDHGLANLYDAAMLSVMWGLLNGFLHGTALLGTAGVSATSVVPMLGQGICAVTGWIARYADQIDAGVYPADDKTIDTQRAAMQHLVEESRAAGINGELPAFVTKLADRAVAEGRGGDSYAALIEQFRKSA

SEQ ID NO: 101 - DNA, 879 bp, synthetic construct
  misc_feature 1..879: note = Imine reductase variant from Pseudonocardia spinosispora
  source 1..879: mol_type = other DNA
atgagtgattcacctgtgcccgtgacagttctgggtcttggtctgatgggtcaggccttagcgggagcgtttctggcagccggtcaccctacgacggtttggaatcgcagcgcagctaaagctgatgaactggttggtcgcggtgcaaccctggccgcgtctcccgcggctgccgtcgcagcgggtagtctgatcgttgtttgcgtcacagatcatcgtgcggtgcgcgaactgctggaaccacttggcgatgcactgccaggtcgcgttctggtcaacctgacgagcggtacgtcgcgtgaagcccgtgagaacgcagaacatactgcggctcagggagccacctacctggatggtgtgattctgggtattccaagcggcattggcaccccagaagctaccattctgtattcgggaccgcgcagtaccttcgatgaacatgaaagcgcactgcgcgcattaggtccgggggcgacctttgtaggggaagatcacggactggctgcactgtatgatgcagcaatgctgagcgtcatgtggggcctgctgaatggtttcctgcatggaaccgcactgctgggaaccgcgggcgtttcggcaacctctgtggttccgatgctgggtcaaggtatcggagctgtgaccggttggattgcgcgctacgcagatcagattgatgccggtgtctatccagcagacgacaagacgattgatacccagcgtgctgcaatgcagcacctggtcgaggagagccgtgcggcgggcatcaatggcgaacttccggcgtttgtgaccaaactggccgatcgcgcagtggcagaaggtcgtggtggtgactcttacgctgcactgattgaacagtttcgcaagtcagcttaa

SEQ ID NO: 102 - protein, 292 aa, synthetic construct
  REGION 1..292: note = Imine reductase variant from Pseudonocardia spinosispora
MSDSPVPVTVLGLGLMGQALAGAFLAAGHPTTVWNRSAAKADELVGRGATLAASPAAAVAAGSLIVVCVTDHRAVRELLEPLGDALPGRVLVNLTSGTSREARENAEHTAAQGATYLDGVILGIPSGIGTPEATILYSGPRSTFDEHESALRALGPGATFVGEDHGLAALYDAAMLSVMWGLLNGFLHGTALLGTAGVSATSVVPMLGQGIGAVTGWIARYADQIDAGVYPADDKTIDTQRAAMQHLVEESRAAGINGELPAFVTKLADRAVAEGRGGDSYAALIEQFRKSA

SEQ ID NO: 103 - DNA, 879 bp, synthetic construct
  misc_feature 1..879: note = Imine reductase variant from Pseudonocardia spinosispora
  source 1..879: mol_type = other DNA
atgagtgattcacctgtgcccgtgacagttctgggtcttggtctgatgggtcaggccttagcgggagcgtttctggcagccggtcaccctacgacggtttggaatcgcagcgcagctaaagctgatgaactggttggtcgcggtgcaaccctggccgcgtctcccgcggctgccgtcgcagcgggtagtctgatcgttgtttgcgtcacagatcatcgtgcggtgcgcgaactgctggaaccacttggcgatgcactgccaggtcgcgttctggtcaacctgacgagcggtacgtcgcgtgaagcccgtgagaacgcagaacatactgcggctcagggagccacctacctggatggtgtgattctgacgattccaagcggcattggcaccccagaagctaccattctgtattcgggaccgcgcagtaccttcgatgaacatgaaagcgcactgcgcgcattaggtccgggggcgacctttgtaggggaagatcacggactggctgccctgtacgatattgcacacctgagcgtcatgtggggcctgctgaatggtttcctgcatggaaccgcactgctgggaaccgcgggcgtttcggcaacctctgtggttccgatgctgggtcaaggtatcgaagtggtgaccggttggattgcgcgctacgcagatcagattgatgccggtgtctatccagcagacgacgcgacgattgatacccagcgtgctgcaatgcagcacctggtcgaggagagccgtgcggcgggcatcaatggcgaacttccggcgtttgtgaccaaactggccgatcgcgcagtggcagaaggtcgtggtggtgactcttacgctgcactgattgaacagtttcgcaagtcagcttaa

SEQ ID NO: 104 - protein, 292 aa, synthetic construct
  REGION 1..292: note = Imine reductase variant from Pseudonocardia spinosispora
MSDSPVPVTVLGLGLMGQALAGAFLAAGHPTTVWNRSAAKADELVGRGATLAASPAAAVAAGSLIVVCVTDHRAVRELLEPLGDALPGRVLVNLTSGTSREARENAEHTAAQGATYLDGVILTIPSGIGTPEATILYSGPRSTFDEHESALRALGPGATFVGEDHGLAALYDIAHLSVMWGLLNGFLHGTALLGTAGVSATSVVPMLGQGIEVVTGWIARYADQIDAGVYPADDATIDTQRAAMQHLVEESRAAGINGELPAFVTKLADRAVAEGRGGDSYAALIEQFRKSA

SEQ ID NO: 105 - DNA, 879 bp, synthetic construct
  misc_feature 1..879: note = Imine reductase variant from Pseudonocardia spinosispora
  source 1..879: mol_type = other DNA
atgagtgattcacctgtgcccgtgacagttctgggtcttggtctgatgggtcaggccttagcgggagcgtttctggcagccggtcaccctacgacggtttggaatcgcagcgcagctaaagctgatgaactggttggtcgcggtgcaaccctggccgcgtctcccgcggctgccgtcgcagcgggtagtctgatcgttgtttgcgtcacagatcatcgtgcggtgcgcgaactgctggaaccacttggcgatgcactgccaggtcgcgttctggtcaacctgacgagcggtacgtcgcgtgaagcccgtgagaacgcagaacatactgcggctcagggagccacctacctggatggtgtgattctgacgattccaagcggcattggcaccccagaagctaccattctgtattcgggaccgcgcagtaccttcgatgaacatgaaagcgcactgcgcgcattaggtccgggggcgacctttgtaggggaagatcacggactggctgcactgtatgatgcagcaatgctgagcgtcatgtggggcctgctgaatggtttcctgcatggaaccgcactgctgggaaccgcgggcgtttcggcaacctctgtggttccgatgctgggtcaaggtatcgaaactgtgaccggttggattgcgcgctacgcagatcagattgatgccggtgtctatccagcagacgacaagacgattgatacccagcgtgctgcaatgcagcacctggtcgaggagagccgtgcggcgggcatcaatggcgaacttccggcgtttgtgaccaaactggccgatcgcgcagtggcagaaggtcgtggtggtgactcttacgctgcactgattgaacagtttcgcaagtcagcttaa

SEQ ID NO: 106 - protein, 292 aa, synthetic construct
  REGION 1..292: note = Imine reductase variant from Pseudonocardia spinosispora
MSDSPVPVTVLGLGLMGQALAGAFLAAGHPTTVWNRSAAKADELVGRGATLAASPAAAVAAGSLIVVCVTDHRAVRELLEPLGDALPGRVLVNLTSGTSREARENAEHTAAQGATYLDGVILTIPSGIGTPEATILYSGPRSTFDEHESALRALGPGATFVGEDHGLAALYDAAMLSVMWGLLNGFLHGTALLGTAGVSATSVVPMLGQGIETVTGWIARYADQIDAGVYPADDKTIDTQRAAMQHLVEESRAAGINGELPAFVTKLADRAVAEGRGGDSYAALIEQFRKSA

SEQ ID NO: 107 - DNA, 879 bp, synthetic construct
  misc_feature 1..879: note = Imine reductase variant from Pseudonocardia spinosispora
  source 1..879: mol_type = other DNA
atgagtgattcacctgtgcccgtgacagttctgggtcttggtctgatgggtcaggccttagcgggagcgtttctggcagccggtcaccctacgacggtttggaatcgcagcgcagctaaagctgatgaactggttggtcgcggtgcaaccctggccgcgtctcccgcggctgccgtcgcagcgggtagtctgatcgttgtttgcgtcacagatcatcgtgcggtgcgcgaactgctggaaccacttggcgatgcactgccaggtcgcgttctggtcaacctgacgagcggtacgtcgcgtgaagcccgtgagaacgcagaacatactgcggctcagggagccacctacctggatggtgtgattctgaccattccaagcggcattggcaccccagaagctaccattctgtattcgggaccgcgcagtaccttcgatgaacatgaaagcgcactgcgcgcattaggtccgggggcgacctttgtaggggaagatcacggactggctgccctgtacgatgccgcacacctgagcgtcatgtggggcctgctgaatggtttcctgcatggaaccgcactgctgggaaccgcgggcgtttcggcaacctctgtggttccgatgctgggtcaaggtatcgaacctgtgaccggttggattgcgcgctacgcagatcagattgatgccggtgtctatccagcagacgacaagacgattgatacccagcgtgctgcaatgcagcacctggtcgaggagagccgtgcggcgggcatcaatggcgaacttccggcgtttgtgaccaaactggccgatcgcgcagtggcagaaggtcgtggtggtgactcttacgctgcactgattgaacagtttcgcaagtcagcttaa

SEQ ID NO: 108 - protein, 292 aa, synthetic construct
  REGION 1..292: note = Imine reductase variant from Pseudonocardia spinosispora
MSDSPVPVTVLGLGLMGQALAGAFLAAGHPTTVWNRSAAKADELVGRGATLAASPAAAVAAGSLIVVCVTDHRAVRELLEPLGDALPGRVLVNLTSGTSREARENAEHTAAQGATYLDGVILTIPSGIGTPEATILYSGPRSTFDEHESALRALGPGATFVGEDHGLAALYDAAHLSVMWGLLNGFLHGTALLGTAGVSATSVVPMLGQGIEPVTGWIARYADQIDAGVYPADDKTIDTQRAAMQHLVEESRAAGINGELPAFVTKLADRAVAEGRGGDSYAALIEQFRKSA

SEQ ID NO: 109 - DNA, 879 bp, synthetic construct
  misc_feature 1..879: note = Imine reductase variant from Pseudonocardia spinosispora
  source 1..879: mol_type = other DNA
atgagtgattcacctgtgcccgtgacagttctgggtcttggtctgatgggtcaggccttagcgggagcgtttctggcagccggtcaccctacgacggtttggaatcgcagcgcagctaaagctgatgaactggttggtcgcggtgcaaccctggccgcgtctcccgcggctgccgtcgcagcgggtagtctgatcgttgtttgcgtcacagatcatcgtgcggtgcgcgaactgctggaaccacttggcgatgcactgccaggtcgcgttctggtcaacctgacgagcggtacgtcgcgtgaagcccgtgagaacgcagaacatactgcggctcagggagccacctacctggatggtgtgattctgacgggcccaagcggcattggcaccccagaagctaccattctgtattcgggaccgcgcagtaccttcgatgaacatgaaagcgcactgcgcgcattaggtccgggggcgacctttgtaggggaagatcacggactggctaatctgtacgatgccgcaatgctgagcgtcatgtggggcctgctgaatggtttcctgcatggaaccgcactgctgggaaccgcgggcgtttcggcaacctctgtggttccgatgctgggtcaaggtatcggagtggtgaccggttggattgcgcgctacgcagatcagattgatgccggtgtctatccagcagacgacaagacgattgatacccagcgtgctgcaatgcagcacctggtcgaggagagccgtgcggcgggcatcaatggcgaacttccggcgtttgtgaccaaactggccgatcgcgcagtggcagaaggtcgtggtggtgactcttacgctgcactgattgaacagtttcgcaagtcagcttaa

SEQ ID NO: 110 - protein, 292 aa, synthetic construct
  REGION 1..292: note = Imine reductase variant from Pseudonocardia spinosispora
MSDSPVPVTVLGLGLMGQALAGAFLAAGHPTTVWNRSAAKADELVGRGATLAASPAAAVAAGSLIVVCVTDHRAVRELLEPLGDALPGRVLVNLTSGTSREARENAEHTAAQGATYLDGVILTGPSGIGTPEATILYSGPRSTFDEHESALRALGPGATFVGEDHGLANLYDAAMLSVMWGLLNGFLHGTALLGTAGVSATSVVPMLGQGIGVVTGWIARYADQIDAGVYPADDKTIDTQRAAMQHLVEESRAAGINGELPAFVTKLADRAVAEGRGGDSYAALIEQFRKSA

SEQ ID NO: 111 - DNA, 879 bp, synthetic construct
  misc_feature 1..879: note = Imine reductase variant from Pseudonocardia spinosispora
  source 1..879: mol_type = other DNA
atgagtgattcacctgtgcccgtgacagttctgggtcttggtctgatgggtcaggccttagcgggagcgtttctggcagccggtcaccctacgacggtttggaatcgcagcgcagctaaagctgatgaactggttggtcgcggtgcaaccctggccgcgtctcccgcggctgccgtcgcagcgggtagtctgatcgttgtttgcgtcacagatcatcgtgcggtgcgcgaactgctggaaccacttggcgatgcactgccaggtcgcgttctggtcaacctgacgagcggtacgtcgcgtgaagcccgtgagaacgcagaacatactgcggctcagggagccacctacctggatggtgtgattctgacgggcccaagcggcattggcaccccagaagctaccattctgtattcgggaccgcgcagtaccttcgatgaacatgaaagcgcactgcgcgcattaggtccgggggcgacctttgtaggggaagatcacggactggctaatctgtacgatgccgcaatgctgagcgtcatgtggggcctgctgaatggtttcctgcatggaaccgcactgctgggaaccgcgggcgtttcggcaacctctgtggttccgatgctgggtcaaggtatcgtagtggtgaccggttggattgcgcgctacgcagatcagattgatgccggtgtctatccagcagacgacaagacgattgatacccagcgtgctgcaatgcagcacctggtcgaggagagccgtgcggcgggcatcaatggcgaacttccggcgtttgtgaccaaactggccgatcgcgcagtggcagaaggtcgtggtggtgactcttacgctgcactgattgaacagtttcgcaagtcagcttaa

SEQ ID NO: 112 - protein, 292 aa, synthetic construct
  REGION 1..292: note = Imine reductase variant from Pseudonocardia spinosispora
MSDSPVPVTVLGLGLMGQALAGAFLAAGHPTTVWNRSAAKADELVGRGATLAASPAAAVAAGSLIVVCVTDHRAVRELLEPLGDALPGRVLVNLTSGTSREARENAEHTAAQGATYLDGVILTGPSGIGTPEATILYSGPRSTFDEHESALRALGPGATFVGEDHGLANLYDAAMLSVMWGLLNGFLHGTALLGTAGVSATSVVPMLGQGIVVVTGWIARYADQIDAGVYPADDKTIDTQRAAMQHLVEESRAAGINGELPAFVTKLADRAVAEGRGGDSYAALIEQFRKSA

SEQ ID NO: 113 - DNA, 879 bp, synthetic construct
  misc_feature 1..879: note = Imine reductase variant from Pseudonocardia spinosispora
  source 1..879: mol_type = other DNA
atgagtgattcacctgtgcccgtgacagttctgggtcttggtctgatgggtcaggccttagcgggagcgtttctggcagccggtcaccctacgacggtttggaatcgcagcgcagctaaagctgatgaactggttggtcgcggtgcaaccctggccgcgtctcccgcggctgccgtcgcagcgggtagtctgatcgttgtttgcgtcacagatcatcgtgcggtgcgcgaactgctggaaccacttggcgatgcactgccaggtcgcgttctggtcaacctgacgagcggtacgtcgcgtgaagcccgtgagaacgcagaacatactgcggctcagggagccacctacctggatggtgtgattctgggtattccaagcggcattggcaccccagaagctaccattctgtattcgggaccgcgcagtaccttcgatgaacatgaaagcgcactgcgcgcattaggtccgggggcgacctttgtaggggaagatcacggactggctaatctgtacgatgccgcaatgctgagcgtcatgtggggcctgctgaatggtttcctgcatggaaccgcactgctgggaaccgcgggcgtttcggcaacctctgtggttccgatgctgggtcaaggtatcggagtggtgaccggttggattgcgcgctacgcagatcagattgatgccggtgtctatccagcagacgacgcgacgattgatacccagcgtgctgcaatgcagcacctggtcgaggagagccgtgcggcgggcatcaatggcgaacttccggcgtttgtgaccaaactggccgatcgcgcagtggcagaaggtcgtggtggtgactcttacgctgcactgattgaacagtttcgcaagtcagcttaa

SEQ ID NO: 114 - protein, 292 aa, synthetic construct
  REGION 1..292: note = Imine reductase variant from Pseudonocardia spinosispora
MSDSPVPVTVLGLGLMGQALAGAFLAAGHPTTVWNRSAAKADELVGRGATLAASPAAAVAAGSLIVVCVTDHRAVRELLEPLGDALPGRVLVNLTSGTSREARENAEHTAAQGATYLDGVILGIPSGIGTPEATILYSGPRSTFDEHESALRALGPGATFVGEDHGLANLYDAAMLSVMWGLLNGFLHGTALLGTAGVSATSVVPMLGQGIGVVTGWIARYADQIDAGVYPADDATIDTQRAAMQHLVEESRAAGINGELPAFVTKLADRAVAEGRGGDSYAALIEQFRKSA

SEQ ID NO: 115 - DNA, 879 bp, synthetic construct
  misc_feature 1..879: note = Imine reductase variant from Pseudonocardia spinosispora
  source 1..879: mol_type = other DNA
atgagtgattcacctgtgcccgtgacagttctgggtcttggtctgatgggtcaggccttagcgggagcgtttctggcagccggtcaccctacgacggtttggaatcgcagcgcagctaaagctgatgaactggttggtcgcggtgcaaccctggccgcgtctcccgcggctgccgtcgcagcgggtagtctgatcgttgtttgcgtcacagatcatcgtgcggtgcgcgaactgctggaaccacttggcgatgcactgccaggtcgcgttctggtcaacctgacgagcggtacgtcgcgtgaagcccgtgagaacgcagaacatactgcggctcagggagccacctacctggatggtgtgattctgacgattccaagcggcattggcaccccagaagctaccattctgtattcgggaccgcgcagtaccttcgatgaacatgaaagcgcactgcgcgcattaggtccgggggcgacctttgtaggggaagatcacggactggctgcactgtatgatgcagcaatgctgagcgtcatgtggggcctgctgaatggtttcctgcatggaaccgcactgctgggaaccgcgggcgtttcggcaacctctgtggttccgatgctgggtcaaggtatcgtagtggtgaccggttggattgcgcgctacgcagatcagattgatgccggtgtctatccagcagacgacaagacgattgatacccagcgtgctgcaatgcagcacctggtcgaggagagccgtgcggcgggcatcaatggcgaacttccggcgtttgtgaccaaactggccgatcgcgcagtggcagaaggtcgtggtggtgactcttacgctgcactgattgaacagtttcgcaagtcagcttaa

SEQ ID NO: 116 - protein, 292 aa, synthetic construct
  REGION 1..292: note = Imine reductase variant from Pseudonocardia spinosispora
MSDSPVPVTVLGLGLMGQALAGAFLAAGHPTTVWNRSAAKADELVGRGATLAASPAAAVAAGSLIVVCVTDHRAVRELLEPLGDALPGRVLVNLTSGTSREARENAEHTAAQGATYLDGVILTIPSGIGTPEATILYSGPRSTFDEHESALRALGPGATFVGEDHGLAALYDAAMLSVMWGLLNGFLHGTALLGTAGVSATSVVPMLGQGIVVVTGWIARYADQIDAGVYPADDKTIDTQRAAMQHLVEESRAAGINGELPAFVTKLADRAVAEGRGGDSYAALIEQFRKSA

SEQ ID NO: 117 - DNA, 879 bp, synthetic construct
  misc_feature 1..879: note = Imine reductase variant from Pseudonocardia spinosispora
  source 1..879: mol_type = other DNA
atgagtgattcacctgtgcccgtgacagttctgggtcttggtctgatgggtcaggccttagcgggagcgtttctggcagccggtcaccctacgacggtttggaatcgcagcgcagctaaagctgatgaactggttggtcgcggtgcaaccctggccgcgtctcccgcggctgccgtcgcagcgggtagtctgatcgttgtttgcgtcacagatcatcgtgcggtgcgcgaactgctggaaccacttggcgatgcactgccaggtcgcgttctggtcaacctgacgagcggtacgtcgcgtgaagcccgtgagaacgcagaacatactgcggctcagggagccacctacctggatggtgtgattctgggtattccaagcggcattggcaccccagaagctaccattctgtattcgggaccgcgcagtaccttcgatgaacatgaaagcgcactgcgcgcattaggtccgggggcgacctttgtaggggaagatcacggactggctgcactgtatgatgcagcaatgctgagcgtcatgtggggcctgctgaatggtttcctgcatggaaccgcactgctgggaaccgcgggcgtttcggcaacctctgtggttccgatgctgggtcaaggtatctgcgtggtgaccggttggattgcgcgctacgcagatcagattgatgccggtgtctatccagcagacgacaagacgattgatacccagcgtgctgcaatgcagcacctggtcgaggagagccgtgcggcgggcatcaatggcgaacttccggcgtttgtgaccaaactggccgatcgcgcagtggcagaaggtcgtggtggtgactcttacgctgcactgattgaacagtttcgcaagtcagcttaa

SEQ ID NO: 118 - protein, 292 aa, synthetic construct
  REGION 1..292: note = Imine reductase variant from Pseudonocardia spinosispora
MSDSPVPVTVLGLGLMGQALAGAFLAAGHPTTVWNRSAAKADELVGRGATLAASPAAAVAAGSLIVVCVTDHRAVRELLEPLGDALPGRVLVNLTSGTSREARENAEHTAAQGATYLDGVILGIPSGIGTPEATILYSGPRSTFDEHESALRALGPGATFVGEDHGLAALYDAAMLSVMWGLLNGFLHGTALLGTAGVSATSVVPMLGQGICVVTGWIARYADQIDAGVYPADDKTIDTQRAAMQHLVEESRAAGINGELPAFVTKLADRAVAEGRGGDSYAALIEQFRKSA

SEQ ID NO: 119 - DNA, 879 bp, synthetic construct
  misc_feature 1..879: note = Imine reductase variant from Pseudonocardia spinosispora
  source 1..879: mol_type = other DNA
atgagtgattcacctgtgcccgtgacagttctgggtcttggtctgatgggtcaggccttagcgggagcgtttctggcagccggtcaccctacgacggtttggaatcgcagcgcagctaaagctgatgaactggttggtcgcggtgcaaccctggccgcgtctcccgcggctgccgtcgcagcgggtagtctgatcgttgtttgcgtcacagatcatcgtgcggtgcgcgaactgctggaaccacttggcgatgcactgccaggtcgcgttctggtcaacctgacgagcggtacgtcgcgtgaagcccgtgagaacgcagaacatactgcggctcagggagccacctacctggatggtgtgattctgggtattccaagcggcattggcaccccagaagctaccattctgtattcgggaccgcgcagtaccttcgatgaacatgaaagcgcactgcgcgcattaggtccgggggcgacctttgtaggggaagatcacggactggctaatctggttgatcatgcaatgctgagcgtcatgtggggcctgctgaatggtttcctgcatggaaccgcactgctgggaaccgcgggcgtttcggcaacctctgtggttccgatgctgggtcaaggtatcgaagtggtgaccggttggattgcgcgctacgcagatcagattgatgccggtgtctatccagcagacgacaagacgattgatacccagcgtgctgcaatgcagcacctggtcgaggagagccgtgcggcgggcatcaatggcgaacttccggcgtttgtgaccaaactggccgatcgcgcagtggcagaaggtcgtggtggtgactcttacgctgcactgattgaacagtttcgcaagtcagcttaa

SEQ ID NO: 120 - protein, 292 aa, synthetic construct
  REGION 1..292: note = Imine reductase variant from Pseudonocardia spinosispora
MSDSPVPVTVLGLGLMGQALAGAFLAAGHPTTVWNRSAAKADELVGRGATLAASPAAAVAAGSLIVVCVTDHRAVRELLEPLGDALPGRVLVNLTSGTSREARENAEHTAAQGATYLDGVILGIPSGIGTPEATILYSGPRSTFDEHESALRALGPGATFVGEDHGLANLVDHAMLSVMWGLLNGFLHGTALLGTAGVSATSVVPMLGQGIEVVTGWIARYADQIDAGVYPADDKTIDTQRAAMQHLVEESRAAGINGELPAFVTKLADRAVAEGRGGDSYAALIEQFRKSA

SEQ ID NO: 121 - DNA, 879 bp, synthetic construct
  misc_feature 1..879: note = Imine reductase variant from Pseudonocardia spinosispora
  source 1..879: mol_type = other DNA
atgagtgattcacctgtgcccgtgacagttctgggtcttggtctgatgggtcaggccttagcgggagcgtttctggcagccggtcaccctacgacggtttggaatcgcagcgcagctaaagctgatgaactggttggtcgcggtgcaaccctggccgcgtctcccgcggctgccgtcgcagcgggtagtctgatcgttgtttgcgtcacagatcatcgtgcggtgcgcgaactgctggaaccacttggcgatgcactgccaggtcgcgttctggtcaacctgacgagcggtacgtcgcgtgaagcccgtgagaacgcagaacatactgcggctcagggagccacctacctggatggtgtgattctgacgggcccaagcggcattggcaccccagaagctaccattctgtattcgggaccgcgcagtaccttcgatgaacatgaaagcgcactgcgcgcattaggtccgggggcgacctttgtaggggaagatcacggactggctgcactgtatgatgcagcaatgctgagcgtcatgtggggcctgctgaatggtttcctgcatggaaccgcactgctgggaaccgcgggcgtttcggcaacctctgtggttccgatgctgggtcaaggtatctgcgtggtgaccggttggattgcgcgctacgcagatcagattgatgccggtgtctatccagcagacgacaagacgattgatacccagcgtgctgcaatgcagcacctggtcgaggagagccgtgcggcgggcatcaatggcgaacttccggcgtttgtgaccaaactggccgatcgcgcagtggcagaaggtcgtggtggtgactcttacgctgcactgattgaacagtttcgcaagtcagcttaa

SEQ ID NO: 122 - protein, 292 aa, synthetic construct
  REGION 1..292: note = Imine reductase variant from Pseudonocardia spinosispora
MSDSPVPVTVLGLGLMGQALAGAFLAAGHPTTVWNRSAAKADELVGRGATLAASPAAAVAAGSLIVVCVTDHRAVRELLEPLGDALPGRVLVNLTSGTSREARENAEHTAAQGATYLDGVILTGPSGIGTPEATILYSGPRSTFDEHESALRALGPGATFVGEDHGLAALYDAAMLSVMWGLLNGFLHGTALLGTAGVSATSVVPMLGQGICVVTGWIARYADQIDAGVYPADDKTIDTQRAAMQHLVEESRAAGINGELPAFVTKLADRAVAEGRGGDSYAALIEQFRKSA

SEQ ID NO: 123 - DNA, 879 bp, synthetic construct
  misc_feature 1..879: note = Imine reductase variant from Pseudonocardia spinosispora
  source 1..879: mol_type = other DNA
atgagtgattcacctgtgcccgtgacagttctgggtcttggtctgatgggtcaggccttagcgggagcgtttctggcagccggtcaccctacgacggtttggaatcgcagcgcagctaaagctgatgaactggttggtcgcggtgcaaccctggccgcgtctcccgcggctgccgtcgcagcgggtagtctgatcgttgtttgcgtcacagatcatcgtgcggtgcgcgaactgctggaaccacttggcgatgcactgccaggtcgcgttctggtcaacctgacgagcggtacgtcgcgtgaagcccgtgagaacgcagaacatactgcggctcagggagccacctacctggatggtgtgattctgacgggcccaagcggcattggcaccccagaagctaccattctgtattcgggaccgcgcagtaccttcgatgaacatgaaagcgcactgcgcgcattaggtccgggggcgacctttgtaggggaagatcacggactggctaatctgtacgatattgcaatgctgagcgtcatgtggggcctgctgaatggtttcctgcatggaaccgcactgctgggaaccgcgggcgtttcggcaacctctgtggttccgatgctgggtcaaggtatcgtagtggtgaccggttggattgcgcgctacgcagatcagattgatgccggtgtctatccagcagacgacaagacgattgatacccagcgtgctgcaatgcagcacctggtcgaggagagccgtgcggcgggcatcaatggcgaacttccggcgtttgtgaccaaactggccgatcgcgcagtggcagaaggtcgtggtggtgactcttacgctgcactgattgaacagtttcgcaagtcagcttaa

SEQ ID NO: 124 - protein, 292 aa, synthetic construct
  REGION 1..292: note = Imine reductase variant from Pseudonocardia spinosispora
MSDSPVPVTVLGLGLMGQALAGAFLAAGHPTTVWNRSAAKADELVGRGATLAASPAAAVAAGSLIVVCVTDHRAVRELLEPLGDALPGRVLVNLTSGTSREARENAEHTAAQGATYLDGVILTGPSGIGTPEATILYSGPRSTFDEHESALRALGPGATFVGEDHGLANLYDIAMLSVMWGLLNGFLHGTALLGTAGVSATSVVPMLGQGIVVVTGWIARYADQIDAGVYPADDKTIDTQRAAMQHLVEESRAAGINGELPAFVTKLADRAVAEGRGGDSYAALIEQFRKSA

SEQ ID NO: 125 - DNA, 879 bp, synthetic construct
  misc_feature 1..879: note = Imine reductase variant from Pseudonocardia spinosispora
  source 1..879: mol_type = other DNA
atgagtgattcacctgtgcccgtgacagttctgggtcttggtctgatgggtcaggccttagcgggagcgtttctggcagccggtcaccctacgacggtttggaatcgcagcgcagctaaagctgatgaactggttggtcgcggtgcaaccctggccgcgtctcccgcggctgccgtcgcagcgggtagtctgatcgttgtttgcgtcacagatcatcgtgcggtgcgcgaactgctggaaccacttggcgatgcactgccaggtcgcgttctggtcaacctgacgagcggtacgtcgcgtgaagcccgtgagaacgcagaacatactgcggctcagggagccacctacctggatggtgtgattctgggtattccaagcggcattggcaccccagaagctaccattctgtattcgggaccgcgcagtaccttcgatgaacatgaaagcgcactgcgcgcattaggtccgggggcgacctttgtaggggaagatcacggactggctaatctgtacgatattgcaatgctgagcgtcatgtggggcctgctgaatggtttcctgcatggaaccgcactgctgggaaccgcgggcgtttcggcaacctctgtggttccgatgctgggtcaaggtatcgaagcggtgaccggttggattgcgcgctacgcagatcagattgatgccggtgtctatccagcagacgacgcgacgattgatacccagcgtgctgcaatgcagcacctggtcgaggagagccgtgcggcgggcatcaatggcgaacttccggcgtttgtgaccaaactggccgatcgcgcagtggcagaaggtcgtggtggtgactcttacgctgcactgattgaacagtttcgcaagtcagcttaa

SEQ ID NO: 126 - protein, 292 aa, synthetic construct
  REGION 1..292: note = Imine reductase variant from Pseudonocardia spinosispora
MSDSPVPVTVLGLGLMGQALAGAFLAAGHPTTVWNRSAAKADELVGRGATLAASPAAAVAAGSLIVVCVTDHRAVRELLEPLGDALPGRVLVNLTSGTSREARENAEHTAAQGATYLDGVILGIPSGIGTPEATILYSGPRSTFDEHESALRALGPGATFVGEDHGLANLYDIAMLSVMWGLLNGFLHGTALLGTAGVSATSVVPMLGQGIEAVTGWIARYADQIDAGVYPADDATIDTQRAAMQHLVEESRAAGINGELPAFVTKLADRAVAEGRGGDSYAALIEQFRKSA

SEQ ID NO: 127 - DNA, 879 bp, synthetic construct
  misc_feature 1..879: note = Imine reductase variant from Pseudonocardia spinosispora
  source 1..879: mol_type = other DNA
atgagtgattcacctgtgcccgtgacagttctgggtcttggtctgatgggtcaggccttagcgggagcgtttctggcagccggtcaccctacgacggtttggaatcgcagcgcagctaaagctgatgaactggttggtcgcggtgcaaccctggccgcgtctcccgcggctgccgtcgcagcgggtagtctgatcgttgtttgcgtcacagatcatcgtgcggtgcgcgaactgctggaaccacttggcgatgcactgccaggtcgcgttctggtcaacctgacgagcggtacgtcgcgtgaagcccgtgagaacgcagaacatactgcggctcagggagccacctacctggatggtgtgattctgacgattccaagcggcattggcaccccagaagctaccattctgtattcgggaccgcgcagtaccttcgatgaacatgaaagcgcactgcgcgcattaggtccgggggcgacctttgtaggggaagatcacggactggctaatctgtacgatgccgcaatgctgagcgtcatgtggggcctgctgaatggtttcctgcatggaaccgcactgctgggaaccgcgggcgtttcggcaacctctgtggttccgatgctgggtcaaggtatctgcgtggtgaccggttggattgcgcgctacgcagatcagattgatgccggtgtctatccagcagacgacaagacgattgatacccagcgtgctgcaatgcagcacctggtcgaggagagccgtgcggcgggcatcaatggcgaacttccggcgtttgtgaccaaactggccgatcgcgcagtggcagaaggtcgtggtggtgactcttacgctgcactgattgaacagtttcgcaagtcagcttaa

SEQ ID NO: 128 - protein, 292 aa, synthetic construct
  REGION 1..292: note = Imine reductase variant from Pseudonocardia spinosispora
MSDSPVPVTVLGLGLMGQALAGAFLAAGHPTTVWNRSAAKADELVGRGATLAASPAAAVAAGSLIVVCVTDHRAVRELLEPLGDALPGRVLVNLTSGTSREARENAEHTAAQGATYLDGVILTIPSGIGTPEATILYSGPRSTFDEHESALRALGPGATFVGEDHGLANLYDAAMLSVMWGLLNGFLHGTALLGTAGVSATSVVPMLGQGICVVTGWIARYADQIDAGVYPADDKTIDTQRAAMQHLVEESRAAGINGELPAFVTKLADRAVAEGRGGDSYAALIEQFRKSA

SEQ ID NO: 129 - DNA, 879 bp, synthetic construct
  misc_feature 1..879: note = Imine reductase variant from Pseudonocardia spinosispora
  misc_feature 634: note = Misc_Feature - n = a, c, g or t
  misc_feature 636: note = Misc_Feature - n = a, c, g or t
  source 1..879: mol_type = other DNA
atgagtgattcacctgtgcccgtgacagttctgggtcttggtctgatgggtcaggccttagcgggagcgtttctggcagccggtcaccctacgacggtttggaatcgcagcgcagctaaagctgatgaactggttggtcgcggtgcaaccctggccgcgtctcccgcggctgccgtcgcagcgggtagtctgatcgttgtttgcgtcacagatcatcgtgcggtgcgcgaactgctggaaccacttggcgatgcactgccaggtcgcgttctggtcaacctgacgagcggtacgtcgcgtgaagcccgtgagaacgcagaacatactgcggctcagggagccacctacctggatggtgtgattctgggtattccaagcggcattggcaccccagaagctaccattctgtattcgggaccgcgcagtaccttcgatgaacatgaaagcgcactgcgcgcattaggtccgggggcgacctttgtaggggaagatcacggactggctaatctggttgatcatgcacacctgagcgtcatgtggggcctgctgaatggtttcctgcatggaaccgcactgctgggaaccgcgggcgtttcggcaacctctgtggttccgatgctgggtcaaggtatcngngtggtgaccggttggattgcgcgctacgcagatcagattgatgccggtgtctatccagcagacgacgccacgattgatacccagcgtgctgcaatgcagcacctggtcgaggagagccgtgcggcgggcatcaatggcgaacttccggcgtttgtgaccaaactggccgatcgcgcagtggcagaaggtcgtggtggtgactcttacgctgcactgattgaacagtttcgcaagtcagcttaa

SEQ ID NO: 130 - protein, 292 aa, synthetic construct
  REGION 1..292: note = Imine reductase variant from Pseudonocardia spinosispora
  SITE 212: note = Misc_Feature - Xaa = Cys, Ter, Ser, Trp, Arg, Gly
MSDSPVPVTVLGLGLMGQALAGAFLAAGHPTTVWNRSAAKADELVGRGATLAASPAAAVAAGSLIVVCVTDHRAVRELLEPLGDALPGRVLVNLTSGTSREARENAEHTAAQGATYLDGVILGIPSGIGTPEATILYSGPRSTFDEHESALRALGPGATFVGEDHGLANLVDHAHLSVMWGLLNGFLHGTALLGTAGVSATSVVPMLGQGIXVVTGWIARYADQIDAGVYPADDATIDTQRAAMQHLVEESRAAGINGELPAFVTKLADRAVAEGRGGDSYAALIEQFRKSA

SEQ ID NO: 131 - DNA, 879 bp, synthetic construct
  misc_feature 1..879: note = Imine reductase variant from Pseudonocardia spinosispora
  source 1..879: mol_type = other DNA
atgagtgattcacctgtgcccgtgacagttctgggtcttggtctgatgggtcaggccttagcgggagcgtttctggcagccggtcaccctacgacggtttggaatcgcagcgcagctaaagctgatgaactggttggtcgcggtgcaaccctggccgcgtctcccgcggctgccgtcgcagcgggtagtctgatcgttgtttgcgtcacagatcatcgtgcggtgcgcgaactgctggaaccacttggcgatgcactgccaggtcgcgttctggtcaacctgacgagcggtacgtcgcgtgaagcccgtgagaacgcagaacatactgcggctcagggagccacctacctggatggtgtgattctgggtattccaagcggcattggcaccccagaagctaccattctgtattcgggaccgcgcagtaccttcgatgaacatgaaagcgcactgcgcgcattaggtccgggggcgacctttgtaggggaagatcacggactggctgcactgtatgatgcagcaatgctgagcgtcatgtggggcctgctgaatggtttcctgcatggaaccgcactgctgggaaccgcgggcgtttcggcaacctctgtggttccgatgctgggtcaaggtatcgaaactgtgaccggttggattgcgcgctacgcagatcagattgatgccggtgtctatccagcagacgacgccacgattgatacccagcgtgctgcaatgcagcacctggtcgaggagagccgtgcggcgggcatcaatggcgaacttccggcgtttgtgaccaaactggccgatcgcgcagtggcagaaggtcgtggtggtgactcttacgctgcactgattgaacagtttcgcaagtcagcttaa

SEQ ID NO: 132 - protein, 292 aa, synthetic construct
  REGION 1..292: note = Imine reductase variant from Pseudonocardia spinosispora
MSDSPVPVTVLGLGLMGQALAGAFLAAGHPTTVWNRSAAKADELVGRGATLAASPAAAVAAGSLIVVCVTDHRAVRELLEPLGDALPGRVLVNLTSGTSREARENAEHTAAQGATYLDGVILGIPSGIGTPEATILYSGPRSTFDEHESALRALGPGATFVGEDHGLAALYDAAMLSVMWGLLNGFLHGTALLGTAGVSATSVVPMLGQGIETVTGWIARYADQIDAGVYPADDATIDTQRAAMQHLVEESRAAGINGELPAFVTKLADRAVAEGRGGDSYAALIEQFRKSA

SEQ ID NO: 133 - DNA, 879 bp, synthetic construct
  misc_feature 1..879: note = Imine reductase variant from Pseudonocardia spinosispora
  source 1..879: mol_type = other DNA
atgagtgattcacctgtgcccgtgacagttctgggtcttggtctgatgggtcaggccttagcgggagcgtttctggcagccggtcaccctacgacggtttggaatcgcagcgcagctaaagctgatgaactggttggtcgcggtgcaaccctggccgcgtctcccgcggctgccgtcgcagcgggtagtctgatcgttgtttgcgtcacagatcatcgtgcggtgcgcgaactgctggaaccacttggcgatgcactgccaggtcgcgttctggtcaacctgacgagcggtacgtcgcgtgaagcccgtgagaacgcagaacatactgcggctcagggagccacctacctggatggtgtgattctgggtattccaagcggcattggcaccccagaagctaccattctgtattcgggaccgcgcagtaccttcgatgaacatgaaagcgcactgcgcgcattaggtccgggggcgacctttgtaggggaagatcacggactggctaatctgtacgatgccgcaatgctgagcgtcatgtggggcctgctgaatggtttcctgcatggaaccgcactgctgggaaccgcgggcgtttcggcaacctctgtggttccgatgctgggtcaaggtatcggagtggtgaccggttggattgcgcgctacgcagatcagattgatgccggtgtctatccagcagacgacaagacgattgatacccagcgtgctgcaatgcagcacctggtcgaggagagccgtgcggcgggcatcaatggcgaacttccggcgtttgtgaccaaactggccgatcgcgcagtggcagaaggtcgtggtggtgactcttacgctgcactgattgaacagtttcgcaagtcagcttaa

SEQ ID NO: 134 - protein, 292 aa, synthetic construct
  REGION 1..292: note = Imine reductase variant from Pseudonocardia spinosispora
MSDSPVPVTVLGLGLMGQALAGAFLAAGHPTTVWNRSAAKADELVGRGATLAASPAAAVAAGSLIVVCVTDHRAVRELLEPLGDALPGRVLVNLTSGTSREARENAEHTAAQGATYLDGVILGIPSGIGTPEATILYSGPRSTFDEHESALRALGPGATFVGEDHGLANLYDAAMLSVMWGLLNGFLHGTALLGTAGVSATSVVPMLGQGIGVVTGWIARYADQIDAGVYPADDKTIDTQRAAMQHLVEESRAAGINGELPAFVTKLADRAVAEGRGGDSYAALIEQFRKSA

SEQ ID NO: 135 - DNA, 879 bp, synthetic construct
  misc_feature 1..879: note = Imine reductase variant from Pseudonocardia spinosispora
  source 1..879: mol_type = other DNA
atgagtgattcacctgtgcccgtgacagttctgggtcttggtctgatgggtcaggccttagcgggagcgtttctggcagccggtcaccctacgacggtttggaatcgcagcgcagctaaagctgatgaactggttggtcgcggtgcaaccctggccgcgtctcccgcggctgccgtcgcagcgggtagtctgatcgttgtttgcgtcacagatcatcgtgcggtgcgcgaactgctggaaccacttggcgatgcactgccaggtcgcgttctggtcaacctgacgagcggtacgtcgcgtgaagcccgtgagaacgcagaacatactgcggctcagggagccacctacctggatggtgtgattctgggtggcccaagcggcattggcaccccagaagctaccattctgtattcgggaccgcgcagtaccttcgatgaacatgaaagcgcactgcgcgcattaggtccgggggcgacctttgtaggggaagatcacggactggctaatctgtacgatgccgcaatgctgagcgtcatgtggggcctgctgaatggtttcctgcatggaaccgcactgctgggaaccgcgggcgtttcggcaacctctgtggttccgatgctgggtcaaggtatcgtagtggtgaccggttggattgcgcgctacgcagatcagattgatgccggtgtctatccagcagacgacaagacgattgatacccagcgtgctgcaatgcagcacctggtcgaggagagccgtgcggcgggcatcaatggcgaacttccggcgtttgtgaccaaactggccgatcgcgcagtggcagaaggtcgtggtggtgactcttacgctgcactgattgaacagtttcgcaagtcagcttaa

SEQ ID NO: 136 - protein, 292 aa, synthetic construct
  REGION 1..292: note = Imine reductase variant from Pseudonocardia spinosispora
MSDSPVPVTVLGLGLMGQALAGAFLAAGHPTTVWNRSAAKADELVGRGATLAASPAAAVAAGSLIVVCVTDHRAVRELLEPLGDALPGRVLVNLTSGTSREARENAEHTAAQGATYLDGVILGGPSGIGTPEATILYSGPRSTFDEHESALRALGPGATFVGEDHGLANLYDAAMLSVMWGLLNGFLHGTALLGTAGVSATSVVPMLGQGIVVVTGWIARYADQIDAGVYPADDKTIDTQRAAMQHLVEESRAAGINGELPAFVTKLADRAVAEGRGGDSYAALIEQFRKSA

SEQ ID NO: 137 - DNA, 879 bp, synthetic construct
  misc_feature 1..879: note = Imine reductase variant from Pseudonocardia spinosispora
  source 1..879: mol_type = other DNA
atgagtgattcacctgtgcccgtgacagttctgggtcttggtctgatgggtcaggccttagcgggagcgtttctggcagccggtcaccctacgacggtttggaatcgcagcgcagctaaagctgatgaactggttggtcgcggtgcaaccctggccgcgtctcccgcggctgccgtcgcagcgggtagtctgatcgttgtttgcgtcacagatcatcgtgcggtgcgcgaactgctggaaccacttggcgatgcactgccaggtcgcgttctggtcaacctgacgagcggtacgtcgcgtgaagcccgtgagaacgcagaacatactgcggctcagggagccacctacctggatggtgtgattctgaccattccaagcggcattggcaccccagaagctaccattctgtattcgggaccgcgcagtaccttcgatgaacatgaaagcgcactgcgcgcattaggtccgggggcgacctttgtaggggaagatcacggactggctgcactgtatgatgcagcaatgctgagcgtcatgtggggcctgctgaatggtttcctgcatggaaccgcactgctgggaaccgcgggcgtttcggcaacctctgtggttccgatgctgggtcaaggtatcgaagtggtgaccggttggattgcgcgctacgcagatcagattgatgccggtgtctatccagcagacgacaagacgattgatacccagcgtgctgcaatgcagcacctggtcgaggagagccgtgcggcgggcatcaatggcgaacttccggcgtttgtgaccaaactggccgatcgcgcagtggcagaaggtcgtggtggtgactcttacgctgcactgattgaacagtttcgcaagtcagcttaa

SEQ ID NO: 138 - protein, 292 aa, synthetic construct
  REGION 1..292: note = Imine reductase variant from Pseudonocardia spinosispora
MSDSPVPVTVLGLGLMGQALAGAFLAAGHPTTVWNRSAAKADELVGRGATLAASPAAAVAAGSLIVVCVTDHRAVRELLEPLGDALPGRVLVNLTSGTSREARENAEHTAAQGATYLDGVILTIPSGIGTPEATILYSGPRSTFDEHESALRALGPGATFVGEDHGLAALYDAAMLSVMWGLLNGFLHGTALLGTAGVSATSVVPMLGQGIEVVTGWIARYADQIDAGVYPADDKTIDTQRAAMQHLVEESRAAGINGELPAFVTKLADRAVAEGRGGDSYAALIEQFRKSA

SEQ ID NO: 139 - DNA, 879 bp, synthetic construct
  misc_feature 1..879: note = Imine reductase variant from Pseudonocardia spinosispora
  source 1..879: mol_type = other DNA
atgagtgattcacctgtgcccgtgacagttctgggtcttggtctgatgggtcaggccttagcgggagcgtttctggcagccggtcaccctacgacggtttggaatcgcagcgcagctaaagctgatgaactggttggtcgcggtgcaaccctggccgcgtctcccgcggctgccgtcgcagcgggtagtctgatcgttgtttgcgtcacagatcatcgtgcggtgcgcgaactgctggaaccacttggcgatgcactgccaggtcgcgttctggtcaacctgacgagcggtacgtcgcgtgaagcccgtgagaacgcagaacatactgcggctcagggagccacctacctggatggtgtgattctgacgattccaagcggcattggcaccccagaagctaccattctgtattcgggaccgcgcagtaccttcgatgaacatgaaagcgcactgcgcgcattaggtccgggggcgacctttgtaggggaagatcacggactggctgcactgtatgatgcagcaatgctgagcgtcatgtggggcctgctgaatggtttcctgcatggaaccgcactgctgggaaccgcgggcgtttcggcaacctctgtggttccgatgctgggtcaaggtatcggagtggtgaccggttggattgcgcgctacgcagatcagattgatgccggtgtctatccagcagacgacaagacgattgatacccagcgtgctgcaatgcagcacctggtcgaggagagccgtgcggcgggcatcaatggcgaacttccggcgtttgtgaccaaactggccgatcgcgcagtggcagaaggtcgtggtggtgactcttacgctgcactgattgaacagtttcgcaagtcagcttaa

SEQ ID NO: 140 - protein, 292 aa, synthetic construct
  REGION 1..292: note = Imine reductase variant from Pseudonocardia spinosispora
MSDSPVPVTVLGLGLMGQALAGAFLAAGHPTTVWNRSAAKADELVGRGATLAASPAAAVAAGSLIVVCVTDHRAVRELLEPLGDALPGRVLVNLTSGTSREARENAEHTAAQGATYLDGVILTIPSGIGTPEATILYSGPRSTFDEHESALRALGPGATFVGEDHGLAALYDAAMLSVMWGLLNGFLHGTALLGTAGVSATSVVPMLGQGIGVVTGWIARYADQIDAGVYPADDKTIDTQRAAMQHLVEESRAAGINGELPAFVTKLADRAVAEGRGGDSYAALIEQFRKSA

SEQ ID NO: 141 - DNA, 879 bp, synthetic construct
  misc_feature 1..879: note = Imine reductase variant from Pseudonocardia spinosispora
  source 1..879: mol_type = other DNA
atgagtgattcacctgtgcccgtgacagttctgggtcttggtctgatgggtcaggccttagcgggagcgtttctggcagccggtcaccctacgacggtttggaatcgcagcgcagctaaagctgatgaactggttggtcgcggtgcaaccctggccgcgtctcccgcggctgccgtcgcagcgggtagtctgatcgttgtttgcgtcacagatcatcgtgcggtgcgcgaactgctggaaccacttggcgatgcactgccaggtcgcgttctggtcaacctgacgagcggtacgtcgcgtgaagcccgtgagaacgcagaacatactgcggctcagggagccacctacctggatggtgtgattctgacgggcccaagcggcattggcaccccagaagctaccattctgtattcgggaccgcgcagtaccttcgatgaacatgaaagcgcactgcgcgcattaggtccgggggcgacctttgtaggggaagatcacggactggctaatctgtacgatattgcaatgctgagcgtcatgtggggcctgctgaatggtttcctgcatggaaccgcactgctgggaaccgcgggcgtttcggcaacctctgtggttccgatgctgggtcaaggtatctgcgtggtgaccggttggattgcgcgctacgcagatcagattgatgccggtgtctatccagcagacgacgccacgattgatacccagcgtgctgcaatgcagcacctggtcgaggagagccgtgcggcgggcatcaatggcgaacttccggcgtttgtgaccaaactggccgatcgcgcagtggcagaaggtcgtggtggtgactcttacgctgcactgattgaacagtttcgcaagtcagcttaa

SEQ ID NO: 142 - protein, 292 aa, synthetic construct
  REGION 1..292: note = Imine reductase variant from Pseudonocardia spinosispora
MSDSPVPVTVLGLGLMGQALAGAFLAAGHPTTVWNRSAAKADELVGRGATLAASPAAAVAAGSLIVVCVTDHRAVRELLEPLGDALPGRVLVNLTSGTSREARENAEHTAAQGATYLDGVILTGPSGIGTPEATILYSGPRSTFDEHESALRALGPGATFVGEDHGLANLYDIAMLSVMWGLLNGFLHGTALLGTAGVSATSVVPMLGQGICVVTGWIARYADQIDAGVYPADDATIDTQRAAMQHLVEESRAAGINGELPAFVTKLADRAVAEGRGGDSYAALIEQFRKSA

SEQ ID NO: 143 - DNA, 879 bp, synthetic construct
  misc_feature 1..879: note = Imine reductase variant from Pseudonocardia spinosispora
  source 1..879: mol_type = other DNA
atgagtgattcacctgtgcccgtgacagttctgggtcttggtctgatgggtcaggccttagcgggagcgtttctggcagccggtcaccctacgacggtttggaatcgcagcgcagctaaagctgatgaactggttggtcgcggtgcaaccctggccgcgtctcccgcggctgccgtcgcagcgggtagtctgatcgttgtttgcgtcacagatcatcgtgcggtgcgcgaactgctggaaccacttggcgatgcactgccaggtcgcgttctggtcaacctgacgagcggtacgtcgcgtgaagcccgtgagaacgcagaacatactgcggctcagggagccacctacctggatggtgtgattctgggtattccaagcggcattggcaccccagaagctaccattctgtattcgggaccgcgcagtaccttcgatgaacatgaaagcgcactgcgcgcattaggtccgggggcgacctttgtaggggaagatcacggactggctaatctggttgatattgcaatgctgagcgtcatgtggggcctgctgaatggtttcctgcatggaaccgcactgctgggaaccgcgggcgtttcggcaacctctgtggttccgatgctgggtcaaggtatctgcgtggtgaccggttggattgcgcgctacgcagatcagattgatgccggtgtctatccagcagacgacaagacgattgatacccagcgtgctgcaatgcagcacctggtcgaggagagccgtgcggcgggcatcaatggcgaacttccggcgtttgtgaccaaactggccgatcgcgcagtggcagaaggtcgtggtggtgactcttacgctgcactgattgaacagtttcgcaagtcagcttaa

SEQ ID NO: 144 - protein, 292 aa, synthetic construct
  REGION 1..292: note = Imine reductase variant from Pseudonocardia spinosispora
MSDSPVPVTVLGLGLMGQALAGAFLAAGHPTTVWNRSAAKADELVGRGATLAASPAAAVAAGSLIVVCVTDHRAVRELLEPLGDALPGRVLVNLTSGTSREARENAEHTAAQGATYLDGVILGIPSGIGTPEATILYSGPRSTFDEHESALRALGPGATFVGEDHGLANLVDIAMLSVMWGLLNGFLHGTALLGTAGVSATSVVPMLGQGICVVTGWIARYADQIDAGVYPADDKTIDTQRAAMQHLVEESRAAGINGELPAFVTKLADRAVAEGRGGDSYAALIEQFRKSA

SEQ ID NO: 145 - DNA, 879 bp, synthetic construct
  misc_feature 1..879: note = Imine reductase variant from Pseudonocardia spinosispora
  source 1..879: mol_type = other DNA
atgagtgattcacctgtgcccgtgacagttctgggtcttggtctgatgggtcaggccttagcgggagcgtttctggcagccggtcaccctacgacggtttggaatcgcagcgcagctaaagctgatgaactggttggtcgcggtgcaaccctggccgcgtctcccgcggctgccgtcgcagcgggtagtctgatcgttgtttgcgtcacagatcatcgtgcggtgcgcgaactgctggaaccacttggcgatgcactgccaggtcgcgttctggtcaacctgacgagcggtacgtcgcgtgaagcccgtgagaacgcagaacatactgcggctcagggagccacctacctggatggtgtgattctgacggccccaagcggcattggcaccccagaagctaccattctgtattcgggaccgcgcagtaccttcgatgaacatgaaagcgcactgcgcgcattaggtccgggggcgacctttgtaggggaagatcacggactggctaatctgtacgatattgcacacctgagcgtcatgtggggcctgctgaatggtttcctgcatggaaccgcactgctgggaaccgcgggcgtttcggcaacctctgtggttccgatgctgggtcaaggtatcggagtggtgaccggttggattgcgcgctacgcagatcagattgatgccggtgtctatccagcagacgacgcgacgattgatacccagcgtgctgcaatgcagcacctggtcgaggagagccgtgcggcgggcatcaatggcgaacttccggcgtttgtgaccaaactggccgatcgcgcagtggcagaaggtcgtggtggtgactcttacgctgcactgattgaacagtttcgcaagtcagcttaa

SEQ ID NO: 146 - protein, 292 aa, synthetic construct
  REGION 1..292: note = Imine reductase variant from Pseudonocardia spinosispora
MSDSPVPVTVLGLGLMGQALAGAFLAAGHPTTVWNRSAAKADELVGRGATLAASPAAAVAAGSLIVVCVTDHRAVRELLEPLGDALPGRVLVNLTSGTSREARENAEHTAAQGATYLDGVILTAPSGIGTPEATILYSGPRSTFDEHESALRALGPGATFVGEDHGLANLYDIAHLSVMWGLLNGFLHGTALLGTAGVSATSVVPMLGQGIGVVTGWIARYADQIDAGVYPADDATIDTQRAAMQHLVEESRAAGINGELPAFVTKLADRAVAEGRGGDSYAALIEQFRKSA

SEQ ID NO: 147 - DNA, 879 bp, synthetic construct
  misc_feature 1..879: note = Imine reductase variant from Pseudonocardia spinosispora
  source 1..879: mol_type = other DNA
atgagtgattcacctgtgcccgtgacagttctgggtcttggtctgatgggtcaggccttagcgggagcgtttctggcagccggtcaccctacgacggtttggaatcgcagcgcagctaaagctgatgaactggttggtcgcggtgcaaccctggccgcgtctcccgcggctgccgtcgcagcgggtagtctgatcgttgtttgcgtcacagatcatcgtgcggtgcgcgaactgctggaaccacttggcgatgcactgccaggtcgcgttctggtcaacctgacgagcggtacgtcgcgtgaagcccgtgagaacgcagaacatactgcggctcagggagccacctacctggatggtgtgattctgacgattccaagcggcattggcaccccagaagctaccattctgtattcgggaccgcgcagtaccttcgatgaacatgaaagcgcactgcgcgcattaggtccgggggcgacctttgtaggggaagatcacggactggctaatctgtacgatgccgcacacctgagcgtcatgtggggcctgctgaatggtttcctgcatggaaccgcactgctgggaaccgcgggcgtttcggcaacctctgtggttccgatgctgggtcaaggtatcggagtggtgaccggttggattgcgcgctacgcagatcagattgatgccggtgtctatccagcagacgacaagacgattgatacccagcgtgctgcaatgcagcacctggtcgaggagagccgtgcggcgggcatcaatggcgaacttccggcgtttgtgaccaaactggccgatcgcgcagtggcagaaggtcgtggtggtgactcttacgctgcactgattgaacagtttcgcaagtcagcttaa

SEQ ID NO: 148 - protein, 292 aa, synthetic construct
  REGION 1..292: note = Imine reductase variant from Pseudonocardia spinosispora
MSDSPVPVTVLGLGLMGQALAGAFLAAGHPTTVWNRSAAKADELVGRGATLAASPAAAVAAGSLIVVCVTDHRAVRELLEPLGDALPGRVLVNLTSGTSREARENAEHTAAQGATYLDGVILTIPSGIGTPEATILYSGPRSTFDEHESALRALGPGATFVGEDHGLANLYDAAHLSVMWGLLNGFLHGTALLGTAGVSATSVVPMLGQGIGVVTGWIARYADQIDAGVYPADDKTIDTQRAAMQHLVEESRAAGINGELPAFVTKLADRAVAEGRGGDSYAALIEQFRKSA

SEQ ID NO: 149 - DNA, 879 bp, synthetic construct
  misc_feature 1..879: note = Imine reductase variant from Pseudonocardia spinosispora
  source 1..879: mol_type = other DNA
atgagtgattcacctgtgcccgtgacagttctgggtcttggtctgatgggtcaggccttagcgggagcgtttctggcagccggtcaccctacgacggtttggaatcgcagcgcagctaaagctgatgaactggttggtcgcggtgcaaccctggccgcgtctcccgcggctgccgtcgcagcgggtagtctgatcgttgtttgcgtcacagatcatcgtgcggtgcgcgaactgctggaaccacttggcgatgcactgccaggtcgcgttctggtcaacctgacgagcggtacgtcgcgtgaagcccgtgagaacgcagaacatactgcggctcagggagccacctacctggatggtgtgattctgggtattccaagcggcattggcaccccagaagctaccattctgtattcgggaccgcgcagtaccttcgatgaacatgaaagcgcactgcgcgcattaggtccgggggcgacctttgtaggggaagatcacggactggctaatctgtacgatgccgcaggcctgagcgtcatgtggggcctgctgaatggtttcctgcatggaaccgcactgctgggaaccgcgggcgtttcggcaacctctgtggttccgatgctgggtcaaggtatcgaagctgtgaccggttggattgcgcgctacgcagatcagattgatgccggtgtctatccagcagacgacgccacgattgatacccagcgtgctgcaatgcagcacctggtcgaggagagccgtgcggcgggcatcaatggcgaacttccggcgtttgtgaccaaactggccgatcgcgcagtggcagaaggtcgtggtggtgactcttacgctgcactgattgaacagtttcgcaagtcagcttaa

SEQ ID NO: 150 - protein, 292 aa, synthetic construct
  REGION 1..292: note = Imine reductase variant from Pseudonocardia spinosispora
MSDSPVPVTVLGLGLMGQALAGAFLAAGHPTTVWNRSAAKADELVGRGATLAASPAAAVAAGSLIVVCVTDHRAVRELLEPLGDALPGRVLVNLTSGTSREARENAEHTAAQGATYLDGVILGIPSGIGTPEATILYSGPRSTFDEHESALRALGPGATFVGEDHGLANLYDAAGLSVMWGLLNGFLHGTALLGTAGVSATSVVPMLGQGIEAVTGWIARYADQIDAGVYPADDATIDTQRAAMQHLVEESRAAGINGELPAFVTKLADRAVAEGRGGDSYAALIEQFRKSA

SEQ ID NO: 151 - DNA, 879 bp, synthetic construct
  misc_feature 1..879: note = Imine reductase variant from Pseudonocardia spinosispora
  source 1..879: mol_type = other DNA
atgagtgattcacctgtgcccgtgacagttctgggtcttggtctgatgggtcaggccttagcgggagcgtttctggcagccggtcaccctacgacggtttggaatcgcagcgcagctaaagctgatgaactggttggtcgcggtgcaaccctggccgcgtctcccgcggctgccgtcgcagcgggtagtctgatcgttgtttgcgtcacagatcatcgtgcggtgcgcgaactgctggaaccacttggcgatgcactgccaggtcgcgttctggtcaacctgacgagcggtacgtcgcgtgaagcccgtgagaacgcagaacatactgcggctcagggagccacctacctggatggtgtgattctgggtattccaagcggcattggcaccccagaagctaccattctgtattcgggaccgcgcagtaccttcgatgaacatgaaagcgcactgcgcgcattaggtccgggggcgacctttgtaggggaagatcacggactggctaatctgtacgatgccgcaggcctgagcgtcatgtggggcctgctgaatggtttcctgcatggaaccgcactgctgggaaccgcgggcgtttcggcaacctctgtggttccgatgctgggtcaaggtatctgcgctgtgaccggttggattgcgcgctacgcagatcagattgatgccggtgtctatccagcagacgacaagacgattgatacccagcgtgctgcaatgcagcacctggtcgaggagagccgtgcggcgggcatcaatggcgaacttccggcgtttgtgaccaaactggccgatcgcgcagtggcagaaggtcgtggtggtgactcttacgctgcactgattgaacagtttcgcaagtcagcttaa

SEQ ID NO: 152 - protein, 292 aa, synthetic construct
  REGION 1..292: note = Imine reductase variant from Pseudonocardia spinosispora
MSDSPVPVTVLGLGLMGQALAGAFLAAGHPTTVWNRSAAKADELVGRGATLAASPAAAVAAGSLIVVCVTDHRAVRELLEPLGDALPGRVLVNLTSGTSREARENAEHTAAQGATYLDGVILGIPSGIGTPEATILYSGPRSTFDEHESALRALGPGATFVGEDHGLANLYDAAGLSVMWGLLNGFLHGTALLGTAGVSATSVVPMLGQGICAVTGWIARYADQIDAGVYPADDKTIDTQRAAMQHLVEESRAAGINGELPAFVTKLADRAVAEGRGGDSYAALIEQFRKSA

SEQ ID NO: 153 - DNA, 879 bp, synthetic construct
  misc_feature 1..879: note = Imine reductase variant from Pseudonocardia spinosispora
  source 1..879: mol_type = other DNA
atgagtgattcacctgtgcccgtgacagttctgggtcttggtctgatgggtcaggccttagcgggagcgtttctggcagccggtcaccctacgacggtttggaatcgcagcgcagctaaagctgatgaactggttggtcgcggtgcaaccctggccgcgtctcccgcggctgccgtcgcagcgggtagtctgatcgttgtttgcgtcacagatcatcgtgcggtgcgcgaactgctggaaccacttggcgatgcactgccaggtcgcgttctggtcaacctgacgagcggtacgtcgcgtgaagcccgtgagaacgcagaacatactgcggctcagggagccacctacctggatggtgtgattctgacgattccaagcggcattggcaccccagaagctaccattctgtattcgggaccgcgcagtaccttcgatgaacatgaaagcgcactgcgcgcattaggtccgggggcgacctttgtaggggaagatcacggactggctaatctgtacgatgccgcaatgctgagcgtcatgtggggcctgctgaatggtttcctgcatggaaccgcactgctgggaaccgcgggcgtttcggcaacctctgtggttccgatgctgggtcaaggtatcgtagtggtgaccggttggattgcgcgctacgcagatcagattgatgccggtgtctatccagcagacgacaagacgattgatacccagcgtgctgcaatgcagcacctggtcgaggagagccgtgcggcgggcatcaatggcgaacttccggcgtttgtgaccaaactggccgatcgcgcagtggcagaaggtcgtggtggtgactcttacgctgcactgattgaacagtttcgcaagtcagcttaa

SEQ ID NO: 154 - protein, 292 aa, synthetic construct
  REGION 1..292: note = Imine reductase variant from Pseudonocardia spinosispora
MSDSPVPVTVLGLGLMGQALAGAFLAAGHPTTVWNRSAAKADELVGRGATLAASPAAAVAAGSLIVVCVTDHRAVRELLEPLGDALPGRVLVNLTSGTSREARENAEHTAAQGATYLDGVILTIPSGIGTPEATILYSGPRSTFDEHESALRALGPGATFVGEDHGLANLYDAAMLSVMWGLLNGFLHGTALLGTAGVSATSVVPMLGQGIVVVTGWIARYADQIDAGVYPADDKTIDTQRAAMQHLVEESRAAGINGELPAFVTKLADRAVAEGRGGDSYAALIEQFRKSA

SEQ ID NO: 155 - DNA, 879 bp, synthetic construct
  misc_feature 1..879: note = Imine reductase variant from Pseudonocardia spinosispora
  source 1..879: mol_type = other DNA
atgagtgattcacctgtgcccgtgacagttctgggtcttggtctgatgggtcaggccttagcgggagcgtttctggcagccggtcaccctacgacggtttggaatcgcagcgcagctaaagctgatgaactggttggtcgcggtgcaaccctggccgcgtctcccgcggctgccgtcgcagcgggtagtctgatcgttgtttgcgtcacagatcatcgtgcggtgcgcgaactgctggaaccacttggcgatgcactgccaggtcgcgttctggtcaacctgacgagcggtacgtcgcgtgaagcccgtgagaacgcagaacatactgcggctcagggagccacctacctggatggtgtgattctgacgattccaagcggcattggcaccccagaagctaccattctgtattcgggaccgcgcagtaccttcgatgaacatgaaagcgcactgcgcgcattaggtccgggggcgacctttgtaggggaagatcacggactggctaatctgtacgatgccgcaggcctgagcgtcatgtggggcctgctgaatggtttcctgcatggaaccgcactgctgggaaccgcgggcgtttcggcaacctctgtggttccgatgctgggtcaaggtatctgcgtggtgaccggttggattgcgcgctacgcagatcagattgatgccggtgtctatccagcagacgacaagacgattgatacccagcgtgctgcaatgcagcacctggtcgaggagagccgtgcggcgggcatcaatggcgaacttccggcgtttgtgaccaaactggccgatcgcgcagtggcagaaggtcgtggtggtgactcttacgctgcactgattgaacagtttcgcaagtcagcttaa

SEQ ID NO: 156 - protein, 292 aa, synthetic construct
  REGION 1..292: note = Imine reductase variant from Pseudonocardia spinosispora
MSDSPVPVTVLGLGLMGQALAGAFLAAGHPTTVWNRSAAKADELVGRGATLAASPAAAVAAGSLIVVCVTDHRAVRELLEPLGDALPGRVLVNLTSGTSREARENAEHTAAQGATYLDGVILTIPSGIGTPEATILYSGPRSTFDEHESALRALGPGATFVGEDHGLANLYDAAGLSVMWGLLNGFLHGTALLGTAGVSATSVVPMLGQGICVVTGWIARYADQIDAGVYPADDKTIDTQRAAMQHLVEESRAAGINGELPAFVTKLADRAVAEGRGGDSYAALIEQFRKSA

SEQ ID NO: 157 - DNA, 879 bp, synthetic construct
  misc_feature 1..879: note = Imine reductase variant from Pseudonocardia spinosispora
  source 1..879: mol_type = other DNA
atgagtgattcacctgtgcccgtgacagttctgggtcttggtctgatgggtcaggccttagcgggagcgtttctggcagccggtcaccctacgacggtttggaatcgcagcgcagctaaagctgatgaactggttggtcgcggtgcaaccctggccgcgtctcccgcggctgccgtcgcagcgggtagtctgatcgttgtttgcgtcacagatcatcgtgcggtgcgcgaactgctggaaccacttggcgatgcactgccaggtcgcgttctggtcaacctgacgagcggtacgtcgcgtgaagcccgtgagaacgcagaacatactgcggctcagggagccacctacctggatggtgtgattctgacgattccaagcggcattggcaccccagaagctaccattctgtattcgggaccgcgcagtaccttcgatgaacatgaaagcgcactgcgcgcattaggtccgggggcgacctttgtaggggaagatcacggactggctaatctggttgatattgcaatgctgagcgtcatgtggggcctgctgaatggtttcctgcatggaaccgcactgctgggaaccgcgggcgtttcggcaacctctgtggttccgatgctgggtcaaggtatcgaagtggtgaccggttggattgcgcgctacgcagatcagattgatgccggtgtctatccagcagacgacaagacgattgatacccagcgtgctgcaatgcagcacctggtcgaggagagccgtgcggcgggcatcaatggcgaacttccggcgtttgtgaccaaactggccgatcgcgcagtggcagaaggtcgtggtggtgactcttacgctgcactgattgaacagtttcgcaagtcagcttaa

SEQ ID NO: 158 - protein, 292 aa, synthetic construct
  REGION 1..292: note = Imine reductase variant from Pseudonocardia spinosispora
MSDSPVPVTVLGLGLMGQALAGAFLAAGHPTTVWNRSAAKADELVGRGATLAASPAAAVAAGSLIVVCVTDHRAVRELLEPLGDALPGRVLVNLTSGTSREARENAEHTAAQGATYLDGVILTIPSGIGTPEATILYSGPRSTFDEHESALRALGPGATFVGEDHGLANLVDIAMLSVMWGLLNGFLHGTALLGTAGVSATSVVPMLGQGIEVVTGWIARYADQIDAGVYPADDKTIDTQRAAMQHLVEESRAAGINGELPAFVTKLADRAVAEGRGGDSYAALIEQFRKSA

SEQ ID NO: 159 - DNA, 879 bp, synthetic construct
  misc_feature 1..879: note = Imine reductase variant from Pseudonocardia spinosispora
  source 1..879: mol_type = other DNA
atgagtgattcacctgtgcccgtgacagttctgggtcttggtctgatgggtcaggccttagcgggagcgtttctggcagccggtcaccctacgacggtttggaatcgcagcgcagctaaagctgatgaactggttggtcgcggtgcaaccctggccgcgtctcccgcggctgccgtcgcagcgggtagtctgatcgttgtttgcgtcacagatcatcgtgcggtgcgcgaactgctggaaccacttggcgatgcactgccaggtcgcgttctggtcaacctgacgagcggtacgtcgcgtgaagcccgtgagaacgcagaacatactgcggctcagggagccacctacctggatggtgtgattctgacgggcccaagcggcattggcaccccagaagctaccattctgtattcgggaccgcgcagtaccttcgatgaacatgaaagcgcactgcgcgcattaggtccgggggcgacctttgtaggggaagatcacggactggctaatctgtacgatgccgcaatgctgagcgtcatgtggggcctgctgaatggtttcctgcatggaaccgcactgctgggaaccgcgggcgtttcggcaacctctgtggttccgatgctgggtcaaggtatcgaagtggtgaccggttggattgcgcgctacgcagatcagattgatgccggtgtctatccagcagacgacaagacgattgatacccagcgtgctgcaatgcagcacctggtcgaggagagccgtgcggcgggcatcaatggcgaacttccggcgtttgtgaccaaactggccgatcgcgcagtggcagaaggtcgtggtggtgactcttacgctgcactgattgaacagtttcgcaagtcagcttaa

SEQ ID NO: 160 - protein, 292 aa, synthetic construct
  REGION 1..292: note = Imine reductase variant from Pseudonocardia spinosispora
MSDSPVPVTVLGLGLMGQALAGAFLAAGHPTTVWNRSAAKADELVGRGATLAASPAAAVAAGSLIVVCVTDHRAVRELLEPLGDALPGRVLVNLTSGTSREARENAEHTAAQGATYLDGVILTGPSGIGTPEATILYSGPRSTFDEHESALRALGPGATFVGEDHGLANLYDAAMLSVMWGLLNGFLHGTALLGTAGVSATSVVPMLGQGIEVVTGWIARYADQIDAGVYPADDKTIDTQRAAMQHLVEESRAAGINGELPAFVTKLADRAVAEGRGGDSYAALIEQFRKSA

SEQ ID NO: 161 - DNA, 879 bp, synthetic construct
  misc_feature 1..879: note = Imine reductase variant from Pseudonocardia spinosispora
  source 1..879: mol_type = other DNA
atgagtgattcacctgtgcccgtgacagttctgggtcttggtctgatgggtcaggccttagcgggagcgtttctggcagccggtcaccctacgacggtttggaatcgcagcgcagctaaagctgatgaactggttggtcgcggtgcaaccctggccgcgtctcccgcggctgccgtcgcagcgggtagtctgatcgttgtttgcgtcacagatcatcgtgcggtgcgcgaactgctggaaccacttggcgatgcactgccaggtcgcgttctggtcaacctgacgagcggtacgtcgcgtgaagcccgtgagaacgcagaacatactgcggctcagggagccacctacctggatggtgtgattctgacgggcccaagcggcattggcaccccagaagctaccattctgtattcgggaccgcgcagtaccttcgatgaacatgaaagcgcactgcgcgcattaggtccgggggcgacctttgtaggggaagatcacggactggctgccctgtacgatgccgcaggcctgagcgtcatgtggggcctgctgaatggtttcctgcatggaaccgcactgctgggaaccgcgggcgtttcggcaacctctgtggttccgatgctgggtcaaggtatcgtagtggtgaccggttggattgcgcgctacgcagatcagattgatgccggtgtctatccagcagacgacaagacgattgatacccagcgtgctgcaatgcagcacctggtcgaggagagccgtgcggcgggcatcaatggcgaacttccggcgtttgtgaccaaactggccgatcgcgcagtggcagaaggtcgtggtggtgactcttacgctgcactgattgaacagtttcgcaagtcagcttaa

SEQ ID NO: 162 - protein, 292 aa, synthetic construct
  REGION 1..292: note = Imine reductase variant from Pseudonocardia spinosispora
MSDSPVPVTVLGLGLMGQALAGAFLAAGHPTTVWNRSAAKADELVGRGATLAASPAAAVAAGSLIVVCVTDHRAVRELLEPLGDALPGRVLVNLTSGTSREARENAEHTAAQGATYLDGVILTGPSGIGTPEATILYSGPRSTFDEHESALRALGPGATFVGEDHGLAALYDAAGLSVMWGLLNGFLHGTALLGTAGVSATSVVPMLGQGIVVVTGWIARYADQIDAGVYPADDKTIDTQRAAMQHLVEESRAAGINGELPAFVTKLADRAVAEGRGGDSYAALIEQFRKSA

SEQ ID NO: 163 - DNA, 879 bp, synthetic construct
  misc_feature 1..879: note = Imine reductase variant from Pseudonocardia spinosispora
  source 1..879: mol_type = other DNA
atgagtgattcacctgtgcccgtgacagttctgggtcttggtctgatgggtcaggccttagcgggagcgtttctggcagccggtcaccctacgacggtttggaatcgcagcgcagctaaagctgatgaactggttggtcgcggtgcaaccctggccgcgtctcccgcggctgccgtcgcagcgggtagtctgatcgttgtttgcgtcacagatcatcgtgcggtgcgcgaactgctggaaccacttggcgatgcactgccaggtcgcgttctggtcaacctgacgagcggtacgtcgcgtgaagcccgtgagaacgcagaacatactgcggctcagggagccacctacctggatggtgtgattctgacgattccaagcggcattggcaccccagaagctaccattctgtattcgggaccgcgcagtaccttcgatgaacatgaaagcgcactgcgcgcattaggtccgggggcgacctttgtaggggaagatcacggactggctaatctgtacgatattgcacacctgagcgtcatgtggggcctgctgaatggtttcctgcatggaaccgcactgctgggaaccgcgggcgtttcggcaacctctgtggttccgatgctgggtcaaggtatcgaagtggtgaccggttggattgcgcgctacgcagatcagattgatgccggtgtctatccagcagacgacaagacgattgatacccagcgtgctgcaatgcagcacctggtcgaggagagccgtgcggcgggcatcaatggcgaacttccggcgtttgtgaccaaactggccgatcgcgcagtggcagaaggtcgtggtggtgactcttacgctgcactgattgaacagtttcgcaagtcagcttaa

SEQ ID NO: 164 - protein, 292 aa, synthetic construct
  REGION 1..292: note = Imine reductase variant from Pseudonocardia spinosispora
MSDSPVPVTVLGLGLMGQALAGAFLAAGHPTTVWNRSAAKADELVGRGATLAASPAAAVAAGSLIVVCVTDHRAVRELLEPLGDALPGRVLVNLTSGTSREARENAEHTAAQGATYLDGVILTIPSGIGTPEATILYSGPRSTFDEHESALRALGPGATFVGEDHGLANLYDIAHLSVMWGLLNGFLHGTALLGTAGVSATSVVPMLGQGIEVVTGWIARYADQIDAGVYPADDKTIDTQRAAMQHLVEESRAAGINGELPAFVTKLADRAVAEGRGGDSYAALIEQFRKSA

SEQ ID NO: 165 - DNA, 879 bp, synthetic construct
  misc_feature 1..879: note = Imine reductase variant from Pseudonocardia spinosispora
  source 1..879: mol_type = other DNA
atgagtgattcacctgtgcccgtgacagttctgggtcttggtctgatgggtcaggccttagcgggagcgtttctggcagccggtcaccctacgacggtttggaatcgcagcgcagctaaagctgatgaactggttggtcgcggtgcaaccctggccgcgtctcccgcggctgccgtcgcagcgggtagtctgatcgttgtttgcgtcacagatcatcgtgcggtgcgcgaactgctggaaccacttggcgatgcactgccaggtcgcgttctggtcaacctgacgagcggtacgtcgcgtgaagcccgtgagaacgcagaacatactgcggctcagggagccacctacctggatggtgtgattctgaccattccaagcggcattggcaccccagaagctacgattctgtattcgggaccgcgcagtaccttcgatgaacatgaaagcgcactgcgcgcattaggtccgggggcgacctttgtaggggaagatcacggactggctaacctgtatgatgcagcaatgtcgagcgtgatgtggggcctgctgaatggtttcctgcatggaaccgcactgctgggaaccgcgggcgtttcggcaacctctgtggttccgatgctgggtcaaggttgggaagcggtgactggtctaattgcgcgctacgcagatcagattgatgccggtgtctatccagcagacgatgccacgattgatacccagcgtgctgcaatgcagcacctggtcgaggagagccgtgcggcgggcatcaatggcgaacttccggcgtttgtgaccaaactggccgatcgcgcagtggcagaaggtcgtggtggtgactcttacgctgcactgattgaacagtttcgcaagtcagcttaa

SEQ ID NO: 166 - protein, 292 aa, synthetic construct
  REGION 1..292: note = Imine reductase variant from Pseudonocardia spinosispora
MSDSPVPVTVLGLGLMGQALAGAFLAAGHPTTVWNRSAAKADELVGRGATLAASPAAAVAAGSLIVVCVTDHRAVRELLEPLGDALPGRVLVNLTSGTSREARENAEHTAAQGATYLDGVILTIPSGIGTPEATILYSGPRSTFDEHESALRALGPGATFVGEDHGLANLYDAAMSSVMWGLLNGFLHGTALLGTAGVSATSVVPMLGQGWEAVTGLIARYADQIDAGVYPADDATIDTQRAAMQHLVEESRAAGINGELPAFVTKLADRAVAEGRGGDSYAALIEQFRKSA

SEQ ID NO: 167 - DNA, 879 bp, synthetic construct
  misc_feature 1..879: note = Imine reductase variant from Pseudonocardia spinosispora
  source 1..879: mol_type = other DNA
atgagtgattcacctgtgcccgtgacagttctgggtcttggtctgatgggtcaggccttagcgggagcgtttctggcagccggtcaccctacgacggtttggaatcgcagcgcagctaaagctgatgaactggttggtcgcggtgcaaccctggccgcgtctcccgcggctgccgtcgcagcgggtagtctgatcgttgtttgcgtcacagatcatcgtgcggtgcgcgaactgctggaaccacttggcgatgcactgccaggtcgcgttctggtcaacctgacgagcggtacgtcgcgtgaagcccgtgagaacgcagaacatactgcggctcagggagccacctacctggatggtgtgattctgaccattccaagcggcattggcaccccagaagctaggattctgtattcgggaccgcgcagtaccttcgatgaacatgaaagcgcactgcgcgcattaggtccgggggcgacctttgtaggggaagatcacggactggctaacctgtatgatgcagcaatgttgagcgtgatgtggggcctgctgaatggtttcctgcatggaaccgcactgctgggaaccgcgggcgtttcggcaacctctgtggttccgatgctgggtcaaggttgggaagcgatgactggtctaattgcgcgctacgcagatcagattgatgccggtgtctatccagcagacgatgccacgattgatacccagcgtgctgcaatgcagcacctggtcgaggagagccgtgcggcgggcatcaatggcgaacttccggcgtttgtgaccaaactggccgatcgcgcagtggcagaaggtcgtggtggtgactcttacgctgcactgattgaacagtttcgcaagtcagcttaa

SEQ ID NO: 168 - protein, 292 aa, synthetic construct
  REGION 1..292: note = Imine reductase variant from Pseudonocardia spinosispora
MSDSPVPVTVLGLGLMGQALAGAFLAAGHPTTVWNRSAAKADELVGRGATLAASPAAAVAAGSLIVVCVTDHRAVRELLEPLGDALPGRVLVNLTSGTSREARENAEHTAAQGATYLDGVILTIPSGIGTPEARILYSGPRSTFDEHESALRALGPGATFVGEDHGLANLYDAAMLSVMWGLLNGFLHGTALLGTAGVSATSVVPMLGQGWEAMTGLIARYADQIDAGVYPADDATIDTQRAAMQHLVEESRAAGINGELPAFVTKLADRAVAEGRGGDSYAALIEQFRKSA

SEQ ID NO: 169 - DNA, 879 bp, synthetic construct
  misc_feature 1..879: note = Imine reductase variant from Pseudonocardia spinosispora
  source 1..879: mol_type = other DNA
atgagtgattcacctgtgcccgtgacagttctgggtcttggtctgatgggtcaggccttagcgggagcgtttctggcagccggtcaccctacgacggtttggaatcgcagcgcagctaaagctgatgaactggttggtcgcggtgcaaccctggccgcgtctcccgcggctgccgtcgcagcgggtagtctgatcgttgtttgcgtcacagatcatcgtgcggtgcgcgaactgctggaaccacttggcgatgcactgccaggtcgcgttctggtcaacctgacgagcggtacgtcgcgtgaagcccgtgagaacgcagaacatactgcggctcagggagccacctacctggatggtgtgattctgaccattccaagcggcattggcaccccagaagctaggattctgtattcgggaccgcgcagtaccttcgatgaacatgaaagcgcactgcgcgcattaggtccgggggcgacctttgtaggggaagatcacggactggctaacctgtatgatgcagcaatgttgagcatgatgtggggcctgctgaatggtttcctgcatggaaccgcactgctgggaaccgcgggcgtttcggcaacctctgtggttccgatgctgggtcaaggttgggaagcgatgactggtataattgcgcgctacgcagatcagattgatgccggtgtctatccagcagacgatgccacgattgatacccagcgtgctgcaatgcagcacctggtcgaggagagccgtgcggcgggcatcaatggcgaacttccggcgtttgtgaccaaactggccgatcgcgcagtggcagaaggtcgtggtggtgactcttacgctgcactgattgaacagtttcgcaagtcagcttaa

SEQ ID NO: 170 - protein, 292 aa, synthetic construct
  REGION 1..292: note = Imine reductase variant from Pseudonocardia spinosispora
MSDSPVPVTVLGLGLMGQALAGAFLAAGHPTTVWNRSAAKADELVGRGATLAASPAAAVAAGSLIVVCVTDHRAVRELLEPLGDALPGRVLVNLTSGTSREARENAEHTAAQGATYLDGVILTIPSGIGTPEARILYSGPRSTFDEHESALRALGPGATFVGEDHGLANLYDAAMLSMMWGLLNGFLHGTALLGTAGVSATSVVPMLGQGWEAMTGIIARYADQIDAGVYPADDATIDTQRAAMQHLVEESRAAGINGELPAFVTKLADRAVAEGRGGDSYAALIEQFRKSA

SEQ ID NO: 171 - DNA, 879 bp, synthetic construct
  misc_feature 1..879: note = Imine reductase variant from Pseudonocardia spinosispora
  source 1..879: mol_type = other DNA
atgagtgattcacctgtgcccgtgacagttctgggtcttggtctgatgggtcaggccttagcgggagcgtttctggcagccggtcaccctacgacggtttggaatcgcagcgcagctaaagctgatgaactggttggtcgcggtgcaaccctggccgcgtctcccgcggctgccgtcgcagcgggtagtctgatcgttgtttgcgtcacagatcatcgtgcggtgcgcgaactgctggaaccacttggcgatgcactgccaggtcgcgttctggtcaacctgacgagcggtacgtcgcgtgaagcccgtgagaacgcagaacatactgcggctcagggagccacctacctggatggtgtgattctgaccattccaagcggcattggcaccccagaagctacgattctgtattcgggaccgcgcagtaccttcgatgaacatgaaagcgcactgcgcgcattaggtccgggggcgacctttgtaggggaagatcacggactggctgccctgtatgatgcagcaatgttgagcatgatgtggggcctgctgaatggtttcctgcatggaaccgcactgctgggaaccgcgggcgtttcggcaacctctgtggttccgatgctgggtcaaggttgggaagcggtgactggtctaattgcgcgctacgcagatcagattgatgccggtgtctatccagcagacgatgccacgattgatacccagcgtgctgcaatgcagcacctggtcgaggagagccgtgcggcgggcatcaatggcgaacttccggcgtttgtgaccaaactggccgatcgcgcagtggcagaaggtcgtggtggtgactcttacgctgcactgattgaacagtttcgcaagtcagcttaa

SEQ ID NO: 172 - protein, 292 aa, synthetic construct
  REGION 1..292: note = Imine reductase variant from Pseudonocardia spinosispora
MSDSPVPVTVLGLGLMGQALAGAFLAAGHPTTVWNRSAAKADELVGRGATLAASPAAAVAAGSLIVVCVTDHRAVRELLEPLGDALPGRVLVNLTSGTSREARENAEHTAAQGATYLDGVILTIPSGIGTPEATILYSGPRSTFDEHESALRALGPGATFVGEDHGLAALYDAAMLSMMWGLLNGFLHGTALLGTAGVSATSVVPMLGQGWEAVTGLIARYADQIDAGVYPADDATIDTQRAAMQHLVEESRAAGINGELPAFVTKLADRAVAEGRGGDSYAALIEQFRKSA

SEQ ID NO: 173 - DNA, 879 bp, synthetic construct
  misc_feature 1..879: note = Imine reductase variant from Pseudonocardia spinosispora
  source 1..879: mol_type = other DNA
atgagtgattcacctgtgcccgtgacagttctgggtcttggtctgatgggtcaggccttagcgggagcgtttctggcagccggtcaccctacgacggtttggaatcgcagcgcagctaaagctgatgaactggttggtcgcggtgcaaccctggccgcgtctcccgcggctgccgtcgcagcgggtagtctgatcgttgtttgcgtcacagatcatcgtgcggtgcgcgaactgctggaaccacttggcgatgcactgccaggtcgcgttctggtcaacctgacgagcggtacgtcgcgtgaagcccgtgagaacgcagaacatactgcggctcagggagccacctacctggatggtgtgattctgaccattccaagcggcattggcaccccagaagctaggattctgtattcgggaccgcgcagtaccttcgatgaacatgaaagcgcactgcgcgcattaggtccgggggcgacctttgtaggggaagatcacggactggctgccctgtatgatgcagcaatgtcgagcgtgatgtggggcctgctgaatggtttcctgcatggaaccgcactgctgggaaccgcgggcgtttcggcaacctctgtggttccgatgctgggtcaaggttgggaagcggtgatgggttggattgcgcgctacgcagatcagattgatgccggtgtctatccagcagacgatgccacgattgatacccagcgtgctgcaatgcagcacctggtcgaggagagccgtgcggcgggcatcaatggcgaacttccggcgtttgtgaccaaactggccgatcgcgcagtggcagaaggtcgtggtggtgactcttacgctgcactgattgaacagtttcgcaagtcagcttaa

SEQ ID NO: 174 - protein, 292 aa, synthetic construct
  REGION 1..292: note = Imine reductase variant from Pseudonocardia spinosispora
MSDSPVPVTVLGLGLMGQALAGAFLAAGHPTTVWNRSAAKADELVGRGATLAASPAAAVAAGSLIVVCVTDHRAVRELLEPLGDALPGRVLVNLTSGTSREARENAEHTAAQGATYLDGVILTIPSGIGTPEARILYSGPRSTFDEHESALRALGPGATFVGEDHGLAALYDAAMSSVMWGLLNGFLHGTALLGTAGVSATSVVPMLGQGWEAVMGWIARYADQIDAGVYPADDATIDTQRAAMQHLVEESRAAGINGELPAFVTKLADRAVAEGRGGDSYAALIEQFRKSA

SEQ ID NO: 175 - DNA, 879 bp, synthetic construct
  misc_feature 1..879: note = Imine reductase variant from Pseudonocardia spinosispora
  source 1..879: mol_type = other DNA
atgagtgattcacctgtgcccgtgacagttctgggtcttggtctgatgggtcaggccttagcgggagcgtttctggcagccggtcaccctacgacggtttggaatcgcagcgcagctaaagctgatgaactggttggtcgcggtgcaaccctggccgcgtctcccgcggctgccgtcgcagcgggtagtctgatcgttgtttgcgtcacagatcatcgtgcggtgcgcgaactgctggaaccacttggcgatgcactgccaggtcgcgttctggtcaacctgacgagcggtacgtcgcgtgaagcccgtgagaacgcagaacatactgcggctcagggagccacctacctggatggtgtgattctgaccattccaagcggcattggcaccccagaagctacgattctgtattcgggaccgcgcagtaccttcgatgaacatgaaagcgcactgcgcgcattaggtccgggggcgacctttgtaggggaagatcacggactggctaacctgtatgatgcagcaatgtcgagcgtgatgtggggcctgctgaatggtttcctgcatggaaccgcactgctgggaaccgcgggcgtttcggcaacctctgtggttccgatgctgggtcaaggttgggaagcgatgactggttggattgcgcgctacgcagatcagattgatgccggtgtctatccagcagacgatgccacgattgatacccagcgtgctgcaatgcagcacctggtcgaggagagccgtgcggcgggcatcaatggcgaacttccggcgtttgtgaccaaactggccgatcgcgcagtggcagaaggtcgtggtggtgactcttacgctgcactgattgaacagtttcgcaagtcagcttaa

SEQ ID NO: 176 - protein, 292 aa, synthetic construct
  REGION 1..292: note = Imine reductase variant from Pseudonocardia spinosispora
MSDSPVPVTVLGLGLMGQALAGAFLAAGHPTTVWNRSAAKADELVGRGATLAASPAAAVAAGSLIVVCVTDHRAVRELLEPLGDALPGRVLVNLTSGTSREARENAEHTAAQGATYLDGVILTIPSGIGTPEATILYSGPRSTFDEHESALRALGPGATFVGEDHGLANLYDAAMSSVMWGLLNGFLHGTALLGTAGVSATSVVPMLGQGWEAMTGWIARYADQIDAGVYPADDATIDTQRAAMQHLVEESRAAGINGELPAFVTKLADRAVAEGRGGDSYAALIEQFRKSA

SEQ ID NO: 177 - DNA, 879 bp, synthetic construct
  misc_feature 1..879: note = Imine reductase variant from Pseudonocardia spinosispora
  source 1..879: mol_type = other DNA
atgagtgattcacctgtgcccgtgacagttctgggtcttggtctgatgggtcaggccttagcgggagcgtttctggcagccggtcaccctacgacggtttggaatcgcagcgcagctaaagctgatgaactggttggtcgcggtgcaaccctggccgcgtctcccgcggctgccgtcgcagcgggtagtctgatcgttgtttgcgtcacagatcatcgtgcggtgcgcgaactgctggaaccacttggcgatgcactgccaggtcgcgttctggtcaacctgacgagcggtacgtcgcgtgaagcccgtgagaacgcagaacatactgcggctcagggagccacctacctggatggtgtgattctgaccattccaagcggcattggcaccccagaagctaggattctgtattcgggaccgcgcagtaccttcgatgaacatgaaagcgcactgcgcgcattaggtccgggggcgacctttgtaggggaagatcacggactggctaacctgtatgatgcagcaatgtcgagcgttatgtggggcctgctgaatggtttcctgcatggaaccgcactgctgggaaccgcgggcgtttcggcaacctctgtggttccgatgctgggtcaaggttgggaagcggtgactggttggattgcgcgctacgcagatcagattgatgccggtgtctatccagcagacgatgccacgattgatacccagcgtgctgcaatgcagcacctggtcgaggagagccgtgcggcgggcatcaatggcgaacttccggcgtttgtgaccaaactggccgatcgcgcagtggcagaaggtcgtggtggtgactcttacgctgcactgattgaacagtttcgcaagtcagcttaa

SEQ ID NO: 178 - protein, 292 aa, synthetic construct
  REGION 1..292: note = Imine reductase variant from Pseudonocardia spinosispora
MSDSPVPVTVLGLGLMGQALAGAFLAAGHPTTVWNRSAAKADELVGRGATLAASPAAAVAAGSLIVVCVTDHRAVRELLEPLGDALPGRVLVNLTSGTSREARENAEHTAAQGATYLDGVILTIPSGIGTPEARILYSGPRSTFDEHESALRALGPGATFVGEDHGLANLYDAAMSSVMWGLLNGFLHGTALLGTAGVSATSVVPMLGQGWEAVTGWIARYADQIDAGVYPADDATIDTQRAAMQHLVEESRAAGINGELPAFVTKLADRAVAEGRGGDSYAALIEQFRKSA

SEQ ID NO: 179 - DNA, 879 bp, synthetic construct
  misc_feature 1..879: note = Imine reductase variant from Pseudonocardia spinosispora
  source 1..879: mol_type = other DNA
atgagtgattcacctgtgcccgtgacagttctgggtcttggtctgatgggtcaggccttagcgggagcgtttctggcagccggtcaccctacgacggtttggaatcgcagcgcagctaaagctgatgaactggttggtcgcggtgcaaccctggccgcgtctcccgcggctgccgtcgcagcgggtagtctgatcgttgtttgcgtcacagatcatcgtgcggtgcgcgaactgctggaaccacttggcgatgcactgccaggtcgcgttctggtcaacctgacgagcggtacgtcgcgtgaagcccgtgagaacgcagaacatactgcggctcagggagccacctacctggatggtgtgattctgaccattccaagcggcattggcaccccagaagctacgattctgtattcgggaccgcgcagtaccttcgatgaacatgaaagcgcactgcgcgcattaggtccgggggcgacctttgtaggggaagatcacggactggctaacctgtatgatgcagcaatgtcgagcgttatgtggggcctgctgaatggtttcctgcatggaaccgcactgctgggaaccgcgggcgtttcggcaacctctgtggttccgatgctgggtcaaggtatagaagcgatgatgggtataattgcgcgctacgcagatcagattgatgccggtgtctatccagcagacgatgccacgattgatacccagcgtgctgcaatgcagcacctggtcgaggagagccgtgcggcgggcatcaatggcgaacttccggcgtttgtgaccaaactggccgatcgcgcagtggcagaaggtcgtggtggtgactcttacgctgcactgattgaacagtttcgcaagtcagcttaa

SEQ ID NO: 180 - protein, 292 aa, synthetic construct
  REGION 1..292: note = Imine reductase variant from Pseudonocardia spinosispora
MSDSPVPVTVLGLGLMGQALAGAFLAAGHPTTVWNRSAAKADELVGRGATLAASPAAAVAAGSLIVVCVTDHRAVRELLEPLGDALPGRVLVNLTSGTSREARENAEHTAAQGATYLDGVILTIPSGIGTPEATILYSGPRSTFDEHESALRALGPGATFVGEDHGLANLYDAAMSSVMWGLLNGFLHGTALLGTAGVSATSVVPMLGQGIEAMMGIIARYADQIDAGVYPADDATIDTQRAAMQHLVEESRAAGINGELPAFVTKLADRAVAEGRGGDSYAALIEQFRKSA

SEQ ID NO: 181 - DNA, 879 bp, synthetic construct
  misc_feature 1..879: note = Imine reductase variant from Pseudonocardia spinosispora
  source 1..879: mol_type = other DNA
atgagtgattcacctgtgcccgtgacagttctgggtcttggtctgatgggtcaggccttagcgggagcgtttctggcagccggtcaccctacgacggtttggaatcgcagcgcagctaaagctgatgaactggttggtcgcggtgcaaccctggccgcgtctcccgcggctgccgtcgcagcgggtagtctgatcgttgtttgcgtcacagatcatcgtgcggtgcgcgaactgctggaaccacttggcgatgcactgccaggtcgcgttctggtcaacctgacgagcggtacgtcgcgtgaagcccgtgagaacgcagaacatactgcggctcagggagccacctacctggatggtgtgattctgaccattccaagcggcattggcaccccagaagctacgattctgtattcgggaccgcgcagtaccttcgatgaacatgaaagcgcactgcgcgcattaggtccgggggcgacctttgtaggggaagatcacggactggctaacctgtatgatgcagcaatgttgagcgtgatgtggggcctgctgaatggtttcctgcatggaaccgcactgctgggaaccgcgggcgtttcggcaacctctgtggttccgatgctgggtcaaggttgggaagcggtgactggtataattgcgcgctacgcagatcagattgatgccggtgtctatccagcagacgatgccacgattgatacccagcgtgctgcaatgcagcacctggtcgaggagagccgtgcggcgggcatcaatggcgaacttccggcgtttgtgaccaaactggccgatcgcgcagtggcagaaggtcgtggtggtgactcttacgctgcactgattgaacagtttcgcaagtcagcttaa

SEQ ID NO: 182 - protein, 292 aa, synthetic construct
  REGION 1..292: note = Imine reductase variant from Pseudonocardia spinosispora
MSDSPVPVTVLGLGLMGQALAGAFLAAGHPTTVWNRSAAKADELVGRGATLAASPAAAVAAGSLIVVCVTDHRAVRELLEPLGDALPGRVLVNLTSGTSREARENAEHTAAQGATYLDGVILTIPSGIGTPEATILYSGPRSTFDEHESALRALGPGATFVGEDHGLANLYDAAMLSVMWGLLNGFLHGTALLGTAGVSATSVVPMLGQGWEAVTGIIARYADQIDAGVYPADDATIDTQRAAMQHLVEESRAAGINGELPAFVTKLADRAVAEGRGGDSYAALIEQFRKSA

SEQ ID NO: 183 - DNA, 879 bp, synthetic construct
  misc_feature 1..879: note = Imine reductase variant from Pseudonocardia spinosispora
  source 1..879: mol_type = other DNA
atgagtgattcacctgtgcccgtgacagttctgggtcttggtctgatgggtcaggccttagcgggagcgtttctggcagccggtcaccctacgacggtttggaatcgcagcgcagctaaagctgatgaactggttggtcgcggtgcaaccctggccgcgtctcccgcggctgccgtcgcagcgggtagtctgatcgttgtttgcgtcacagatcatcgtgcggtgcgcgaactgctggaaccacttggcgatgcactgccaggtcgcgttctggtcaacctgacgagcggtacgtcgcgtgaagcccgtgagaacgcagaacatactgcggctcagggagccacctacctggatggtgtgattctgaccattccaagcggcattggcaccccagaagctaggattctgtattcgggaccgcgcagtaccttcgatgaacatgaaagcgcactgcgcgcattaggtccgggggcgacctttgtaggggaagatcacggactggctgcactgtatgatgcagcaatgttgagcgtgatgtggggcctgctgaatggtttcctgcatggaaccgcactgctgggaaccgcgggcgtttcggcaacctctgtggttccgatgctgggtcaaggttgggaagcgatgactggttggattgcgcgctacgcagatcagattgatgccggtgtctatccagcagacgatgccacgattgatacccagcgtgctgcaatgcagcacctggtcgaggagagccgtgcggcgggcatcaatggcgaacttccggcgtttgtgaccaaactggccgatcgcgcagtggcagaaggtcgtggtggtgactcttacgctgcactgattgaacagtttcgcaagtcagcttaa

SEQ ID NO: 184 - protein, 292 aa, synthetic construct
  REGION 1..292: note = Imine reductase variant from Pseudonocardia spinosispora
MSDSPVPVTVLGLGLMGQALAGAFLAAGHPTTVWNRSAAKADELVGRGATLAASPAAAVAAGSLIVVCVTDHRAVRELLEPLGDALPGRVLVNLTSGTSREARENAEHTAAQGATYLDGVILTIPSGIGTPEARILYSGPRSTFDEHESALRALGPGATFVGEDHGLAALYDAAMLSVMWGLLNGFLHGTALLGTAGVSATSVVPMLGQGWEAMTGWIARYADQIDAGVYPADDATIDTQRAAMQHLVEESRAAGINGELPAFVTKLADRAVAEGRGGDSYAALIEQFRKSA

SEQ ID NO: 185 - DNA, 879 bp, synthetic construct
  misc_feature 1..879: note = Imine reductase variant from Pseudonocardia spinosispora
  source 1..879: mol_type = other DNA
atgagtgattcacctgtgcccgtgacagttctgggtcttggtctgatgggtcaggccttagcgggagcgtttctggcagccggtcaccctacgacggtttggaatcgcagcgcagctaaagctgatgaactggttggtcgcggtgcaaccctggccgcgtctcccgcggctgccgtcgcagcgggtagtctgatcgttgtttgcgtcacagatcatcgtgcggtgcgcgaactgctggaaccacttggcgatgcactgccaggtcgcgttctggtcaacctgacgagcggtacgtcgcgtgaagcccgtgagaacgcagaacatactgcggctcagggagccacctacctggatggtgtgattctgaccattccaagcggcattggcaccccagaagctaggattctgtattcgggaccgcgcagtaccttcgatgaacatgaaagcgcactgcgcgcattaggtccgggggcgacctttgtaggggaagatcacggactggctgccctgtatgatgcagcaatgtcgagcgtgatgtggggcctgctgaatggtttcctgcatggaaccgcactgctgggaaccgcgggcgtttcggcaacctctgtggttccgatgctgggtcaaggttgggaagcgatgactggttggattgcgcgctacgcagatcagattgatgccggtgtctatccagcagacgatgccacgattgatacccagcgtgctgcaatgcagcacctggtcgaggagagccgtgcggcgggcatcaatggcgaacttccggcgtttgtgaccaaactggccgatcgcgcagtggcagaaggtcgtggtggtgactcttacgctgcactgattgaacagtttcgcaagtcagcttaa

SEQ ID NO: 186 - protein, 292 aa, synthetic construct
  REGION 1..292: note = Imine reductase variant from Pseudonocardia spinosispora
MSDSPVPVTVLGLGLMGQALAGAFLAAGHPTTVWNRSAAKADELVGRGATLAASPAAAVAAGSLIVVCVTDHRAVRELLEPLGDALPGRVLVNLTSGTSREARENAEHTAAQGATYLDGVILTIPSGIGTPEARILYSGPRSTFDEHESALRALGPGATFVGEDHGLAALYDAAMSSVMWGLLNGFLHGTALLGTAGVSATSVVPMLGQGWEAMTGWIARYADQIDAGVYPADDATIDTQRAAMQHLVEESRAAGINGELPAFVTKLADRAVAEGRGGDSYAALIEQFRKSA

SEQ ID NO: 187 - DNA, 879 bp, synthetic construct
  misc_feature 1..879: note = Imine reductase variant from Pseudonocardia spinosispora
  source 1..879: mol_type = other DNA
atgagtgattcacctgtgcccgtgacagttctgggtcttggtctgatgggtcaggccttagcgggagcgtttctggcagccggtcaccctacgacggtttggaatcgcagcgcagctaaagctgatgaactggttggtcgcggtgcaaccctggccgcgtctcccgcggctgccgtcgcagcgggtagtctgatcgttgtttgcgtcacagatcatcgtgcggtgcgcgaactgctggaaccacttggcgatgcactgccaggtcgcgttctggtcaacctgacgagcggtacgtcgcgtgaagcccgtgagaacgcagaacatactgcggctcagggagccacctacctggatggtgtgattctgaccattccaagcggcattggcaccccagaagctacgattctgtattcgggaccgcgcagtaccttcgatgaacatgaaagcgcactgcgcgcattaggtccgggggcgacctttgtaggggaagatcacggactggctaacctgtatgatgcagcaatgtcgagcgtgatgtggggcctgctgaatggtttcctgcatggaaccgcactgctgggaaccgcgggcgtttcggcaacctctgtggttccgatgctgggtcaaggtctagaagcgatgactggtataattgcgcgctacgcagatcagattgatgccggtgtctatccagcagacgatgccacgattgatacccagcgtgctgcaatgcagcacctggtcgaggagagccgtgcggcgggcatcaatggcgaacttccggcgtttgtgaccaaactggccgatcgcgcagtggcagaaggtcgtggtggtgactcttacgctgcactgattgaacagtttcgcaagtcagcttaa

SEQ ID NO: 188 - protein, 292 aa, synthetic construct
  REGION 1..292: note = Imine reductase variant from Pseudonocardia spinosispora
MSDSPVPVTVLGLGLMGQALAGAFLAAGHPTTVWNRSAAKADELVGRGATLAASPAAAVAAGSLIVVCVTDHRAVRELLEPLGDALPGRVLVNLTSGTSREARENAEHTAAQGATYLDGVILTIPSGIGTPEATILYSGPRSTFDEHESALRALGPGATFVGEDHGLANLYDAAMSSVMWGLLNGFLHGTALLGTAGVSATSVVPMLGQGLEAMTGIIARYADQIDAGVYPADDATIDTQRAAMQHLVEESRAAGINGELPAFVTKLADRAVAEGRGGDSYAALIEQFRKSA

SEQ ID NO: 189 - DNA, 879 bp, synthetic construct
  misc_feature 1..879: note = Imine reductase variant from Pseudonocardia spinosispora
  source 1..879: mol_type = other DNA
atgagtgattcacctgtgcccgtgacagttctgggtcttggtctgatgggtcaggccttagcgggagcgtttctggcagccggtcaccctacgacggtttggaatcgcagcgcagctaaagctgatgaactggttggtcgcggtgcaaccctggccgcgtctcccgcggctgccgtcgcagcgggtagtctgatcgttgtttgcgtcacagatcatcgtgcggtgcgcgaactgctggaaccacttggcgatgcactgccaggtcgcgttctggtcaacctgacgagcggtacgtcgcgtgaagcccgtgagaacgcagaacatactgcggctcagggagccacctacctggatggtgtgattctgaccattccaagcggcattggcaccccagaagctacgattctgtattcgggaccgcgcagtaccttcgatgaacatgaaagcgcactgcgcgcattaggtccgggggcgacctttgtaggggaagatcacggactggctaacctgtatgatgcagcaatgttgagcatgatgtggggcctgctgaatggtttcctgcatggaaccgcactgctgggaaccgcgggcgtttcggcaacctctgtggttccgatgctgggtcaaggtatagaagcggtgactggttggattgcgcgctacgcagatcagattgatgccggtgtctatccagcagacctcgccacgattgatacccagcgtgctgcaatgcagcacctggtcgaggagagccgtgcggcgggcatcaatggcgaacttccggcgtttgtgaccaaactggccgatcgcgcagtggcagaaggtcgtggtggtgactcttacgctgcactgattgaacagtttcgcaagtcagcttaa

SEQ ID NO: 190 - protein, 292 aa, synthetic construct
  REGION 1..292: note = Imine reductase variant from Pseudonocardia spinosispora
MSDSPVPVTVLGLGLMGQALAGAFLAAGHPTTVWNRSAAKADELVGRGATLAASPAAAVAAGSLIVVCVTDHRAVRELLEPLGDALPGRVLVNLTSGTSREARENAEHTAAQGATYLDGVILTIPSGIGTPEATILYSGPRSTFDEHESALRALGPGATFVGEDHGLANLYDAAMLSMMWGLLNGFLHGTALLGTAGVSATSVVPMLGQGIEAVTGWIARYADQIDAGVYPADLATIDTQRAAMQHLVEESRAAGINGELPAFVTKLADRAVAEGRGGDSYAALIEQFRKSA

SEQ ID NO: 191 - DNA, 879 bp, synthetic construct
  misc_feature 1..879: note = Imine reductase variant from Pseudonocardia spinosispora
  source 1..879: mol_type = other DNA
atgagtgattcacctgtgcccgtgacagttctgggtcttggtctgatgggtcaggccttagcgggagcgtttctggcagccggtcaccctacgacggtttggaatcgcagcgcagctaaagctgatgaactggttggtcgcggtgcaaccctggccgcgtctcccgcggctgccgtcgcagcgggtagtctgatcgttgtttgcgtcacagatcatcgtgcggtgcgcgaactgctggaaccacttggcgatgcactgccaggtcgcgttctggtcaacctgacgagcggtacgtcgcgtgaagcccgtgagaacgcagaacatactgcggctcagggagccacctacctggatggtgtgattctgaccattccaagcggcattggcaccccagaagctaccattctgtattcgggaccgcgcagtaccttcgatgaacatgaaagcgcactgcgcgcattaggtccgggggcgacctttgtaggggaagatcacggactggctaacctgtatgatgcagcaatgtcgagcattatgtggggcctgctgaatggtttcctgcatggaaccgcactgctgggaaccgcgggcgtttcggcaacctctgtggttccgatgctgggtcaaggttgggaagcggtgactggtctaattgcgcgctacgcagatcagattgatgccggtgtctatccagcagacgatgccacgattgatacccagcgtgctgcaatgcagcacctggtcgaggagagccgtgcggcgggcatcaatggcgaacttccggcgtttgtgaccaaactggccgatcgcgcagtggcagaaggtcgtggtggtgactcttacgctgcactgattgaacagtttcgcaagtcagcttaa

SEQ ID NO: 192 - protein, 292 aa, synthetic construct
  REGION 1..292: note = Imine reductase variant from Pseudonocardia spinosispora
MSDSPVPVTVLGLGLMGQALAGAFLAAGHPTTVWNRSAAKADELVGRGATLAASPAAAVAAGSLIVVCVTDHRAVRELLEPLGDALPGRVLVNLTSGTSREARENAEHTAAQGATYLDGVILTIPSGIGTPEATILYSGPRSTFDEHESALRALGPGATFVGEDHGLANLYDAAMSSIMWGLLNGFLHGTALLGTAGVSATSVVPMLGQGWEAVTGLIARYADQIDAGVYPADDATIDTQRAAMQHLVEESRAAGINGELPAFVTKLADRAVAEGRGGDSYAALIEQFRKSA

SEQ ID NO: 193 - DNA, 879 bp, synthetic construct
  misc_feature 1..879: note = Imine reductase variant from Pseudonocardia spinosispora
  source 1..879: mol_type = other DNA
atgagtgattcacctgtgcccgtgacagttctgggtcttggtctgatgggtcaggccttagcgggagcgtttctggcagccggtcaccctacgacggtttggaatcgcagcgcagctaaagctgatgaactggttggtcgcggtgcaaccctggccgcgtctcccgcggctgccgtcgcagcgggtagtctgatcgttgtttgcgtcacagatcatcgtgcggtgcgcgaactgctggaaccacttggcgatgcactgccaggtcgcgttctggtcaacctgacgagcggtacgtcgcgtgaagcccgtgagaacgcagaacatactgcggctcagggagccacctacctggatggtgtgattctgaccattccaagcggcattggcaccccagaagctacgattctgtattcgggaccgcgcagtaccttcgatgaacatgaaagcgcactgcgcgcattaggtccgggggcgacctttgtaggggaagatcacggactggctaacctgtatgatgcagcaatgtcgagcattatgtggggcctgctgaatggtttcctgcatggaaccgcactgctgggaaccgcgggcgtttcggcaacctctgtggttccgatgctgggtcaaggttgggaagcgatgactggtctaattgcgcgctacgcagatcagattgatgccggtgtctatccagcagacgatgccacgattgatacccagcgtgctgcaatgcagcacctggtcgaggagagccgtgcggcgggcatcaatggcgaacttccggcgtttgtgaccaaactggccgatcgcgcagtggcagaaggtcgtggtggtgactcttacgctgcactgattgaacagtttcgcaagtcagcttaa

SEQ ID NO: 194 - protein, 292 aa, synthetic construct
  REGION 1..292: note = Imine reductase variant from Pseudonocardia spinosispora
MSDSPVPVTVLGLGLMGQALAGAFLAAGHPTTVWNRSAAKADELVGRGATLAASPAAAVAAGSLIVVCVTDHRAVRELLEPLGDALPGRVLVNLTSGTSREARENAEHTAAQGATYLDGVILTIPSGIGTPEATILYSGPRSTFDEHESALRALGPGATFVGEDHGLANLYDAAMSSIMWGLLNGFLHGTALLGTAGVSATSVVPMLGQGWEAMTGLIARYADQIDAGVYPADDATIDTQRAAMQHLVEESRAAGINGELPAFVTKLADRAVAEGRGGDSYAALIEQFRKSA

SEQ ID NO: 195 - DNA, 879 bp, synthetic construct
  misc_feature 1..879: note = Imine reductase variant from Pseudonocardia spinosispora
  source 1..879: mol_type = other DNA
atgagtgattcacctgtgcccgtgacagttctgggtcttggtctgatgggtcaggccttagcgggagcgtttctggcagccggtcaccctacgacggtttggaatcgcagcgcagctaaagctgatgaactggttggtcgcggtgcaaccctggccgcgtctcccgcggctgccgtcgcagcgggtagtctgatcgttgtttgcgtcacagatcatcgtgcggtgcgcgaactgctggaaccacttggcgatgcactgccaggtcgcgttctggtcaacctgacgagcggtacgtcgcgtgaagcccgtgagaacgcagaacatactgcggctcagggagccacctacctggatggtgtgattctgaccattccaagcggcattggcaccccagaagctaccattctgtattcgggaccgcgcagtaccttcgatgaacatgaaagcgcactgcgcgcattaggtccgggggcgacctttgtaggggaagatcacggactggctgcactgtatgatgcagcaatgctgagcgtcatgtggggcctgctgaatggtttcctgcatggaaccgcactgctgggaaccgcgggcgtttcggcaacctctgtggttccgatgctgggtcaaggttgggaagcggtgactggttggattgcgcgctacgcagatcagattgatgccggtgtctatccagcagacctcgccacgattgatacccagcgtgctgcaatgcagcacctggtcgaggagagccgtgcggcgggcatcaatggcgaacttccggcgtttgtgaccaaactggccgatcgcgcagtggcagaaggtcgtggtggtgactcttacgctgcactgattgaacagtttcgcaagtcagcttaa

SEQ ID NO: 196 - protein, 292 aa, synthetic construct
  REGION 1..292: note = Imine reductase variant from Pseudonocardia spinosispora
MSDSPVPVTVLGLGLMGQALAGAFLAAGHPTTVWNRSAAKADELVGRGATLAASPAAAVAAGSLIVVCVTDHRAVRELLEPLGDALPGRVLVNLTSGTSREARENAEHTAAQGATYLDGVILTIPSGIGTPEATILYSGPRSTFDEHESALRALGPGATFVGEDHGLAALYDAAMLSVMWGLLNGFLHGTALLGTAGVSATSVVPMLGQGWEAVTGWIARYADQIDAGVYPADLATIDTQRAAMQHLVEESRAAGINGELPAFVTKLADRAVAEGRGGDSYAALIEQFRKSA

SEQ ID NO: 197 - DNA, 879 bp, synthetic construct
  misc_feature 1..879: note = Imine reductase variant from Pseudonocardia spinosispora
  source 1..879: mol_type = other DNA
atgagtgattcacctgtgcccgtgacagttctgggtcttggtctgatgggtcaggccttagcgggagcgtttctggcagccggtcaccctacgacggtttggaatcgcagcgcagctaaagctgatgaactggttggtcgcggtgcaaccctggccgcgtctcccgcggctgccgtcgcagcgggtagtctgatcgttgtttgcgtcacagatcatcgtgcggtgcgcgaactgctggaaccacttggcgatgcactgccaggtcgcgttctggtcaacctgacgagcggtacgtcgcgtgaagcccgtgagaacgcagaacatactgcggctcagggagccacctacctggatggtgtgattctgaccattccaagcggcattggcaccccagaagctaccattctgtattcgggaccgcgcagtaccttcgatgaacatgaaagcgcactgcgcgcattaggtccgggggcgacctttgtaggggaagatcacggactggctgccctgtatgatgcagcaatgtcgagcgtgatgtggggcctgctgaatggtttcctgcatggaaccgcactgctgggaaccgcgggcgtttcggcaacctctgtggttccgatgctgggtcaaggtatagaagcgatgactggtctaattgcgcgctacgcagatcagattgatgccggtgtctatccagcagacgatgccacgattgatacccagcgtgctgcaatgcagcacctggtcgaggagagccgtgcggcgggcatcaatggcgaacttccggcgtttgtgaccaaactggccgatcgcgcagtggcagaaggtcgtggtggtgactcttacgctgcactgattgaacagtttcgcaagtcagcttaa

SEQ ID NO: 198 - protein, 292 aa, synthetic construct
  REGION 1..292: note = Imine reductase variant from Pseudonocardia spinosispora
MSDSPVPVTVLGLGLMGQALAGAFLAAGHPTTVWNRSAAKADELVGRGATLAASPAAAVAAGSLIVVCVTDHRAVRELLEPLGDALPGRVLVNLTSGTSREARENAEHTAAQGATYLDGVILTIPSGIGTPEATILYSGPRSTFDEHESALRALGPGATFVGEDHGLAALYDAAMSSVMWGLLNGFLHGTALLGTAGVSATSVVPMLGQGIEAMTGLIARYADQIDAGVYPADDATIDTQRAAMQHLVEESRAAGINGELPAFVTKLADRAVAEGRGGDSYAALIEQFRKSA

SEQ ID NO: 199 - DNA, 879 bp, synthetic construct
  misc_feature 1..879: note = Imine reductase variant from Pseudonocardia spinosispora
  source 1..879: mol_type = other DNA
atgagtgattcacctgtgcccgtgacagttctgggtcttggtctgatgggtcaggccttagcgggagcgtttctggcagccggtcaccctacgacggtttggaatcgcagcgcagctaaagctgatgaactggttggtcgcggtgcaaccctggccgcgtctcccgcggctgccgtcgcagcgggtagtctgatcgttgtttgcgtcacagatcatcgtgcggtgcgcgaactgctggaaccacttggcgatgcactgccaggtcgcgttctggtcaacctgacgagcggtacgtcgcgtgaagcccgtgagaacgcagaacatactgcggctcagggagccacctacctggatggtgtgattctgaccattccaagcggcattggcaccccagaagctacgattctgtattcgggaccgcgcagtaccttcgatgaacatgaaagcgcactgcgcgcattaggtccgggggcgacctttgtaggggaagatcacggactggctgccctgtatgatgcagcaatgtcgagcattatgtggggcctgctgaatggtttcctgcatggaaccgcactgctgggaaccgcgggcgtttcggcaacctctgtggttccgatgctgggtcaaggttgggaagcggtgttgggtctaattgcgcgctacgcagatcagattgatgccggtgtctatccagcagacgatgccacgattgatacccagcgtgctgcaatgcagcacctggtcgaggagagccgtgcggcgggcatcaatggcgaacttccggcgtttgtgaccaaactggccgatcgcgcagtggcagaaggtcgtggtggtgactcttacgctgcactgattgaacagtttcgcaagtcagcttaa

SEQ ID NO: 200 - protein, 292 aa, synthetic construct
  REGION 1..292: note = Imine reductase variant from Pseudonocardia spinosispora
MSDSPVPVTVLGLGLMGQALAGAFLAAGHPTTVWNRSAAKADELVGRGATLAASPAAAVAAGSLIVVCVTDHRAVRELLEPLGDALPGRVLVNLTSGTSREARENAEHTAAQGATYLDGVILTIPSGIGTPEATILYSGPRSTFDEHESALRALGPGATFVGEDHGLAALYDAAMSSIMWGLLNGFLHGTALLGTAGVSATSVVPMLGQGWEAVLGLIARYADQIDAGVYPADDATIDTQRAAMQHLVEESRAAGINGELPAFVTKLADRAVAEGRGGDSYAALIEQFRKSA

SEQ ID NO: 201 - DNA, 879 bp, synthetic construct
  misc_feature 1..879: note = Imine reductase variant from Pseudonocardia spinosispora
  source 1..879: mol_type = other DNA
atgagtgattcacctgtgcccgtgacagttctgggtcttggtctgatgggtcaggccttagcgggagcgtttctggcagccggtcaccctacgacggtttggaatcgcagcgcagctaaagctgatgaactggttggtcgcggtgcaaccctggccgcgtctcccgcggctgccgtcgcagcgggtagtctgatcgttgtttgcgtcacagatcatcgtgcggtgcgcgaactgctggaaccacttggcgatgcactgccaggtcgcgttctggtcaacctgacgagcggtacgtcgcgtgaagcccgtgagaacgcagaacatactgcggctcagggagccacctacctggatggtgtgattctgaccattccaagcggcattggcaccccagaagctacgattctgtattcgggaccgcgcagtaccttcgatgaacatgaaagcgcactgcgcgcattaggtccgggggcgacctttgtaggggaagatcacggactggctgccctgtatgatgcagcaatgtcgagcattatgtggggcctgctgaatggtttcctgcatggaaccgcactgctgggaaccgcgggcgtttcggcaacctctgtggttccgatgctgggtcaaggttgggaagcggtgactggtataattgcgcgctacgcagatcagattgatgccggtgtctatccagcagacgatgccacgattgatacccagcgtgctgcaatgcagcacctggtcgaggagagccgtgcggcgggcatcaatggcgaacttccggcgtttgtgaccaaactggccgatcgcgcagtggcagaaggtcgtggtggtgactcttacgctgcactgattgaacagtttcgcaagtcagcttaa

SEQ ID NO: 202 - protein, 292 aa, synthetic construct
  REGION 1..292: note = Imine reductase variant from Pseudonocardia spinosispora
MSDSPVPVTVLGLGLMGQALAGAFLAAGHPTTVWNRSAAKADELVGRGATLAASPAAAVAAGSLIVVCVTDHRAVRELLEPLGDALPGRVLVNLTSGTSREARENAEHTAAQGATYLDGVILTIPSGIGTPEATILYSGPRSTFDEHESALRALGPGATFVGEDHGLAALYDAAMSSIMWGLLNGFLHGTALLGTAGVSATSVVPMLGQGWEAVTGIIARYADQIDAGVYPADDATIDTQRAAMQHLVEESRAAGINGELPAFVTKLADRAVAEGRGGDSYAALIEQFRKSA

SEQ ID NO: 203 - DNA, 879 bp, synthetic construct
  misc_feature 1..879: note = Imine reductase variant from Pseudonocardia spinosispora
  source 1..879: mol_type = other DNA
atgagtgattcacctgtgcccgtgacagttctgggtcttggtctgatgggtcaggccttagcgggagcgtttctggcagccggtcaccctacgacggtttggaatcgcagcgcagctaaagctgatgaactggttggtcgcggtgcaaccctggccgcgtctcccgcggctgccgtcgcagcgggtagtctgatcgttgtttgcgtcacagatcatcgtgcggtgcgcgaactgctggaaccacttggcgatgcactgccaggtcgcgttctggtcaacctgacgagcggtacgtcgcgtgaagcccgtgagaacgcagaacatactgcggctcagggagccacctacctggatggtgtgattctgaccattccaagcggcattggcaccccagaagctacgattctgtattcgggaccgcgcagtaccttcgatgaacatgaaagcgcactgcgcgcattaggtccgggggcgacctttgtaggggaagatcacggactggctaacctgtatgatgcagcaatgtcgagcatgatgtggggcctgctgaatggtttcctgcatggaaccgcactgctgggaaccgcgggcgtttcggcaacctctgtggttccgatgctgggtcaaggtatcgaagcggtgaccggttggattgcgcgctacgcagatcagattgatgccggtgtctatccagcagacgatgccacgattgatacccagcgtgctgcaatgcagcacctggtcgaggagagccgtgcggcgggcatcaatggcgaacttccggcgtttgtgaccaaactggccgatcgcgcagtggcagaaggtcgtggtggtgactcttacgctgcactgattgaacagtttcgcaagtcagcttaa

SEQ ID NO: 204 - protein, 292 aa, synthetic construct
  REGION 1..292: note = Imine reductase variant from Pseudonocardia spinosispora
MSDSPVPVTVLGLGLMGQALAGAFLAAGHPTTVWNRSAAKADELVGRGATLAASPAAAVAAGSLIVVCVTDHRAVRELLEPLGDALPGRVLVNLTSGTSREARENAEHTAAQGATYLDGVILTIPSGIGTPEATILYSGPRSTFDEHESALRALGPGATFVGEDHGLANLYDAAMSSMMWGLLNGFLHGTALLGTAGVSATSVVPMLGQGIEAVTGWIARYADQIDAGVYPADDATIDTQRAAMQHLVEESRAAGINGELPAFVTKLADRAVAEGRGGDSYAALIEQFRKSA

SEQ ID NO: 205 - DNA, 879 bp, synthetic construct
  misc_feature 1..879: note = Imine reductase variant from Pseudonocardia spinosispora
  source 1..879: mol_type = other DNA
atgagtgattcacctgtgcccgtgacagttctgggtcttggtctgatgggtcaggccttagcgggagcgtttctggcagccggtcaccctacgacggtttggaatcgcagcgcagctaaagctgatgaactggttggtcgcggtgcaaccctggccgcgtctcccgcggctgccgtcgcagcgggtagtctgatcgttgtttgcgtcacagatcatcgtgcggtgcgcgaactgctggaaccacttggcgatgcactgccaggtcgcgttctggtcaacctgacgagcggtacgtcgcgtgaagcccgtgagaacgcagaacatactgcggctcagggagccacctacctggatggtgtgattctgaccattccaagcggcattggcaccccagaagctacgattctgtattcgggaccgcgcagtaccttcgatgaacatgaaagcgcactgcgcgcattaggtccgggggcgacctttgtaggggaagatcacggactggctaacctgtatgatgcagcaatgttgagcattatgtggggcctgctgaatggtttcctgcatggaaccgcactgctgggaaccgcgggcgtttcggcaacctctgtggttccgatgctgggtcaaggtatcgaagcggtgactggtataattgcgcgctacgcagatcagattgatgccggtgtctatccagcagacgacgccacgattgatacccagcgtgctgcaatgcagcacctggtcgaggagagccgtgcggcgggcatcaatggcgaacttccggcgtttgtgaccaaactggccgatcgcgcagtggcagaaggtcgtggtggtgactcttacgctgcactgattgaacagtttcgcaagtcagcttaa

SEQ ID NO: 206 - protein, 292 aa, synthetic construct
  REGION 1..292: note = Imine reductase variant from Pseudonocardia spinosispora
MSDSPVPVTVLGLGLMGQALAGAFLAAGHPTTVWNRSAAKADELVGRGATLAASPAAAVAAGSLIVVCVTDHRAVRELLEPLGDALPGRVLVNLTSGTSREARENAEHTAAQGATYLDGVILTIPSGIGTPEATILYSGPRSTFDEHESALRALGPGATFVGEDHGLANLYDAAMLSIMWGLLNGFLHGTALLGTAGVSATSVVPMLGQGIEAVTGIIARYADQIDAGVYPADDATIDTQRAAMQHLVEESRAAGINGELPAFVTKLADRAVAEGRGGDSYAALIEQFRKSA

SEQ ID NO: 207 - DNA, 879 bp, synthetic construct
  misc_feature 1..879: note = Imine reductase variant from Pseudonocardia spinosispora
  source 1..879: mol_type = other DNA
atgagtgattcacctgtgcccgtgacagttctgggtcttggtctgatgggtcaggccttagcgggagcgtttctggcagccggtcaccctacgacggtttggaatcgcagcgcagctaaagctgatgaactggttggtcgcggtgcaaccctggccgcgtctcccgcggctgccgtcgcagcgggtagtctgatcgttgtttgcgtcacagatcatcgtgcggtgcgcgaactgctggaaccacttggcgatgcactgccaggtcgcgttctggtcaacctgacgagcggtacgtcgcgtgaagcccgtgagaacgcagaacatactgcggctcagggagccacctacctggatggtgtgattctgaccattccaagcggcattggcaccccagaagctaggattctgtattcgggaccgcgcagtaccttcgatgaacatgaaagcgcactgcgcgcattaggtccgggggcgacctttgtaggggaagatcacggactggctaacctgtatgatgcagcaatgtcgagcattatgtggggcctgctgaatggtttcctgcatggaaccgcactgctgggaaccgcgggcgtttcggcaacctctgtggttccgatgctgggtcaaggttgggaagcggtgactggttggattgcgcgctacgcagatcagattgatgccggtgtctatccagcagacgatgccacgattgatacccagcgtgctgcaatgcagcacctggtcgaggagagccgtgcggcgggcatcaatggcgaacttccggcgtttgtgaccaaactggccgatcgcgcagtggcagaaggtcgtggtggtgactcttacgctgcactgattgaacagtttcgcaagtcagcttaa

SEQ ID NO: 208 - protein, 292 aa, synthetic construct
  REGION 1..292: note = Imine reductase variant from Pseudonocardia spinosispora
MSDSPVPVTVLGLGLMGQALAGAFLAAGHPTTVWNRSAAKADELVGRGATLAASPAAAVAAGSLIVVCVTDHRAVRELLEPLGDALPGRVLVNLTSGTSREARENAEHTAAQGATYLDGVILTIPSGIGTPEARILYSGPRSTFDEHESALRALGPGATFVGEDHGLANLYDAAMSSIMWGLLNGFLHGTALLGTAGVSATSVVPMLGQGWEAVTGWIARYADQIDAGVYPADDATIDTQRAAMQHLVEESRAAGINGELPAFVTKLADRAVAEGRGGDSYAALIEQFRKSA

SEQ ID NO: 209 - DNA, 879 bp, synthetic construct
  misc_feature 1..879: note = Imine reductase variant from Pseudonocardia spinosispora
  source 1..879: mol_type = other DNA
atgagtgattcacctgtgcccgtgacagttctgggtcttggtctgatgggtcaggccttagcgggagcgtttctggcagccggtcaccctacgacggtttggaatcgcagcgcagctaaagctgatgaactggttggtcgcggtgcaaccctggccgcgtctcccgcggctgccgtcgcagcgggtagtctgatcgttgtttgcgtcacagatcatcgtgcggtgcgcgaactgctggaaccacttggcgatgcactgccaggtcgcgttctggtcaacctgacgagcggtacgtcgcgtgaagcccgtgagaacgcagaacatactgcggctcagggagccacctacctggatggtgtgattctgaccattccaagcggcattggcaccccagaagctaccattctgtattcgggaccgcgcagtaccttcgatgaacatgaaagcgcactgcgcgcattaggtccgggggcgacctttgtaggggaagatcacggactggctaacctgtatgatgcagcaatgttgagcgtgatgtggggcctgctgaatggtttcctgcatggaaccgcactgctgggaaccgcgggcgtttcggcaacctctgtggttccgatgctgggtcaaggttgggaagcgatgttgggttggattgcgcgctacgcagatcagattgatgccggtgtctatccagcagacgacgccacgattgatacccagcgtgctgcaatgcagcacctggtcgaggagagccgtgcggcgggcatcaatggcgaacttccggcgtttgtgaccaaactggccgatcgcgcagtggcagaaggtcgtggtggtgactcttacgctgcactgattgaacagtttcgcaagtcagcttaa

SEQ ID NO: 210 - protein, 292 aa, synthetic construct
  REGION 1..292: note = Imine reductase variant from Pseudonocardia spinosispora
MSDSPVPVTVLGLGLMGQALAGAFLAAGHPTTVWNRSAAKADELVGRGATLAASPAAAVAAGSLIVVCVTDHRAVRELLEPLGDALPGRVLVNLTSGTSREARENAEHTAAQGATYLDGVILTIPSGIGTPEATILYSGPRSTFDEHESALRALGPGATFVGEDHGLANLYDAAMLSVMWGLLNGFLHGTALLGTAGVSATSVVPMLGQGWEAMLGWIARYADQIDAGVYPADDATIDTQRAAMQHLVEESRAAGINGELPAFVTKLADRAVAEGRGGDSYAALIEQFRKSA

SEQ ID NO: 211 - DNA, 879 bp, synthetic construct
  misc_feature 1..879: note = Imine reductase variant from Pseudonocardia spinosispora
  source 1..879: mol_type = other DNA
atgagtgattcacctgtgcccgtgacagttctgggtcttggtctgatgggtcaggccttagcgggagcgtttctggcagccggtcaccctacgacggtttggaatcgcagcgcagctaaagctgatgaactggttggtcgcggtgcaaccctggccgcgtctcccgcggctgccgtcgcagcgggtagtctgatcgttgtttgcgtcacagatcatcgtgcggtgcgcgaactgctggaaccacttggcgatgcactgccaggtcgcgttctggtcaacctgacgagcggtacgtcgcgtgaagcccgtgagaacgcagaacatactgcggctcagggagccacctacctggatggtgtgattctgaccattccaagcggcattggcaccccagaagctaccattctgtattcgggaccgcgcagtaccttcgatgaacatgaaagcgcactgcgcgcattaggtccgggggcgacctttgtaggggaagatcacggactggctgccctgtatgatgcagcaatgttgagcattatgtggggcctgctgaatggtttcctgcatggaaccgcactgctgggaaccgcgggcgtttcggcaacctctgtggttccgatgctgggtcaaggtatcgaagcggtgatgggttggattgcgcgctacgcagatcagattgatgccggtgtctatccagcagacgatgccacgattgatacccagcgtgctgcaatgcagcacctggtcgaggagagccgtgcggcgggcatcaatggcgaacttccggcgtttgtgaccaaactggccgatcgcgcagtggcagaaggtcgtggtggtgactcttacgctgcactgattgaacagtttcgcaagtcagcttaa

SEQ ID NO: 212 - protein, 292 aa, synthetic construct
  REGION 1..292: note = Imine reductase variant from Pseudonocardia spinosispora
MSDSPVPVTVLGLGLMGQALAGAFLAAGHPTTVWNRSAAKADELVGRGATLAASPAAAVAAGSLIVVCVTDHRAVRELLEPLGDALPGRVLVNLTSGTSREARENAEHTAAQGATYLDGVILTIPSGIGTPEATILYSGPRSTFDEHESALRALGPGATFVGEDHGLAALYDAAMLSIMWGLLNGFLHGTALLGTAGVSATSVVPMLGQGIEAVMGWIARYADQIDAGVYPADDATIDTQRAAMQHLVEESRAAGINGELPAFVTKLADRAVAEGRGGDSYAALIEQFRKSA

SEQ ID NO: 213 - DNA, 879 bp, synthetic construct
  misc_feature 1..879: note = Imine reductase variant from Pseudonocardia spinosispora
  source 1..879: mol_type = other DNA
atgagtgattcacctgtgcccgtgacagttctgggtcttggtctgatgggtcaggccttagcgggagcgtttctggcagccggtcaccctacgacggtttggaatcgcagcgcagctaaagctgatgaactggttggtcgcggtgcaaccctggccgcgtctcccgcggctgccgtcgcagcgggtagtctgatcgttgtttgcgtcacagatcatcgtgcggtgcgcgaactgctggaaccacttggcgatgcactgccaggtcgcgttctggtcaacctgacgagcggtacgtcgcgtgaagcccgtgagaacgcagaacatactgcggctcagggagccacctacctggatggtgtgattctgaccattccaagcggcattggcaccccagaagctaggattctgtattcgggaccgcgcagtaccttcgatgaacatgaaagcgcactgcgcgcattaggtccgggggcgacctttgtaggggaagatcacggactggctaacctgtatgatgcagcaatgtcgagcgtgatgtggggcctgctgaatggtttcctgcatggaaccgcactgctgggaaccgcgggcgtttcggcaacctctgtggttccgatgctgggtcaaggtctagaagcggtgatgggtataattgcgcgctacgcagatcagattgatgccggtgtctatccagcagacctcgccacgattgatacccagcgtgctgcaatgcagcacctggtcgaggagagccgtgcggcgggcatcaatggcgaacttccggcgtttgtgaccaaactggccgatcgcgcagtggcagaaggtcgtggtggtgactcttacgctgcactgattgaacagtttcgcaagtcagcttaa

SEQ ID NO: 214 - protein, 292 aa, synthetic construct
  REGION 1..292: note = Imine reductase variant from Pseudonocardia spinosispora
MSDSPVPVTVLGLGLMGQALAGAFLAAGHPTTVWNRSAAKADELVGRGATLAASPAAAVAAGSLIVVCVTDHRAVRELLEPLGDALPGRVLVNLTSGTSREARENAEHTAAQGATYLDGVILTIPSGIGTPEARILYSGPRSTFDEHESALRALGPGATFVGEDHGLANLYDAAMSSVMWGLLNGFLHGTALLGTAGVSATSVVPMLGQGLEAVMGIIARYADQIDAGVYPADLATIDTQRAAMQHLVEESRAAGINGELPAFVTKLADRAVAEGRGGDSYAALIEQFRKSA

SEQ ID NO: 215 - DNA, 879 bp, synthetic construct
  misc_feature 1..879: note = Imine reductase variant from Pseudonocardia spinosispora
  source 1..879: mol_type = other DNA
atgagtgattcacctgtgcccgtgacagttctgggtcttggtctgatgggtcaggccttagcgggagcgtttctggcagccggtcaccctacgacggtttggaatcgcagcgcagctaaagctgatgaactggttggtcgcggtgcaaccctggccgcgtctcccgcggctgccgtcgcagcgggtagtctgatcgttgtttgcgtcacagatcatcgtgcggtgcgcgaactgctggaaccacttggcgatgcactgccaggtcgcgttctggtcaacctgacgagcggtacgtcgcgtgaagcccgtgagaacgcagaacatactgcggctcagggagccacctacctggatggtgtgattctgaccattccaagcggcattggcaccccagaagctacgattctgtattcgggaccgcgcagtaccttcgatgaacatgaaagcgcactgcgcgcattaggtccgggggcgacctttgtaggggaagatcacggactggctaacctgtatgatgcagcaatgtcgagcgtgatgtggggcctgctgaatggtttcctgcatggaaccgcactgctgggaaccgcgggcgtttcggcaacctctgtggttccgatgctgggtcaaggttgggaagcgatgttgggttggattgcgcgctacgcagatcagattgatgccggtgtctatccagcagacctcgccacgattgatacccagcgtgctgcaatgcagcacctggtcgaggagagccgtgcggcgggcatcaatggcgaacttccggcgtttgtgaccaaactggccgatcgcgcagtggcagaaggtcgtggtggtgactcttacgctgcactgattgaacagtttcgcaagtcagcttaa

SEQ ID NO: 216 - protein, 292 aa, synthetic construct
  REGION 1..292: note = Imine reductase variant from Pseudonocardia spinosispora
MSDSPVPVTVLGLGLMGQALAGAFLAAGHPTTVWNRSAAKADELVGRGATLAASPAAAVAAGSLIVVCVTDHRAVRELLEPLGDALPGRVLVNLTSGTSREARENAEHTAAQGATYLDGVILTIPSGIGTPEATILYSGPRSTFDEHESALRALGPGATFVGEDHGLANLYDAAMSSVMWGLLNGFLHGTALLGTAGVSATSVVPMLGQGWEAMLGWIARYADQIDAGVYPADLATIDTQRAAMQHLVEESRAAGINGELPAFVTKLADRAVAEGRGGDSYAALIEQFRKSA

SEQ ID NO: 217 - DNA, 879 bp, synthetic construct
  misc_feature 1..879: note = Imine reductase variant from Pseudonocardia spinosispora
  source 1..879: mol_type = other DNA
atgagtgattcacctgtgcccgtgacagttctgggtcttggtctgatgggtcaggccttagcgggagcgtttctggcagccggtcaccctacgacggtttggaatcgcagcgcagctaaagctgatgaactggttggtcgcggtgcaaccctggccgcgtctcccgcggctgccgtcgcagcgggtagtctgatcgttgtttgcgtcacagatcatcgtgcggtgcgcgaactgctggaaccacttggcgatgcactgccaggtcgcgttctggtcaacctgacgagcggtacgtcgcgtgaagcccgtgagaacgcagaacatactgcggctcagggagccacctacctggatggtgtgattctgaccattccaagcggcattggcaccccagaagctacgattctgtattcgggaccgcgcagtaccttcgatgaacatgaaagcgcactgcgcgcattaggtccgggggcgacctttgtaggggaagatcacggactggctgccctgtatgatgcagcaatgttgagcatgatgtggggcctgctgaatggtttcctgcatggaaccgcactgctgggaaccgcgggcgtttcggcaacctctgtggttccgatgctgggtcaaggtctagaagcgatgactggttggattgcgcgctacgcagatcagattgatgccggtgtctatccagcagacgacgccacgattgatacccagcgtgctgcaatgcagcacctggtcgaggagagccgtgcggcgggcatcaatggcgaacttccggcgtttgtgaccaaactggccgatcgcgcagtggcagaaggtcgtggtggtgactcttacgctgcactgattgaacagtttcgcaagtcagcttaa

SEQ ID NO: 218 - protein, 292 aa, synthetic construct
  REGION 1..292: note = Imine reductase variant from Pseudonocardia spinosispora
MSDSPVPVTVLGLGLMGQALAGAFLAAGHPTTVWNRSAAKADELVGRGATLAASPAAAVAAGSLIVVCVTDHRAVRELLEPLGDALPGRVLVNLTSGTSREARENAEHTAAQGATYLDGVILTIPSGIGTPEATILYSGPRSTFDEHESALRALGPGATFVGEDHGLAALYDAAMLSMMWGLLNGFLHGTALLGTAGVSATSVVPMLGQGLEAMTGWIARYADQIDAGVYPADDATIDTQRAAMQHLVEESRAAGINGELPAFVTKLADRAVAEGRGGDSYAALIEQFRKSA

SEQ ID NO: 219 - DNA, 879 bp, synthetic construct
  misc_feature 1..879: note = Imine reductase variant from Pseudonocardia spinosispora
  source 1..879: mol_type = other DNA
atgagtgattcacctgtgcccgtgacagttctgggtcttggtctgatgggtcaggccttagcgggagcgtttctggcagccggtcaccctacgacggtttggaatcgcagcgcagctaaagctgatgaactggttggtcgcggtgcaaccctggccgcgtctcccgcggctgccgtcgcagcgggtagtctgatcgttgtttgcgtcacagatcatcgtgcggtgcgcgaactgctggaaccacttggcgatgcactgccaggtcgcgttctggtcaacctgacgagcggtacgtcgcgtgaagcccgtgagaacgcagaacatactgcggctcagggagccacctacctggatggtgtgattctgaccattccaagcggcattggcaccccagaagctacgattctgtattcgggaccgcgcagtaccttcgatgaacatgaaagcgcactgcgcgcattaggtccgggggcgacctttgtaggggaagatcacggactggctgcactgtatgatgcagcaatgtcgagcgttatgtggggcctgctgaatggtttcctgcatggaaccgcactgctgggaaccgcgggcgtttcggcaacctctgtggttccgatgctgggtcaaggtctagaagcgatgactggttggattgcgcgctacgcagatcagattgatgccggtgtctatccagcagacgatgccacgattgatacccagcgtgctgcaatgcagcacctggtcgaggagagccgtgcggcgggcatcaatggcgaacttccggcgtttgtgaccaaactggccgatcgcgcagtggcagaaggtcgtggtggtgactcttacgctgcactgattgaacagtttcgcaagtcagcttaa

SEQ ID NO: 220 - protein, 292 aa, synthetic construct
  REGION 1..292: note = Imine reductase variant from Pseudonocardia spinosispora
MSDSPVPVTVLGLGLMGQALAGAFLAAGHPTTVWNRSAAKADELVGRGATLAASPAAAVAAGSLIVVCVTDHRAVRELLEPLGDALPGRVLVNLTSGTSREARENAEHTAAQGATYLDGVILTIPSGIGTPEATILYSGPRSTFDEHESALRALGPGATFVGEDHGLAALYDAAMSSVMWGLLNGFLHGTALLGTAGVSATSVVPMLGQGLEAMTGWIARYADQIDAGVYPADDATIDTQRAAMQHLVEESRAAGINGELPAFVTKLADRAVAEGRGGDSYAALIEQFRKSA

SEQ ID NO: 221 - DNA, 879 bp, synthetic construct
  misc_feature 1..879: note = Imine reductase variant from Pseudonocardia spinosispora
  source 1..879: mol_type = other DNA
atgagtgattcacctgtgcccgtgacagttctgggtcttggtctgatgggtcaggccttagcgggagcgtttctggcagccggtcaccctacgacggtttggaatcgcagcgcagctaaagctgatgaactggttggtcgcggtgcaaccctggccgcgtctcccgcggctgccgtcgcagcgggtagtctgatcgttgtttgcgtcacagatcatcgtgcggtgcgcgaactgctggaaccacttggcgatgcactgccaggtcgcgttctggtcaacctgacgagcggtacgtcgcgtgaagcccgtgagaacgcagaacatactgcggctcagggagccacctacctggatggtgtgattctgaccattccaagcggcattggcaccccagaagctaggattctgtattcgggaccgcgcagtaccttcgatgaacatgaaagcgcactgcgcgcattaggtccgggggcgacctttgtaggggaagatcacggactggctaacctgtatgatgcagcaatgtcgagcatgatgtggggcctgctgaatggtttcctgcatggaaccgcactgctgggaaccgcgggcgtttcggcaacctctgtggttccgatgctgggtcaaggtctagaagcggtgactggtctaattgcgcgctacgcagatcagattgatgccggtgtctatccagcagacgatgccacgattgatacccagcgtgctgcaatgcagcacctggtcgaggagagccgtgcggcgggcatcaatggcgaacttccggcgtttgtgaccaaactggccgatcgcgcagtggcagaaggtcgtggtggtgactcttacgctgcactgattgaacagtttcgcaagtcagcttaa

SEQ ID NO: 222 - protein, 292 aa, synthetic construct
  REGION 1..292: note = Imine reductase variant from Pseudonocardia spinosispora
MSDSPVPVTVLGLGLMGQALAGAFLAAGHPTTVWNRSAAKADELVGRGATLAASPAAAVAAGSLIVVCVTDHRAVRELLEPLGDALPGRVLVNLTSGTSREARENAEHTAAQGATYLDGVILTIPSGIGTPEARILYSGPRSTFDEHESALRALGPGATFVGEDHGLANLYDAAMSSMMWGLLNGFLHGTALLGTAGVSATSVVPMLGQGLEAVTGLIARYADQIDAGVYPADDATIDTQRAAMQHLVEESRAAGINGELPAFVTKLADRAVAEGRGGDSYAALIEQFRKSA

SEQ ID NO: 223 - DNA, 879 bp, synthetic construct
  misc_feature 1..879: note = Imine reductase variant from Pseudonocardia spinosispora
  source 1..879: mol_type = other DNA
atgagtgattcacctgtgcccgtgacagttctgggtcttggtctgatgggtcaggccttagcgggagcgtttctggcagccggtcaccctacgacggtttggaatcgcagcgcagctaaagctgatgaactggttggtcgcggtgcaaccctggccgcgtctcccgcggctgccgtcgcagcgggtagtctgatcgttgtttgcgtcacagatcatcgtgcggtgcgcgaactgctggaaccacttggcgatgcactgccaggtcgcgttctggtcaacctgacgagcggtacgtcgcgtgaagcccgtgagaacgcagaacatactgcggctcagggagccacctacctggatggtgtgattctgaccattccaagcggcattggcaccccagaagctaggattctgtattcgggaccgcgcagtaccttcgatgaacatgaaagcgcactgcgcgcattaggtccgggggcgacctttgtaggggaagatcacggactggctaacctgtatgatgcagcaatgttgagcgttatgtggggcctgctgaatggtttcctgcatggaaccgcactgctgggaaccgcgggcgtttcggcaacctctgtggttccgatgctgggtcaaggttgggaagcggtgactggtctaattgcgcgctacgcagatcagattgatgccggtgtctatccagcagacgatgccacgattgatacccagcgtgctgcaatgcagcacctggtcgaggagagccgtgcggcgggcatcaatggcgaacttccggcgtttgtgaccaaactggccgatcgcgcagtggcagaaggtcgtggtggtgactcttacgctgcactgattgaacagtttcgcaagtcagcttaa

SEQ ID NO: 224 - protein, 292 aa, synthetic construct
  REGION 1..292: note = Imine reductase variant from Pseudonocardia spinosispora
MSDSPVPVTVLGLGLMGQALAGAFLAAGHPTTVWNRSAAKADELVGRGATLAASPAAAVAAGSLIVVCVTDHRAVRELLEPLGDALPGRVLVNLTSGTSREARENAEHTAAQGATYLDGVILTIPSGIGTPEARILYSGPRSTFDEHESALRALGPGATFVGEDHGLANLYDAAMLSVMWGLLNGFLHGTALLGTAGVSATSVVPMLGQGWEAVTGLIARYADQIDAGVYPADDATIDTQRAAMQHLVEESRAAGINGELPAFVTKLADRAVAEGRGGDSYAALIEQFRKSA

SEQ ID NO: 225 - DNA, 879 bp, synthetic construct
  misc_feature 1..879: note = Imine reductase variant from Pseudonocardia spinosispora
  source 1..879: mol_type = other DNA
atgagtgattcacctgtgcccgtgacagttctgggtcttggtctgatgggtcaggccttagcgggagcgtttctggcagccggtcaccctacgacggtttggaatcgcagcgcagctaaagctgatgaactggttggtcgcggtgcaaccctggccgcgtctcccgcggctgccgtcgcagcgggtagtctgatcgttgtttgcgtcacagatcatcgtgcggtgcgcgaactgctggaaccacttggcgatgcactgccaggtcgcgttctggtcaacctgacgagcggtacgtcgcgtgaagcccgtgagaacgcagaacatactgcggctcagggagccacctacctggatggtgtgattctgaccattccaagcggcattggcaccccagaagctacgattctgtattcgggaccgcgcagtaccttcgatgaacatgaaagcgcactgcgcgcattaggtccgggggcgacctttgtaggggaagatcacggactggctaacctgtatgatgcagcaatgtcgagcgttatgtggggcctgctgaatggtttcctgcatggaaccgcactgctgggaaccgcgggcgtttcggcaacctctgtggttccgatgctgggtcaaggttgggaagcggtgactggtataattgcgcgctacgcagatcagattgatgccggtgtctatccagcagacgatgccacgattgatacccagcgtgctgcaatgcagcacctggtcgaggagagccgtgcggcgggcatcaatggcgaacttccggcgtttgtgaccaaactggccgatcgcgcagtggcagaaggtcgtggtggtgactcttacgctgcactgattgaacagtttcgcaagtcagcttaa

SEQ ID NO: 226 - protein, 292 aa, synthetic construct
  REGION 1..292: note = Imine reductase variant from Pseudonocardia spinosispora
MSDSPVPVTVLGLGLMGQALAGAFLAAGHPTTVWNRSAAKADELVGRGATLAASPAAAVAAGSLIVVCVTDHRAVRELLEPLGDALPGRVLVNLTSGTSREARENAEHTAAQGATYLDGVILTIPSGIGTPEATILYSGPRSTFDEHESALRALGPGATFVGEDHGLANLYDAAMSSVMWGLLNGFLHGTALLGTAGVSATSVVPMLGQGWEAVTGIIARYADQIDAGVYPADDATIDTQRAAMQHLVEESRAAGINGELPAFVTKLADRAVAEGRGGDSYAALIEQFRKSA

SEQ ID NO: 227 - DNA, 879 bp, synthetic construct
  misc_feature 1..879: note = Imine reductase variant from Pseudonocardia spinosispora
  source 1..879: mol_type = other DNA
atgagtgattcacctgtgcccgtgacagttctgggtcttggtctgatgggtcaggccttagcgggagcgtttctggcagccggtcaccctacgacggtttggaatcgcagcgcagctaaagctgatgaactggttggtcgcggtgcaaccctggccgcgtctcccgcggctgccgtcgcagcgggtagtctgatcgttgtttgcgtcacagatcatcgtgcggtgcgcgaactgctggaaccacttggcgatgcactgccaggtcgcgttctggtcaacctgacgagcggtacgtcgcgtgaagcccgtgagaacgcagaacatactgcggctcagggagccacctacctggatggtgtgattctgaccattccaagcggcattggcaccccagaagctacgattctgtattcgggaccgcgcagtaccttcgatgaacatgaaagcgcactgcgcgcattaggtccgggggcgacctttgtaggggaagatcacggactggctaacctgtatgatgcagcaatgtcgagcattatgtggggcctgctgaatggtttcctgcatggaaccgcactgctgggaaccgcgggcgtttcggcaacctctgtggttccgatgctgggtcaaggtctagaagcgatgactggttggattgcgcgctacgcagatcagattgatgccggtgtctatccagcagacgatgccacgattgatacccagcgtgctgcaatgcagcacctggtcgaggagagccgtgcggcgggcatcaatggcgaacttccggcgtttgtgaccaaactggccgatcgcgcagtggcagaaggtcgtggtggtgactcttacgctgcactgattgaacagtttcgcaagtcagcttaa

SEQ ID NO: 228 - protein, 292 aa, synthetic construct
  REGION 1..292: note = Imine reductase variant from Pseudonocardia spinosispora
MSDSPVPVTVLGLGLMGQALAGAFLAAGHPTTVWNRSAAKADELVGRGATLAASPAAAVAAGSLIVVCVTDHRAVRELLEPLGDALPGRVLVNLTSGTSREARENAEHTAAQGATYLDGVILTIPSGIGTPEATILYSGPRSTFDEHESALRALGPGATFVGEDHGLANLYDAAMSSIMWGLLNGFLHGTALLGTAGVSATSVVPMLGQGLEAMTGWIARYADQIDAGVYPADDATIDTQRAAMQHLVEESRAAGINGELPAFVTKLADRAVAEGRGGDSYAALIEQFRKSA

SEQ ID NO: 229 - DNA, 879 bp, synthetic construct
  misc_feature 1..879: note = Imine reductase variant from Pseudonocardia spinosispora
  source 1..879: mol_type = other DNA
atgagtgattcacctgtgcccgtgacagttctgggtcttggtctgatgggtcaggccttagcgggagcgtttctggcagccggtcaccctacgacggtttggaatcgcagcgcagctaaagctgatgaactggttggtcgcggtgcaaccctggccgcgtctcccgcggctgccgtcgcagcgggtagtctgatcgttgtttgcgtcacagatcatcgtgcggtgcgcgaactgctggaaccacttggcgatgcactgccaggtcgcgttctggtcaacctgacgagcggtacgtcgcgtgaagcccgtgagaacgcagaacatactgcggctcagggagccacctacctggatggtgtgattctgaccattccaagcggcattggcaccccagaagctaccattctgtattcgggaccgcgcagtaccttcgatgaacatgaaagcgcactgcgcgcattaggtccgggggcgacctttgtaggggaagatcacggactggctaacctgtatgatgcagcaatgtcgagcatgatgtggggcctgctgaatggtttcctgcatggaaccgcactgctgggaaccgcgggcgtttcggcaacctctgtggttccgatgctgggtcaaggttgggaagcgatgactggtataattgcgcgctacgcagatcagattgatgccggtgtctatccagcagacgatgccacgattgatacccagcgtgctgcaatgcagcacctggtcgaggagagccgtgcggcgggcatcaatggcgaacttccggcgtttgtgaccaaactggccgatcgcgcagtggcagaaggtcgtggtggtgactcttacgctgcactgattgaacagtttcgcaagtcagcttaa

SEQ ID NO: 230 - protein, 292 aa, synthetic construct
  REGION 1..292: note = Imine reductase variant from Pseudonocardia spinosispora
MSDSPVPVTVLGLGLMGQALAGAFLAAGHPTTVWNRSAAKADELVGRGATLAASPAAAVAAGSLIVVCVTDHRAVRELLEPLGDALPGRVLVNLTSGTSREARENAEHTAAQGATYLDGVILTIPSGIGTPEATILYSGPRSTFDEHESALRALGPGATFVGEDHGLANLYDAAMSSMMWGLLNGFLHGTALLGTAGVSATSVVPMLGQGWEAMTGIIARYADQIDAGVYPADDATIDTQRAAMQHLVEESRAAGINGELPAFVTKLADRAVAEGRGGDSYAALIEQFRKSA

SEQ ID NO: 231 - DNA, 879 bp, synthetic construct
  misc_feature 1..879: note = Imine reductase variant from Pseudonocardia spinosispora
  source 1..879: mol_type = other DNA
atgagtgattcacctgtgcccgtgacagttctgggtcttggtctgatgggtcaggccttagcgggagcgtttctggcagccggtcaccctacgacggtttggaatcgcagcgcagctaaagctgatgaactggttggtcgcggtgcaaccctggccgcgtctcccgcggctgccgtcgcagcgggtagtctgatcgttgtttgcgtcacagatcatcgtgcggtgcgcgaactgctggaaccacttggcgatgcactgccaggtcgcgttctggtcaacctgacgagcggtacgtcgcgtgaagcccgtgagaacgcagaacatactgcggctcagggagccacctacctggatggtgtgattctgaccattccaagcggcattggcaccccagaagctaggattctgtattcgggaccgcgcagtaccttcgatgaacatgaaagcgcactgcgcgcattaggtccgggggcgacctttgtaggggaagatcacggactggctaacctgtatgatgcagcaatgtcgagcattatgtggggcctgctgaatggtttcctgcatggaaccgcactgctgggaaccgcgggcgtttcggcaacctctgtggttccgatgctgggtcaaggtctagaagcgatgactggttggattgcgcgctacgcagatcagattgatgccggtgtctatccagcagacgatgccacgattgatacccagcgtgctgcaatgcagcacctggtcgaggagagccgtgcggcgggcatcaatggcgaacttccggcgtttgtgaccaaactggccgatcgcgcagtggcagaaggtcgtggtggtgactcttacgctgcactgattgaacagtttcgcaagtcagcttaa

SEQ ID NO: 232 - protein, 292 aa, synthetic construct
  REGION 1..292: note = Imine reductase variant from Pseudonocardia spinosispora
MSDSPVPVTVLGLGLMGQALAGAFLAAGHPTTVWNRSAAKADELVGRGATLAASPAAAVAAGSLIVVCVTDHRAVRELLEPLGDALPGRVLVNLTSGTSREARENAEHTAAQGATYLDGVILTIPSGIGTPEARILYSGPRSTFDEHESALRALGPGATFVGEDHGLANLYDAAMSSIMWGLLNGFLHGTALLGTAGVSATSVVPMLGQGLEAMTGWIARYADQIDAGVYPADDATIDTQRAAMQHLVEESRAAGINGELPAFVTKLADRAVAEGRGGDSYAALIEQFRKSA

SEQ ID NO: 233 - DNA, 879 bp, synthetic construct
  misc_feature 1..879: note = Imine reductase variant from Pseudonocardia spinosispora
  source 1..879: mol_type = other DNA
atgagtgattcacctgtgcccgtgacagttctgggtcttggtctgatgggtcaggccttagcgggagcgtttctggcagccggtcaccctacgacggtttggaatcgcagcgcagctaaagctgatgaactggttggtcgcggtgcaaccctggccgcgtctcccgcggctgccgtcgcagcgggtagtctgatcgttgtttgcgtcacagatcatcgtgcggtgcgcgaactgctggaaccacttggcgatgcactgccaggtcgcgttctggtcaacctgacgagcggtacgtcgcgtgaagcccgtgagaacgcagaacatactgcggctcagggagccacctacctggatggtgtgattctgaccattccaagcggcattggcaccccagaagctaccattctgtattcgggaccgcgcagtaccttcgatgaacatgaaagcgcactgcgcgcattaggtccgggggcgacctttgtaggggaagatcacggactggctaacctgtatgatgcagcaatgtcgagcatgatgtggggcctgctgaatggtttcctgcatggaaccgcactgctgggaaccgcgggcgtttcggcaacctctgtggttccgatgctgggtcaaggttgggaagcgatgactggtataattgcgcgctacgcaaatcagattgatgccggtgtctatccagcagacgatgccacgattgatacccagcgtgctgcaatgcagcacctggtcgaggagagccgtgcggcgggcatcaatggcgaacttccggcgtttgtgaccaaactggccgatcgcgcagtggcagaaggtcgtggtggtgactcttacgctgcactgattgaacagtttcgcaagtcagcttaa

SEQ ID NO: 234 - protein, 292 aa, synthetic construct
  REGION 1..292: note = Imine reductase variant from Pseudonocardia spinosispora
MSDSPVPVTVLGLGLMGQALAGAFLAAGHPTTVWNRSAAKADELVGRGATLAASPAAAVAAGSLIVVCVTDHRAVRELLEPLGDALPGRVLVNLTSGTSREARENAEHTAAQGATYLDGVILTIPSGIGTPEATILYSGPRSTFDEHESALRALGPGATFVGEDHGLANLYDAAMSSMMWGLLNGFLHGTALLGTAGVSATSVVPMLGQGWEAMTGIIARYANQIDAGVYPADDATIDTQRAAMQHLVEESRAAGINGELPAFVTKLADRAVAEGRGGDSYAALIEQFRKSA

SEQ ID NO: 235 - DNA, 879 bp, synthetic construct
  misc_feature 1..879: note = Imine reductase variant from Pseudonocardia spinosispora
  source 1..879: mol_type = other DNA
atgagtgattcacctgtgcccgtgacagttctgggtcttggtctgatgggtcaggccttagcgggagcgtttctggcagccggtcaccctacgacggtttggaatcgcagcgcagctaaagctgatgaactggttggtcgcggtgcaaccctggccgcgtctcccgcggctgccgtcgcagcgggtagtctgatcgttgtttgcgtcacagatcatcgtgcggtgcgcgaactgctggaaccacttggcgatgcactgccaggtcgcgttctggtcaacctgacgagcggtacgtcgcgtgaagcccgtgagaacgcagaacatactgcggctcagggagccacctacctggatggtgtgattctgaccattccaagcggcattggcaccccagaagctaccattctgtattcgggaccgcgcagtaccttcgatgaacatgaaagcgcactgcgcgcattaggtccgggggcgacctttgtaggggaagatcacggactggctaacctgtatgatgcagcaatgtcgagcatgatgtggggcctgctgaatggtttcctgcatggaaccgcactgctgggaaccgcgggcgtttcggcaacctctgtggttccgatgctgggtcaaggttgggaagcgatgactggtataattgcgcgctacgcagatcagattgatgccggtgtctatccagcagacgatgccacgattgatacccagcgtgctgcaatgcagcacctggtcgaggagagccgtgcggcgggcatcaatggcgaacttccggcgtttgtgaccaaactggccgatcgcgcagtggcagaaggtcgtggtggtgtttcttacgctgcactgattgaacagtttcgcaagtcagcttaa

SEQ ID NO: 236 - protein, 292 aa, synthetic construct
  REGION 1..292: note = Imine reductase variant from Pseudonocardia spinosispora
MSDSPVPVTVLGLGLMGQALAGAFLAAGHPTTVWNRSAAKADELVGRGATLAASPAAAVAAGSLIVVCVTDHRAVRELLEPLGDALPGRVLVNLTSGTSREARENAEHTAAQGATYLDGVILTIPSGIGTPEATILYSGPRSTFDEHESALRALGPGATFVGEDHGLANLYDAAMSSMMWGLLNGFLHGTALLGTAGVSATSVVPMLGQGWEAMTGIIARYADQIDAGVYPADDATIDTQRAAMQHLVEESRAAGINGELPAFVTKLADRAVAEGRGGVSYAALIEQFRKSA

SEQ ID NO: 237 - DNA, 879 bp, synthetic construct
  misc_feature 1..879: note = Imine reductase variant from Pseudonocardia spinosispora
  source 1..879: mol_type = other DNA
atgagtgattcacctgtgcccgtgacagttctgggtcttggtctgatgggtcaggccttagcgggagcgtttctggcagccggtcaccctacgacggtttggaatcgcagcgcagctaaagctgatgaactggttggtcgcggtgcaaccctggccgcgtctcccgcggctgccgtcgcagcgggtagtctgatcgttgtttgcgtcacagatcatcgtgcggtgcgcgaactgctggaaccacttggcgatgcactgccaggtcgcgttctggtcaacctgacgagcggtacgtcgcgtgaagcccgtgagaacgcagaacatactgcggctcagggagccacctacctggatggtgtgattctgaccattccaagcggcattggcaccccagaagctaccattctgtattcgggaccgcgcagtaccttcgatgaacatgaaagcgcactgcgcgcattaggtccgggggcgacctttgtaggggaagatcacggactggctaacctgtatgatgcagcaatgtcgagcatgatgtggggcctgctgaatggtttcctgcatggaaccgcactgctgggaaccgcgggcgtttcggcaacctctgtggttccgatgctgggtcaaggttgggaagcgatgactggtataattgcgcgctacgcagatcagattgatgttggtgtctatccagcagacgatgccacgattgatacccagcgtgctgcaatgcagcacctggtcgaggagagccgtgcggcgggcatcaatggcgaacttccggcgtttgtgaccaaactggccgatcgcgcagtggcagaaggtcgtggtggtgactcttacgctgcactgattgaacagtttcgcaagtcagcttaa

SEQ ID NO: 238 - protein, 292 aa, synthetic construct
  REGION 1..292: note = Imine reductase variant from Pseudonocardia spinosispora
MSDSPVPVTVLGLGLMGQALAGAFLAAGHPTTVWNRSAAKADELVGRGATLAASPAAAVAAGSLIVVCVTDHRAVRELLEPLGDALPGRVLVNLTSGTSREARENAEHTAAQGATYLDGVILTIPSGIGTPEATILYSGPRSTFDEHESALRALGPGATFVGEDHGLANLYDAAMSSMMWGLLNGFLHGTALLGTAGVSATSVVPMLGQGWEAMTGIIARYADQIDVGVYPADDATIDTQRAAMQHLVEESRAAGINGELPAFVTKLADRAVAEGRGGDSYAALIEQFRKSA

SEQ ID NO: 239 - DNA, 879 bp, synthetic construct
  misc_feature 1..879: note = Imine reductase variant from Pseudonocardia spinosispora
  source 1..879: mol_type = other DNA
atgagtgattcacctgtgcccgtgacagttctgggtcttggtctgatgggtcaggccttagcgggagcgtttctggcagccggtcaccctacgacggtttggaatcgcagcgcagctaaagctgatgaactggttggtcgcggtgcaaccctggccgcgtctcccgcggctgccgtcgcagcgggtagtctgatcgttgtttgcgtcacagatcatcgtgcggtgcgcgaactgctggaaccacttggcgatgcactgccaggtcgcgttctggtcaacctgacgagcggtacgtcgcgtgaagcccgtgagaacgcagaacatactgcggctcagggagccacctacctggatggtgtgattctgaccattccaagcaggattggcaccccagaagctaccattctgtattcgggaccgcgcagtaccttcgatgaacatgaaagcgcactgcgcgcattaggtccgggggcgacctttgtaggggaagatcacggactggctaacctgtatgatgcagcaatgtcgagcatgatgtggggcctgctgaatggtttcctgcatggaaccgcactgctgggaaccgcgggcgtttcggcaacctctgtggttccgatgctgggtcaaggttgggaagcgatgactggtataattgcgcgctacgcagatcagattgatgccggtgtctatccagcagacgatgccacgattgatacccagcgtgctgcaatgcagcacctggtcgaggagagccgtgcggcgggcatcaatggcgaacttccggcgtttgtgaccaaactggccgatcgcgcagtggcagaaggtcgtggtggtgactcttacgctgcactgattgaacagtttcgcaagtcagcttaa

SEQ ID NO: 240 - protein, 292 aa, synthetic construct
  REGION 1..292: note = Imine reductase variant from Pseudonocardia spinosispora
MSDSPVPVTVLGLGLMGQALAGAFLAAGHPTTVWNRSAAKADELVGRGATLAASPAAAVAAGSLIVVCVTDHRAVRELLEPLGDALPGRVLVNLTSGTSREARENAEHTAAQGATYLDGVILTIPSRIGTPEATILYSGPRSTFDEHESALRALGPGATFVGEDHGLANLYDAAMSSMMWGLLNGFLHGTALLGTAGVSATSVVPMLGQGWEAMTGIIARYADQIDAGVYPADDATIDTQRAAMQHLVEESRAAGINGELPAFVTKLADRAVAEGRGGDSYAALIEQFRKSA

SEQ ID NO: 241 - DNA, 879 bp, synthetic construct
  misc_feature 1..879: note = Imine reductase variant from Pseudonocardia spinosispora
  source 1..879: mol_type = other DNA
atgagtgattcacctgtgcccgtgacagttctgggtcttggtctgatgggtcaggccttagcgggagcgtttctggcagccggtcaccctacgacggtttggaatcgcagcgcagctaaagctgatgaactggttggtcgcggtgcaaccctggccgcgtctcccgcggctgccgtcgcagcgggtagtctgatcgttgtttgcgtcacagatcatcgtgcggtgcgcgaactgctggaaccacttggcgatgcactgccaggtcgcgttctggtcaacctgacgagcggtacgtcgcgtgaagcccgtgagaacgcagaacatactgcggctcagggagccacctacctggatggtgtgattctgaccattccaagcggcattggcaccccagaagctaccattctgtattcgggaccgcgcagtaccttcgatgaacatgaaagcgcactgcgcgcattaggtccgggggcgacctttgtaggggaagatcacggactggctaacctgtatgatgcagcaatgtcgagcatgatgtggggcctgctgaatggtttcctgcatggaaccgcactgctgggaaccgcgggcgtttcggcaacctctgtggttccgatgctgggtcaaggttgggaagcgatgactagtataattgcgcgctacgcagatcagattgatgccggtgtctatccagcagacgatgccacgattgatacccagcgtgctgcaatgcagcacctggtcgaggagagccgtgcggcgggcatcaatggcgaacttccggcgtttgtgaccaaactggccgatcgcgcagtggcagaaggtcgtggtggtgactcttacgctgcactgattgaacagtttcgcaagtcagcttaa

SEQ ID NO: 242 - protein, 292 aa, synthetic construct
  REGION 1..292: note = Imine reductase variant from Pseudonocardia spinosispora
MSDSPVPVTVLGLGLMGQALAGAFLAAGHPTTVWNRSAAKADELVGRGATLAASPAAAVAAGSLIVVCVTDHRAVRELLEPLGDALPGRVLVNLTSGTSREARENAEHTAAQGATYLDGVILTIPSGIGTPEATILYSGPRSTFDEHESALRALGPGATFVGEDHGLANLYDAAMSSMMWGLLNGFLHGTALLGTAGVSATSVVPMLGQGWEAMTSIIARYADQIDAGVYPADDATIDTQRAAMQHLVEESRAAGINGELPAFVTKLADRAVAEGRGGDSYAALIEQFRKSA

SEQ ID NO: 243 - DNA, 879 bp, synthetic construct
  misc_feature 1..879: note = Imine reductase variant from Pseudonocardia spinosispora
  source 1..879: mol_type = other DNA
atgagtgattcacctgtgcccgtgacagttctgggtcttggtctgatgggtcaggccttagcgggagcgtttctggcagccggtcaccctacgacggtttggaatcgcagcgcagctaaagctgatgaactggttggtcgcggtgcaaccctggccgcgtctcccgcggctgccgtcgcagcgggtagtctgatcgttgtttgcgtcacagatcatcgtgcggtgcgcgaactgctggaaccacttggcgatgcactgccaggtcgcgttctggtcaacctgacgagcggtacgtcgcgtgaagcccgtgagaacgcagaacatactgcggctcagggagccacctacctggatggtgtgattctgaccattccaagcggcattggcaccccagaagctaccattctgtattcgggaccgcgcagtaccttcgatgaacatgaaagcgcactgcgcgcattaggtccgggggcgacctttgtaggggaagatcacggactggctaacctgtatgatgcaatgatgtcgagcatgatgtggggcctgctgaatggtttcctgcatggaaccgcactgctgggaaccgcgggcgtttcggcaacctctgtggttccgatgctgggtcaaggttgggaagcgatgactggtataattgcgcgctacgcagatcagattgatgccggtgtctatccagcagacgatgccacgattgatacccagcgtgctgcaatgcagcacctggtcgaggagagccgtgcggcgggcatcaatggcgaacttccggcgtttgtgaccaaactggccgatcgcgcagtggcagaaggtcgtggtggtgactcttacgctgcactgattgaacagtttcgcaagtcagcttaa

SEQ ID NO: 244 - protein, 292 aa, synthetic construct
  REGION 1..292: note = Imine reductase variant from Pseudonocardia spinosispora
MSDSPVPVTVLGLGLMGQALAGAFLAAGHPTTVWNRSAAKADELVGRGATLAASPAAAVAAGSLIVVCVTDHRAVRELLEPLGDALPGRVLVNLTSGTSREARENAEHTAAQGATYLDGVILTIPSGIGTPEATILYSGPRSTFDEHESALRALGPGATFVGEDHGLANLYDAMMSSMMWGLLNGFLHGTALLGTAGVSATSVVPMLGQGWEAMTGIIARYADQIDAGVYPADDATIDTQRAAMQHLVEESRAAGINGELPAFVTKLADRAVAEGRGGDSYAALIEQFRKSA

SEQ ID NO: 245 - DNA, 879 bp, synthetic construct
  misc_feature 1..879: note = Imine reductase variant from Pseudonocardia spinosispora
  source 1..879: mol_type = other DNA
atgagtgattcacctgtgcccgtgacagttctgggtcttggtctgatgggtcaggccttagcgggagcgtttctggcagccggtcaccctacgacggtttggaatcgcagcgcagctaaagctgatgaactggttggtcgcggtgcaaccctggccgcgtctcccgcggctgccgtcgcagcgggtagtctgatcgttgtttgcgtcacagatcatcgtgcggtgcgcgaactgctggaaccacttggcgatgcactgccaggtcgcgttctggtcaacctgacgagcggtacgtcgcgtgaagcccgtgagaacgcagaacatactgcggctcagggagccacctacctggatggtgtgattctgaccattccaagcggcattggcaccccagaagctaccattctgtattcgggaccgcgcagtaccttcgatgaacatgaaagcgcactgcgcgcattaggtccgggggcgacctttgtaggggaagatcacggactggctaacctgtatgatgcagcaatgtcgagcatgatgtggggcctgctgaatggtttcctgcatggaaccgcactgctgggaaccgcgggcgtttcggcaacctctgtggttccgatgctgggtcaaggttggcatgcgatgactggtataattgcgcgctacgcagatcagattgatgccggtgtctatccagcagacgatgccacgattgatacccagcgtgctgcaatgcagcacctggtcgaggagagccgtgcggcgggcatcaatggcgaacttccggcgtttgtgaccaaactggccgatcgcgcagtggcagaaggtcgtggtggtgactcttacgctgcactgattgaacagtttcgcaagtcagcttaa

SEQ ID NO: 246 - protein, 292 aa, synthetic construct
  REGION 1..292: note = Imine reductase variant from Pseudonocardia spinosispora
MSDSPVPVTVLGLGLMGQALAGAFLAAGHPTTVWNRSAAKADELVGRGATLAASPAAAVAAGSLIVVCVTDHRAVRELLEPLGDALPGRVLVNLTSGTSREARENAEHTAAQGATYLDGVILTIPSGIGTPEATILYSGPRSTFDEHESALRALGPGATFVGEDHGLANLYDAAMSSMMWGLLNGFLHGTALLGTAGVSATSVVPMLGQGWHAMTGIIARYADQIDAGVYPADDATIDTQRAAMQHLVEESRAAGINGELPAFVTKLADRAVAEGRGGDSYAALIEQFRKSA

SEQ ID NO: 247 - DNA, 879 bp, synthetic construct
  misc_feature 1..879: note = Imine reductase variant from Pseudonocardia spinosispora
  source 1..879: mol_type = other DNA
atgagtgattcacctgtgcccgtgacagttctgggtcttggtctgatgggtcaggccttagcgggagcgtttctggcagccggtcaccctacgacggtttggaatcgcagcgcagctaaagctgatgaactggttggtcgcggtgcaaccctggccgcgtctcccgcggctgccgtcgcagcgggtagtctgatcgttgtttgcgtcacagatcatcgtgcggtgcgcgaactgctggaaccacttggcgatgcactgccaggtcgcgttctggtcaacctgacgagcggtacgtcgcgtgaagcccgtgagaacgcagaacatactgcggctcagggagccacctacctggatggtgtgattctgaccattccaagcggcattggcaccccagaagctaccattctgtattcgggaccgcgcagtaccttcgatgaacatgaaagcgcactgcgcgcattaggtccgggggcgacctttgtaggggaagatcacggactggctaacctgtatgatgcagcaatgtcgagcatgatgtggggcctgctgaatggtttcctgcatggaaccgcactgctgggaaccgcgggcgtttcggcaacctctgtggttccgatgctgggtcaaggttggagggcgatgactggtataattgcgcgctacgcagatcagattgatgccggtgtctatccagcagacgatgccacgattgatacccagcgtgctgcaatgcagcacctggtcgaggagagccgtgcggcgggcatcaatggcgaacttccggcgtttgtgaccaaactggccgatcgcgcagtggcagaaggtcgtggtggtgactcttacgctgcactgattgaacagtttcgcaagtcagcttaa

SEQ ID NO: 248 - protein, 292 aa, synthetic construct
  REGION 1..292: note = Imine reductase variant from Pseudonocardia spinosispora
MSDSPVPVTVLGLGLMGQALAGAFLAAGHPTTVWNRSAAKADELVGRGATLAASPAAAVAAGSLIVVCVTDHRAVRELLEPLGDALPGRVLVNLTSGTSREARENAEHTAAQGATYLDGVILTIPSGIGTPEATILYSGPRSTFDEHESALRALGPGATFVGEDHGLANLYDAAMSSMMWGLLNGFLHGTALLGTAGVSATSVVPMLGQGWRAMTGIIARYADQIDAGVYPADDATIDTQRAAMQHLVEESRAAGINGELPAFVTKLADRAVAEGRGGDSYAALIEQFRKSA

SEQ ID NO: 249 - DNA, 879 bp, synthetic construct
  misc_feature 1..879: note = Imine reductase variant from Pseudonocardia spinosispora
  source 1..879: mol_type = other DNA
atgagtgattcacctgtgcccgtgacagttctgggtcttggtctgatgggtcaggccttagcgggagcgtttctggcagccggtcaccctacgacggtttggaatcgcagcgcagctaaagctgatgaactggttggtcgcggtgcaaccctggccgcgtctcccgcggctgccgtcgcagcgggtagtctgatcgttgtttgcgtcacagatcatcgtgcggtgcgcgaactgctggaaccacttggcgatgcactgccaggtcgcgttctggtcaacctgacgagcggtacgtcgcgtgaagcccgtgagaacgcagaacatactgcggctcagggagccacctacctggatggtgtgattctgaccattccaagcggcattggcaccccagaagctaccattctgtattcgggaccgcgcagtaccttcgatgaacatgaaagcgcactgcgcgcattaggtccgggggcgacctttgtaggggaagatcacggactggctaacctgtatgatgcagcaatgtcgagcatgatgtggggcctgctgaatggtttcctgcatggaaccgcactgctgggaaccgcgggcgtttcggcaacctctgtggttccgatgctgggtcaaggttggaaagcgatgactggtataattgcgcgctacgcagatcagattgatgccggtgtctatccagcagacgatgccacgattgatacccagcgtgctgcaatgcagcacctggtcgaggagagccgtgcggcgggcatcaatggcgaacttccggcgtttgtgaccaaactggccgatcgcgcagtggcagaaggtcgtggtggtgactcttacgctgcactgattgaacagtttcgcaagtcagcttaa

SEQ ID NO: 250 - protein, 292 aa, synthetic construct
  REGION 1..292: note = Imine reductase variant from Pseudonocardia spinosispora
MSDSPVPVTVLGLGLMGQALAGAFLAAGHPTTVWNRSAAKADELVGRGATLAASPAAAVAAGSLIVVCVTDHRAVRELLEPLGDALPGRVLVNLTSGTSREARENAEHTAAQGATYLDGVILTIPSGIGTPEATILYSGPRSTFDEHESALRALGPGATFVGEDHGLANLYDAAMSSMMWGLLNGFLHGTALLGTAGVSATSVVPMLGQGWKAMTGIIARYADQIDAGVYPADDATIDTQRAAMQHLVEESRAAGINGELPAFVTKLADRAVAEGRGGDSYAALIEQFRKSA

SEQ ID NO: 251 - DNA, 879 bp, synthetic construct
  misc_feature 1..879: note = Imine reductase variant from Pseudonocardia spinosispora
  source 1..879: mol_type = other DNA
atgagtgattcacctgtgcccgtgacagttctgggtcttggtctgatgggtcaggccttagcgggagcgtttctggcagccggtcaccctacgacggtttggaatcgcagcgcagctaaagctgatgaactggttggtcgcggtgcaaccctggccgcgtctcccgcggctgccgtcgcagcgggtagtctgatcgttgtttgcgtcacagatcatcgtgcggtgcgcgaactgctggaaccacttggcgatgcactgccaggtcgcgttctggtcaacctgacgagcggtacgtcgcgtgaagcccgtgagaacgcagaacatactgcggctcagggagccacctacctggatggtgtgattctgaccattccaagcggcattggcaccccagaagctaccattctgtattcgggaccgcgcagtaccttcgatgaacatgaaagcgcactgcgcgcattaggtccgggggcgacctttgtaggggaagatcacggactggctaacctgtatgatgcagcaatgtcgagcatgatgtggggcctgctgaatggtttcctgcatggaaccgcactgctgggaaccgcgggcgtttcggcaacctctgtggttccgatgctgggtagtggttgggaagcgatgactggtataattgcgcgctacgcagatcagattgatgccggtgtctatccagcagacgatgccacgattgatacccagcgtgctgcaatgcagcacctggtcgaggagagccgtgcggcgggcatcaatggcgaacttccggcgtttgtgaccaaactggccgatcgcgcagtggcagaaggtcgtggtggtgactcttacgctgcactgattgaacagtttcgcaagtcagcttaa

SEQ ID NO: 252 - protein, 292 aa, synthetic construct
  REGION 1..292: note = Imine reductase variant from Pseudonocardia spinosispora
MSDSPVPVTVLGLGLMGQALAGAFLAAGHPTTVWNRSAAKADELVGRGATLAASPAAAVAAGSLIVVCVTDHRAVRELLEPLGDALPGRVLVNLTSGTSREARENAEHTAAQGATYLDGVILTIPSGIGTPEATILYSGPRSTFDEHESALRALGPGATFVGEDHGLANLYDAAMSSMMWGLLNGFLHGTALLGTAGVSATSVVPMLGSGWEAMTGIIARYADQIDAGVYPADDATIDTQRAAMQHLVEESRAAGINGELPAFVTKLADRAVAEGRGGDSYAALIEQFRKSA

SEQ ID NO: 253 - DNA, 879 bp, synthetic construct
  misc_feature 1..879: note = Imine reductase variant from Pseudonocardia spinosispora
  source 1..879: mol_type = other DNA
atgagtgattcacctgtgcccgtgacagttctgggtcttggtctgatgggtcaggccttagcgggagcgtttctggcagccggtcaccctacgacggtttggaatcgcagcgcagctaaagctgatgaactggttggtcgcggtgcaaccctggccgcgtctcccgcggctgccgtcgcagcgggtagtctgatcgttgtttgcgtcacagatcatcgtgcggtgcgcgaactgctggaaccacttggcgatgcactgccaggtcgcgttctggtcaacctgacgagcggtacgtcgcgtgaagcccgtgagaacgcagaacatactgcggctcagggagccacctacctggatggtgtgattctgaccattccaagcggcattggcaccccagaagctaccattctgtattcgggaccgcgcagtaccttcgatgaacatgaaagcgcactgcgcgcattaggtccgggggcgacctttgtaggggaagatcacggactggctaacctgtatgatgcagcaatgtcgagcatgatgtggggcctgctgaatggtttcctgcatggaaccgcactgctgggaaccgcgggcgtttcggcaacctctgtggttccgatgctgggtcaaggttgggaagcgatgactcgtataattgcgcgctacgcagatcagattgatgccggtgtctatccagcagacgatgccacgattgatacccagcgtgctgcaatgcagcacctggtcgaggagagccgtgcggcgggcatcaatggcgaacttccggcgtttgtgaccaaactggccgatcgcgcagtggcagaaggtcgtggtggtgactcttacgctgcactgattgaacagtttcgcaagtcagcttaa

SEQ ID NO: 254 - protein, 292 aa, synthetic construct
  REGION 1..292: note = Imine reductase variant from Pseudonocardia spinosispora
MSDSPVPVTVLGLGLMGQALAGAFLAAGHPTTVWNRSAAKADELVGRGATLAASPAAAVAAGSLIVVCVTDHRAVRELLEPLGDALPGRVLVNLTSGTSREARENAEHTAAQGATYLDGVILTIPSGIGTPEATILYSGPRSTFDEHESALRALGPGATFVGEDHGLANLYDAAMSSMMWGLLNGFLHGTALLGTAGVSATSVVPMLGQGWEAMTRIIARYADQIDAGVYPADDATIDTQRAAMQHLVEESRAAGINGELPAFVTKLADRAVAEGRGGDSYAALIEQFRKSA

SEQ ID NO: 255 - DNA, 879 bp, synthetic construct
  misc_feature 1..879: note = Imine reductase variant from Pseudonocardia spinosispora
  source 1..879: mol_type = other DNA
atgagtgattcacctgtgcccgtgacagttctgggtcttggtctgatgggtcaggccttagcgggagcgtttctggcagccggtcaccctacgacggtttggaatcgcagcgcagctaaagctgatgaactggttggtcgcggtgcaaccctggccgcgtctcccgcggctgccgtcgcagcgggtagtctgatcgttgtttgcgtcacagatcatcgtgcggtgcgcgaactgctggaaccacttggcgatgcactgccaggtcgcgttctggtcaacctgacgagcggtacgtcgcgtgaagcccgtgagaacgcagaacatactgcggctcagggagccacctacctggatggtgtgattctgaccattccaagcggcattggcaccccagaagctaccattctgtattcgggaccgcgcagtaccttcgatgaacatgaaagcgcactgcgcgcattaggtccgggggcgacctttgtaggggaagatcacggactggctaacctgtatgatgcagcaatgtcgagcatgatgtggggcctgctgaatggtttcctgcatggaaccgcactgctgggaaccgcgggcgtttcggcaacctctgtggttccgcttctgggtcaaggttgggaagcgatgactggtataattgcgcgctacgcagatcagattgatgccggtgtctatccagcagacgatgccacgattgatacccagcgtgctgcaatgcagcacctggtcgaggagagccgtgcggcgggcatcaatggcgaacttccggcgtttgtgaccaaactggccgatcgcgcagtggcagaaggtcgtggtggtgactcttacgctgcactgattgaacagtttcgcaagtcagcttaa

SEQ ID NO: 256 - protein, 292 aa, synthetic construct
  REGION 1..292: note = Imine reductase variant from Pseudonocardia spinosispora
MSDSPVPVTVLGLGLMGQALAGAFLAAGHPTTVWNRSAAKADELVGRGATLAASPAAAVAAGSLIVVCVTDHRAVRELLEPLGDALPGRVLVNLTSGTSREARENAEHTAAQGATYLDGVILTIPSGIGTPEATILYSGPRSTFDEHESALRALGPGATFVGEDHGLANLYDAAMSSMMWGLLNGFLHGTALLGTAGVSATSVVPLLGQGWEAMTGIIARYADQIDAGVYPADDATIDTQRAAMQHLVEESRAAGINGELPAFVTKLADRAVAEGRGGDSYAALIEQFRKSA

SEQ ID NO: 257 - DNA, 879 bp, synthetic construct
  misc_feature 1..879: note = Imine reductase variant from Pseudonocardia spinosispora
  source 1..879: mol_type = other DNA
atgagtgattcacctgtgcccgtgacagttctgggtcttggtctgatgggtcaggccttagcgggagcgtttctggcagccggtcaccctacgacggtttggaatcgcagcgcagctaaagctgatgaactggttggtcgcggtgcaaccctggccgcgtctcccgcggctgccgtcgcagcgggtagtctgatcgttgtttgcgtcacagatcatcgtgcggtgcgcgaactgctggaaccacttggcgatgcactgccaggtcgcgttctggtcaacctgacgagcggtacgtcgcgtgaagcccgtgagaacgcagaacatactgcggctcagggagccacctacctggatggtgtgattctgaccattccaagcggcattggcaccccagaagctcttattctgtattcgggaccgcgcagtaccttcgatgaacatgaaagcgcactgcgcgcattaggtccgggggcgacctttgtaggggaagatcacggactggctaacctgtatgatgcagcaatgtcgagcatgatgtggggcctgctgaatggtttcctgcatggaaccgcactgctgggaaccgcgggcgtttcggcaacctctgtggttccgatgctgggtcaaggttgggaagcgatgactggtataattgcgcgctacgcagatcagattgatgccggtgtctatccagcagacgatgccacgattgatacccagcgtgctgcaatgcagcacctggtcgaggagagccgtgcggcgggcatcaatggcgaacttccggcgtttgtgaccaaactggccgatcgcgcagtggcagaaggtcgtggtggtgactcttacgctgcactgattgaacagtttcgcaagtcagcttaa

SEQ ID NO: 258 - protein, 292 aa, synthetic construct
  REGION 1..292: note = Imine reductase variant from Pseudonocardia spinosispora
MSDSPVPVTVLGLGLMGQALAGAFLAAGHPTTVWNRSAAKADELVGRGATLAASPAAAVAAGSLIVVCVTDHRAVRELLEPLGDALPGRVLVNLTSGTSREARENAEHTAAQGATYLDGVILTIPSGIGTPEALILYSGPRSTFDEHESALRALGPGATFVGEDHGLANLYDAAMSSMMWGLLNGFLHGTALLGTAGVSATSVVPMLGQGWEAMTGIIARYADQIDAGVYPADDATIDTQRAAMQHLVEESRAAGINGELPAFVTKLADRAVAEGRGGDSYAALIEQFRKSA

SEQ ID NO: 259 - DNA, 879 bp, synthetic construct
  misc_feature 1..879: note = Imine reductase variant from Pseudonocardia spinosispora
  source 1..879: mol_type = other DNA
atgagtgattcacctgtgcccgtgacagttctgggtcttggtctgatgggtcaggccttagcgggagcgtttctggcagccggtcaccctacgacggtttggaatcgcagcgcagctaaagctgatgaactggttggtcgcggtgcaaccctggccgcgtctcccgcggctgccgtcgcagcgggtagtctgatcgttgtttgcgtcacagatcatcgtgcggtgcgcgaactgctggaaccacttggcgatgcactgccaggtcgcgttctggtcaacctgacgagcggtacgtcgcgtgaagcccgtgagaacgcagaacatactgcggctcagggagccacctacctggatggtgtgattctgaccattccaagcggcattggccgtccagaagctaccattctgtattcgggaccgcgcagtaccttcgatgaacatgaaagcgcactgcgcgcattaggtccgggggcgacctttgtaggggaagatcacggactggctaacctgtatgatgcagcaatgtcgagcatgatgtggggcctgctgaatggtttcctgcatggaaccgcactgctgggaaccgcgggcgtttcggcaacctctgtggttccgatgctgggtcaaggttgggaagcgatgactggtataattgcgcgctacgcagatcagattgatgccggtgtctatccagcagacgatgccacgattgatacccagcgtgctgcaatgcagcacctggtcgaggagagccgtgcggcgggcatcaatggcgaacttccggcgtttgtgaccaaactggccgatcgcgcagtggcagaaggtcgtggtggtgactcttacgctgcactgattgaacagtttcgcaagtcagcttaa

SEQ ID NO: 260 - protein, 292 aa, synthetic construct
  REGION 1..292: note = Imine reductase variant from Pseudonocardia spinosispora
MSDSPVPVTVLGLGLMGQALAGAFLAAGHPTTVWNRSAAKADELVGRGATLAASPAAAVAAGSLIVVCVTDHRAVRELLEPLGDALPGRVLVNLTSGTSREARENAEHTAAQGATYLDGVILTIPSGIGRPEATILYSGPRSTFDEHESALRALGPGATFVGEDHGLANLYDAAMSSMMWGLLNGFLHGTALLGTAGVSATSVVPMLGQGWEAMTGIIARYADQIDAGVYPADDATIDTQRAAMQHLVEESRAAGINGELPAFVTKLADRAVAEGRGGDSYAALIEQFRKSA

SEQ ID NO: 261 - DNA, 879 bp, synthetic construct
  misc_feature 1..879: note = Imine reductase variant from Pseudonocardia spinosispora
  source 1..879: mol_type = other DNA
atgagtgattcacctgtgcccgtgacagttctgggtcttggtctgatgggtcaggccttagcgggagcgtttctggcagccggtcaccctacgacggtttggaatcgcagcgcagctaaagctgatgaactggttggtcgcggtgcaaccctggccgcgtctcccgcggctgccgtcgcagcgggtagtctgatcgttgtttgcgtcacagatcatcgtgcggtgcgcgaactgctggaaccacttggcgatgcactgccaggtcgcgttctggtcaacctgacgagcggtacgtcgcgtgaagcccgtgagaacgcagaacatactgcggctcagggagccacctacctggatggtgtgattctgaccattccaagcggcattggcaccccagaagctaccattctgtattcgggaccgcgcagtaccttcgatgaacatgaaagcgcactgcgcgcattaggtccgggggcgacctttgtaggggaagatcacggactggctaacctgtatgatgcagcaatgtcgagcatgatgtggggcctgctgaatggtttcctgcatggaaccgcactgctgggaaccgcgggcgtttcggcaacctctgtggttccgatgctgggtcaaggttgggaagcgatgactaatataattgcgcgctacgcagatcagattgatgccggtgtctatccagcagacgatgccacgattgatacccagcgtgctgcaatgcagcacctggtcgaggagagccgtgcggcgggcatcaatggcgaacttccggcgtttgtgaccaaactggccgatcgcgcagtggcagaaggtcgtggtggtgactcttacgctgcactgattgaacagtttcgcaagtcagcttaa

SEQ ID NO: 262 - protein, 292 aa, synthetic construct
  REGION 1..292: note = Imine reductase variant from Pseudonocardia spinosispora
MSDSPVPVTVLGLGLMGQALAGAFLAAGHPTTVWNRSAAKADELVGRGATLAASPAAAVAAGSLIVVCVTDHRAVRELLEPLGDALPGRVLVNLTSGTSREARENAEHTAAQGATYLDGVILTIPSGIGTPEATILYSGPRSTFDEHESALRALGPGATFVGEDHGLANLYDAAMSSMMWGLLNGFLHGTALLGTAGVSATSVVPMLGQGWEAMTNIIARYADQIDAGVYPADDATIDTQRAAMQHLVEESRAAGINGELPAFVTKLADRAVAEGRGGDSYAALIEQFRKSA

SEQ ID NO: 263 - DNA, 879 bp, synthetic construct
  misc_feature 1..879: note = Imine reductase variant from Pseudonocardia spinosispora
  source 1..879: mol_type = other DNA
atgagtgattcacctgtgcccgtgacagttctgggtcttggtctgatgggtcaggccttagcgggagcgtttctggcagccggtcaccctacgacggtttggaatcgcagcgcagctaaagctgatgaactgattggtcgcggtgcaaccctggccgcgtctcccgcggctgccgtcgcagcgggtagtctgatcgttgtttgcgtcacagatcatcgtgcggtgcgcgaactgctggaaccacttggcgatgcactgccaggtcgcgttctggtcaacctgacgagcggtacgtcgcgtgaagcccgtgagaacgcagaacatactgcggctcagggagccacctacctggatggtgtgattctgaccattccaagcggcattggcaccccagaagctaccattctgtattcgggaccgcgcagtaccttcgatgaacatgaaagcgcactgcgcgcattaggtccgggggcgacctttgtaggggaagatcacggactggctaacctgtatgatgcagcaatgtcgagcatgatgtggggcctgctgaatggtttcctgcatggaaccgcactgctgggaaccgcgggcgtttcggcaacctctgtggttccgatgctgggtcaaggttgggaagcgatgactggtataattgcgcgctacgcagatcagattgatgccggtgtctatccagcagacgatgccacgattgatacccagcgtgctgcaatgcagcacctggtcgaggagagccgtgcggcgggcatcaatggcgaacttccggcgtttgtgaccaaactggccgatcgcgcagtggcagaaggtcgtggtggtgactcttacgctgcactgattgaacagtttcgcaagtcagcttaa

SEQ ID NO: 264 - protein, 292 aa, synthetic construct
  REGION 1..292: note = Imine reductase variant from Pseudonocardia spinosispora
MSDSPVPVTVLGLGLMGQALAGAFLAAGHPTTVWNRSAAKADELIGRGATLAASPAAAVAAGSLIVVCVTDHRAVRELLEPLGDALPGRVLVNLTSGTSREARENAEHTAAQGATYLDGVILTIPSGIGTPEATILYSGPRSTFDEHESALRALGPGATFVGEDHGLANLYDAAMSSMMWGLLNGFLHGTALLGTAGVSATSVVPMLGQGWEAMTGIIARYADQIDAGVYPADDATIDTQRAAMQHLVEESRAAGINGELPAFVTKLADRAVAEGRGGDSYAALIEQFRKSA

SEQ ID NO: 265 - DNA, 879 bp, synthetic construct
  misc_feature 1..879: note = Imine reductase variant from Pseudonocardia spinosispora
  source 1..879: mol_type = other DNA
atgagtgattcacctgtgcccgtgacagttctgggtcttggtctgatgggtcaggccttagcgggagcgtttctggcagccggtcaccctacgacggtttggaatcgcagcgcagctaaagctgatgaactggttggtcgcggtgcaaccctggccgcgtctcccgcggctgccgtcgcagcgggtagtctgatcgttgtttgcgtcacagatcatcgtgcggtgcgcgaactgctggaaccacttggcgatgcactgccaggtcgcgttctggtcaacctgacgagcggtacgtcgcgtgaagcccgtgagaacgcagaacatactgcggctcagggagccacctacctggatggtgtgattctgaccattccaagcggcattggcaccccagaagctaccattctgtattcgggaccgcgcagtaccttcgatgaacatgaaagcgcactgcgcgcattaggtccgggggcgacctttgtaggggaagatcacggactggctaacctgtatgatgcagcaatgtcgagcatgatgtggggcctgctgaatggtttcctgcatggaaccgcactgctgggaaccgcgggcgtttcggcaacctctgtggttccgatgctgggtaaaggttgggaagcgatgactggtataattgcgcgctacgcagatcagattgatgccggtgtctatccagcagacgatgccacgattgatacccagcgtgctgcaatgcagcacctggtcgaggagagccgtgcggcgggcatcaatggcgaacttccggcgtttgtgaccaaactggccgatcgcgcagtggcagaaggtcgtggtggtgactcttacgctgcactgattgaacagtttcgcaagtcagcttaa

SEQ ID NO: 266 - protein, 292 aa, synthetic construct
  REGION 1..292: note = Imine reductase variant from Pseudonocardia spinosispora
MSDSPVPVTVLGLGLMGQALAGAFLAAGHPTTVWNRSAAKADELVGRGATLAASPAAAVAAGSLIVVCVTDHRAVRELLEPLGDALPGRVLVNLTSGTSREARENAEHTAAQGATYLDGVILTIPSGIGTPEATILYSGPRSTFDEHESALRALGPGATFVGEDHGLANLYDAAMSSMMWGLLNGFLHGTALLGTAGVSATSVVPMLGKGWEAMTGIIARYADQIDAGVYPADDATIDTQRAAMQHLVEESRAAGINGELPAFVTKLADRAVAEGRGGDSYAALIEQFRKSA

SEQ ID NO: 267 - DNA, 879 bp, synthetic construct
  misc_feature 1..879: note = Imine reductase variant from Pseudonocardia spinosispora
  source 1..879: mol_type = other DNA
atgagtgattcacctgtgcccgtgacagttctgggtcttggtctgatgggtcaggccttagcgggagcgtttctggcagccggtcaccctacgacggtttggaatcgcagcgcagctaaagctgatgaactggttggtcgcggtgcaaccctggccgcgtctcccgcggctgccgtcgcagcgggtagtctgatcgttgtttgcgtcacagatcatcgtgcggtgcgcgaactgctggaaccacttggcgatgcactgccaggtcgcgttctggtcaacctgacgagcggtacgtcgcgtgaagcccgtgagaacgcagaacatactgcggctcagggagccacctacctggatggtgtgattctgaccattccaagcggcattggcaccccagaagctaggattctgtattcgggaccgcgcagtaccttcgatgaacatgaaagcgcactgcgcgcattaggtccgggggcgacctttgtaggggaagatcacggactggctaacctgtatgatgcagcaatgtcgagcatgatgtggggcctgctgaatggtttcctgcatggaaccgcactgctgggaaccgcgggcgtttcggcaacctctgtggttccgatgctgggtcaaggttgggaagcgatgactggtataattgcgcgctacgcagatcagattgatgccggtgtctatccagcagacgatgccacgattgatacccagcgtgctgcaatgcagcacctggtcgaggagagccgtgcggcgggcatcaatggcgaacttccggcgtttgtgaccaaactggccgatcgcgcagtggcagaaggtcgtggtggtgactcttacgctgcactgattgaacagtttcgcaagtcagcttaa

SEQ ID NO: 268 - protein, 292 aa, synthetic construct
  REGION 1..292: note = Imine reductase variant from Pseudonocardia spinosispora
MSDSPVPVTVLGLGLMGQALAGAFLAAGHPTTVWNRSAAKADELVGRGATLAASPAAAVAAGSLIVVCVTDHRAVRELLEPLGDALPGRVLVNLTSGTSREARENAEHTAAQGATYLDGVILTIPSGIGTPEARILYSGPRSTFDEHESALRALGPGATFVGEDHGLANLYDAAMSSMMWGLLNGFLHGTALLGTAGVSATSVVPMLGQGWEAMTGIIARYADQIDAGVYPADDATIDTQRAAMQHLVEESRAAGINGELPAFVTKLADRAVAEGRGGDSYAALIEQFRKSA

SEQ ID NO: 269 - DNA, 879 bp, synthetic construct
  misc_feature 1..879: note = Imine reductase variant from Pseudonocardia spinosispora
  source 1..879: mol_type = other DNA
atgagtgattcacctgtgcccgtgacagttctgggtcttggtctgatgggtcaggccttagcgggagcgtttctggcagccggtcaccctacgacggtttggaatcgcagcgcagctaaagctgatgaactggttggtcgcggtgcaaccctggccgcgtctcccgcggctgccgtcgcagcgggtagtctgatcgttgtttgcgtcacagatcatcgtgcggtgcgcgaactgctggaaccacttggcgatgcactgccaggtcgcgttctggtcaacctgacgagcggtacgtcgcgtgaagcccgtgagaacgcagaacatactgcggctcagggagccacctacctggatggtgtgattctgaccattccaagcggcattggcaccccagaagctaccattctgtattcgggaccgcgcagtaccttcgatgaacatgaaagcgcactgcgcgcattaggtccgggggcgacctttgtaggggaagatcacggactggctgcactgtatgatgcagcaatgctgagcgtcatgtggggcctgctgaatggtttcctgcatggaaccgcactgctgggaaccgcgggcgtttcggcaacctctgtggttccgatgctgggtcaaggtatcgaagcggtgaccggttggattgcgcgctacgcagatcagattgatgccggtgtctatccagcagacgacgccacgattgatacccagcgtgctgcaatgcagcacctggtcgaggagagccgtgcggcgggcatcaatggcgaacttccggcgtttgtgaccaaactggccgatcgcgcagtggcagaaggtcgtggtggtgactcttacgctgcactgattgaacagtttcgcaagtcagcttaa

SEQ ID NO: 270 - protein, 292 aa, synthetic construct; identical to SEQ ID NO: 2
  REGION 1..292: note = Imine reductase variant from Pseudonocardia spinosispora